European Patent Application EP 4 159 833 A2, published April 5, 2023. Title: FABRIC & HOME CARE PRODUCTS. Applicant: The Procter & Gamble Company. Application 18181021.9. The sequence listing filed with the application follows.

SEQUENCE LISTING (771 sequences)

SEQ ID NO: 1 - DNA, 1146 bp, Bacillus Amyloliquefaciens
gtgagaagcaaaaaattgtggatcagtttgctgtttgctttagcgttaatctttacgatggcgttcggcagcacatcctctgcccaggcggcagggaaatcaaacggggaaaagaaatatattgtcgggtttaaacagacaatgagcacgatgagcgccgctaagaagaaagatgtcatttctgaaaaaggcgggaaagtgcaaaagcaattcaaatatgtagacgcagcttcagctacattaaacgaaaaagctgtaaaagaattgaaaaaagacccgagcgtcgcttacgttgaagaagatcacgtagcacatgcgtacgcgcagtccgtgccttacggcgtatcacaaattaaagcccctgctctgcactctcaaggctacactggatcaaatgttaaagtagcggttatcgacagcggtatcgactcgagccatccagatcttaaagtcgctggaggggcttctatggtgccgtccgaaacaaacccgtttcaagataacaattctcatggcacacacgtcgcaggaacggttgcggcgttaaacaattctattggcgtgcttggtgtagccccgtctgcttcgctctacgccgttaaagttcttggcgcagacggatcaggccaatactcatggattatcaacggcatcgaatgggccatcgcgaataacatggatgtaatcaacatgagcctgggaggaccaagcggcagtgcggcacttaaagcagcagttgataaagctgttgcatctggtgtcgtcgtagtagcggcagctgggaatgagggaacatccggatcatcgagtaccgtcggttatccaggcaagtacccttcagtgattgcagtgggcgctgtagactcttcaaatcaacgtgcctctttttcctccgtgggaccggagctggatgtcatggcccctggcgtttctattcaatcgacgcttccagggaacaagtatggtgcgtataacgggacttccatggcctcgccgcatgtagctggggcggccgcattgattctttctaagcacccgaactggacaaacactcaagtccgcagcagtttagaaaacaccactacaaaacttggtgattctttctactatggaaaagggctgatcaacgtacaggcggcagctcag

SEQ ID NO: 2 - protein, 275 aa, Bacillus Amyloliquefaciens [sequence omitted]

SEQ ID NO: 3 - DNA, 825 bp, Artificial sequence
  Mutant of BPN'
gcgcagtccgtgccttacggcgtatcacaaattaaagcccctgctctgcactctcaaggctacactggatcaaatgttaaagtagcggttatcgacagcggtatcgactcgagccatccagatcttaaagtcgctggaggggcttctatggtgccgtccgaaacaaacccgtttcaagataacaattctcatggcacacacgtcgcaggaacggttgcggcgttaaacaattctattggcgtgcttggtgtagccccgtctgcttcgctctacgccgttaaagttcttgcagcagacggatcaggccaatactcatggattatcaacggcatcgaatgggccatcgcgaataacatggatgtaatcaacatgagcctgggagcaccaagcggcagtgcggcacttaaagcagcagttgataaagctgttgcatctggtgtcgtcgtagtagcggcagctgggaatgagggaacatccggatcatcgagtaccgtcggttatccaggcaagtacccttcagtgattgcagtgggcgctgtagactcttcaaatcaacgtgcctctttttcctccgtgggaccggagctggatgtcatggcccctggcgtttctattcaatcgacgcttccagggaacaagtatggtgcgcaaaacgggacttccatggcctcgccgcatgtagctggggcggccgcattgattctttctaagcacccgaactggacaaacactcaagtccgcagcagtttagaaaacaccactacaaaacttggtgattctttctactatggaaaagggctgatcaacgtacaggcggcagctcag

SEQ ID NO: 4 - protein, 275 aa, Artificial Sequence
  Mutant of subtilisin BPN'
AQSVPYGVSQIKAPALHSQGYTGSNVKVAVIDSGIDSSHPDLKVAGGASMVPSETNPFQDNNSHGTHVAGTVAALNNSIGVLGVAPSASLYAVKVLAADGSGQYSWIINGIEWAIANNMDVINMSLGAPSGSAALKAAVDKAVASGVVVVAAAGNEGTSGSSSTVGYPGKYPSVIAVGAVDSSNQRASFSSVGPELDVMAPGVSIQSTLPGNKYGAQNGTSMASPHVAGAAALILSKHPNWTNTQVRSSLENTTTKLGDSFYYGKGLINVQAAAQ

SEQ ID NO: 5 - DNA, 825 bp, Artificial Sequence
  Mutant of subtilisisn BPN'
gcgcagtccgtgccttacggcgtatcacaaattaaagcccctgctctgcactctcaaggctacactggaggcaatgttaaagtagcggttatcgacagcggtatcgactcgagccatccagatcttaaagtcgctggaggggcttctatggtgccgggcgaaacaaacccgtttcaagataacaattctcatggcacacacgtcgcaggaacggttgcggcgttaaacaataatattggcgtgcttggtgtagccccgtctgcttcgctctacgccgttaaagttcttggcgcagacggaaatggccaatactcatggattatcaacggcatcgaatgggccatcgcgaataacatggatgtaatcaacatgagcctgggagcaccaagcggcagtgcggcacttaaagcagcagttgataaagctgttgcatctggtgtcgtcgtagtagcggcagctgggaatgagggaacatccggatcatcgagtaccgtcggttatccaggcaagtacccttcagtgattgcagtgggcgctgtagactcttcaaatcaacgtgcctctttttcctccgtgggaccggagctggatgtcatggcccctggcgtttctattcaatcgacgcttccagggaacaagtatggtgcgcaaaacgggacttccatggcctcgccgcatgtagctggggcggccgcattgattctttctaagcacccgaactggacaaacactcaagtccgcagcagtttagaaaacaccactacaaaacttggtgattctttctactatggaaaagggctgatcaacgtacaggcggcagctcag

SEQ ID NO: 6 - protein, 275 aa, Artificial Sequence
  Mutant of subtilisin BPN'
AQSVPYGVSQIKAPALHSQGYTGGNVKVAVIDSGIDSSHPDLKVAGGASMVPGETNPFQDNNSHGTHVAGTVAALNNNIGVLGVAPSASLYAVKVLGADGNGQYSWIINGIEWAIANNMDVINMSLGAPSGSAALKAAVDKAVASGVVVVAAAGNEGTSGSSSTVGYPGKYPSVIAVGAVDSSNQRASFSSVGPELDVMAPGVSIQSTLPGNKYGAQNGTSMASPHVAGAAALILSKHPNWTNTQVRSSLENTTTKLGDSFYYGKGLINVQAAAQ

SEQ ID NO: 7 - DNA, 825 bp, Artificial Sequence
  Mutant of subtilisin BPN'
gcgcagtccgtgccttacggcgtatcacaaattaaagcccctgctctgcactctcaaggctacactggatcaaatgttaaagtagcggttatcgacagcggtattgattcgagccatccagatcttaaagtcgctggaggggcttctatggtgccgtccgaaacaaacccgtttcaagataacaattctcatggcacacacgtcgcaggaacggttgcggcgttaaacaataatattggcgtgcttggtgtagccccgtctgcttcgctctacgccgttaaagttcttgcagcagacggatcaggccaatactcatggattatcaacggcatcgaatgggccatcgcgaataacatggatgtaatcaacatgagcctgggagcaccaagcggcagtgcggcacttaaagcagcagttgataaagctgttgcatctggtgtcgtcgtagtagcggcagctgggaatgagggaacatccggatcatcgagtaccgtcggttatccaggcaagtacccttcagtgattgcagtgggcgctgtagactcttcaaatcaacgtgcctctttttcctccgtgggaccggagctggatgtcatggcccctggcgtttctattcaatcgacgcttccagggaacaagtatggtgcgcaaaacgggacttccatggcctcgccgcatgtagctggggcggccgcattgattctttctaagcacccgaactggacaaacactcaagtccgcagcagtttagaaaacaccactacaaaacttggtgattctttctactatggaaaagggctgatcaacgtacaggcggcagctcag

SEQ ID NO: 8 - protein, 275 aa, Artificial Sequence
  Mutant of subtilisin BPN'
AQSVPYGVSQIKAPALHSQGYTGSNVKVAVIDSGIDSSHPDLKVAGGASMVPSETNPFQDNNSHGTHVAGTVAALNNNIGVLGVAPSASLYAVKVLAADGSGQYSWIINGIEWAIANNMDVINMSLGAPSGSAALKAAVDKAVASGVVVVAAAGNEGTSGSSSTVGYPGKYPSVIAVGAVDSSNQRASFSSVGPELDVMAPGVSIQSTLPGNKYGAQNGTSMASPHVAGAAALILSKHPNWTNTQVRSSLENTTTKLGDSFYYGKGLINVQAAAQ

SEQ ID NO: 9 - DNA, 828 bp, Artificial Sequence
  Mutant of subtilisin BPN'
gcgcagtccgtgccttacggcgtatcacaaattaaagcccctgctctgcactctcaaggctacactggatcaaatgttaaagtagcggttatcgacagcggtatcgactcgagccatccagatcttaaagtcgctggaggggcttctatggtgccgggagaaacaaacccgtttcaagataacaattctcatggcacacacgcagcaggaacggttgcggcgttaaacaataatattggcgtgcttggtgtagccccgtctgcttcgctctacgccgttaaagttcttgcagcagacggatcagcacaatactcatggattatcaacggcatcgaatgggccatcgcgaataacatggatgtaatcaacatgagcctgggagcaacaagcggcagtgcggcacttaaagcagcagttgataaagctgttgcatctggtgtcgtcgtagtagcggcagctgggaatgagggaacatccggatcatcgagtaccgtcggttatccaggcaagtacccttcagtgattgcagtgggcgctgtagactcttcaaatacacgtgcctctttttcctccgtgggaccggagctggatgtcatggcccctggcgtttctattcaatcgacgcttccagggaacaagtatggtgcgcaaaacgggacttccatggcctcgccgcatgtagctggggcggccgcattgattctttctaagcacccgaactggacaaacactcaagtccgcagcagtttagaaaacaccactacaaaacttggtgattctttctactatggaaaagggctgatcaacgtacaggcggcagctcagtaa

SEQ ID NO: 10 - protein, 275 aa, Artificial Sequence
  Mutant of subtilisin BPN'
AQSVPYGVSQIKAPALHSQGYTGSNVKVAVIDSGIDSSHPDLKVAGGASMVPGETNPFQDNNSHGTHAAGTVAALNNNIGVLGVAPSASLYAVKVLAADGSAQYSWIINGIEWAIANNMDVINMSLGATSGSAALKAAVDKAVASGVVVVAAAGNEGTSGSSSTVGYPGKYPSVIAVGAVDSSNTRASFSSVGPELDVMAPGVSIQSTLPGNKYGAQNGTSMASPHVAGAAALILSKHPNWTNTQVRSSLENTTTKLGDSFYYGKGLINVQAAAQ

SEQ ID NO: 11 - DNA, 828 bp, Artificial Sequence
  Mutant of subtilisin BPN'
gcgcagtccgtgccttacggcgtatcacaaattaaagcccctgctctgcactctcaaggctacactggatcaaatgttaaagtagcggttatcgacagcggtatcgactcgagccatccagatcttaaagtcgctggaggggcttctatggtgccgtccgaaacaaacccgtttgtcgataacaattctcatggcacacacgtcgcaggaacggttgcggcgttaaacaataatattggcgtgcttggtgtagccccgtctgcttcgctctacgccgttaaagttcttgcagcagacggatcaggccaatactcatggattgtcaacggcatcgaatgggccatcgcgaataacatggatgtaatcaacatgagcctgggagcaccaagcggcagtgcggcacttaaagcagcagttgataaagctgttgcatctggtcaagtcgtagtagcggcagctgggaatgagggaacatccggatcatcgagtaccgtcggttatccaggcaagtacccttcagtgattgcagtgggcgctgtagactcttcaaatcaacgtgcctctttttcctccgtgggaccggagctggatgtcatggcccctggcgtttctattcaatcgacgcttccagcaaacaagtatggtgcgcaaaacgggacttccatggcctcgccgcatgtagctggggcggccgcattgattctttctaagcacccgaactggacaaacactcaagtccgcagcagtttagaacaaaccactacaaaacttggtgattctttctactatggaaaagggctgatcaacgtacaggcggcagctcagtaa

SEQ ID NO: 12 - protein, 275 aa, Artificial Sequence
  Mutant of subtilisin BPN'
AQSVPYGVSQIKAPALHSQGYTGSNVKVAVIDSGIDSSHPDLKVAGGASMVPSETNPFVDNNSHGTHVAGTVAALNNNIGVLGVAPSASLYAVKVLAADGSGQYSWIVNGIEWAIANNMDVINMSLGAPSGSAALKAAVDKAVASGQVVVAAAGNEGTSGSSSTVGYPGKYPSVIAVGAVDSSNQRASFSSVGPELDVMAPGVSIQSTLPANKYGAQNGTSMASPHVAGAAALILSKHPNWTNTQVRSSLEQTTTKLGDSFYYGKGLINVQAAAQ

SEQ ID NO: 13 - DNA, 828 bp, Artificial Sequence
  Mutant of subtilisin BPN'
gcgcagtccgtgccttacggcgtatcacaaattaaagcccctgctctgcactctcaaggctacactggatcaaatgttaaagtagcggttatcgacagcggtatcgactcgagccatccagatcttaaagtcgctggaggggcttctatggtgccgtccgaaacaaacccgtttcaagatgcaaattctcatggcacacacgtcgcaggaacggttgcggcgttaaacaataatattggcgtgcttggtgtagccccggaagcttcgctctacgccgttaaagttcttgcagcagacggatcaggccaatactcatggattatcaacggcatcgaatgggccatcgcgaataacatggatgtaatcaacatcagcctgggagcaccaagcggcagtgcggcacttaaagcagcagttgataaagctgttgcatctggtgtcgtcgtagtagcggcagctgggaatgagggaacatccggaccttcgagtaccgtcggttatccaggcaagtacccttcagtgattgcagtgggcgctgtagactcttcaaatcaacgtgcctctttttcctccgtgggaccggagctggatgtcatggcccctggcgtttctattcaatcgacgcttccagggaacaagtatggtgcgcaaaacgggacttccatggccgcaccgcatgtagctggggcggccgcattgattctttctaagcacccgaactggacaaacactcaagtccgcagcagtttagaaaacaccactacaaaacttggtgattctttctactatggaaaagggctgatcaacgtacaggcggcagctcagtaa

SEQ ID NO: 14 - protein, 275 aa, Artificial Sequence
  Mutant of subtilisn BPN'
AQSVPYGVSQIKAPALHSQGYTGSNVKVAVIDSGIDSSHPDLKVAGGASMVPSETNPFQDANSHGTHVAGTVAALNNNIGVLGVAPEASLYAVKVLAADGSGQYSWIINGIEWAIANNMDVINISLGAPSGSAALKAAVDKAVASGVVVVAAAGNEGTSGPSSTVGYPGKYPSVIAVGAVDSSNQRASFSSVGPELDVMAPGVSIQSTLPGNKYGAQNGTSMAAPHVAGAAALILSKHPNWTNTQVRSSLENTTTKLGDSFYYGKGLINVQAAAQ

SEQ ID NO: 15 - DNA, 828 bp, Artificial Sequence
  Mutant of subtilisin BPN'
gcgcagtccgtgccttacggcgtatcacaaattaaagcccctgctctgcactctcaaggctacactggatcaaatgttaaagtagcggttatcgacagcggtatcgactcgagccatccagatcttaaagtcgctggaggggcttctatggtgccgtccgaaacaaacccgtttcaagataaccaatctcatggcacacacgtcgcaggaacggttgcggcgttaaacaataatattggcgtgcttggtgtagccccgtctgcttcgctctacgccgttaaagttcttgcagcagacaactcaggccaatactcatggattatcaacggcatcgaatgggccatcgcgaataacatggatgtaatcaacatggcactgggagcaccaagcggcagtgcggcacttaaagcagcagttgataaagctgttgcatctggtgtcgtcgtagtagcggcagctgggaatgagggaacagatggatcatcgagtaccgtcggttatccaggcaagtacccttcagtgattgcagtgggcgctgtagactcttcaaatcaacgtgcctctttttcctccgtgggaccggagctggatgtcatggcccctggcgtttctattcaatcgacgcttccagggaacaagtatggtgcgcaaaacgggacttccatggcctcgccgcatgtagctggggcggccgcattgattctttctaagcacccgtcatggacaaacactcaagtccgcagcagtttagaaaacaccactacaaaacttggtgattctttctactatggaaaagggctgatcaacgtacaggcggcagctcagtaa

SEQ ID NO: 16 - protein, 275 aa, Artificial Sequence
  Mutant of subtilisin BPN'
AQSVPYGVSQIKAPALHSQGYTGSNVKVAVIDSGIDSSHPDLKVAGGASMVPSETNPFQDNQSHGTHVAGTVAALNNNIGVLGVAPSASLYAVKVLAADNSGQYSWIINGIEWAIANNMDVINMALGAPSGSAALKAAVDKAVASGVVVVAAAGNEGTDGSSSTVGYPGKYPSVIAVGAVDSSNQRASFSSVGPELDVMAPGVSIQSTLPGNKYGAQNGTSMASPHVAGAAALILSKHPSWTNTQVRSSLENTTTKLGDSFYYGKGLINVQAAAQ

SEQ ID NO: 17 - DNA, 828 bp, Artificial Sequence
  Mutant of subtilisin BPN'
gcgcagtccgtgccttacggcgtatcacaaattaaagcccctgctctgcactctcaaggctacactggatcaaatgttaaagtagcggttatcgacagcggtatcgactcgagccatccagatcttaaagtcgctggaggggcttctatggtgccgtccgaaacaaacccgtttcaagataacaatacacatggcacacacgtcgcaggaacggttgcggcgttaaacaataatattggcgtgcttggtgtagccccgtctgcttcgctctacgccgttaaagttcttgcagcagacggagcaggccaatactcatggattatcaacggcatcgaatgggccatcgcgaataacatggatgtaatcaacatgagcgtcggagcaccaagcggcagtgcggcacttaaagcagcagttgataaagctgttgcatctggtgtcgtcgtagtagcggcagctgggaatgagggaacatccggatcatcgagtaccgtcggttatccaggcaagtacccttcagtgattgcagtgggcgctgtagactctacaaatcaacgtgcctctttttcctccgtgggaccggagctggatgtcatggcccctggcgtttctattcaatcgacgcttccagggaacaagtatggtgcgcaaaacgggacttccatggcctcgccgcatgtagctggggcggccgcattgattctttctaagcacccgaactggacaaacaaccaagtccgcagcagtttagaaaacaccactacaaaacttggtgattctttctactatggaaaagggctgatcaacgtacaggcggcagctcagtaa

SEQ ID NO: 18 - protein, 275 aa, Artificial Sequence
  Mutant of subtilisin BPN'
AQSVPYGVSQIKAPALHSQGYTGSNVKVAVIDSGIDSSHPDLKVAGGASMVPSETNPFQDNNTHGTHVAGTVAALNNNIGVLGVAPSASLYAVKVLAADGAGQYSWIINGIEWAIANNMDVINMSVGAPSGSAALKAAVDKAVASGVVVVAAAGNEGTSGSSSTVGYPGKYPSVIAVGAVDSTNQRASFSSVGPELDVMAPGVSIQSTLPGNKYGAQNGTSMASPHVAGAAALILSKHPNWTNNQVRSSLENTTTKLGDSFYYGKGLINVQAAAQ

SEQ ID NO: 19 - DNA, 828 bp, Artificial Sequence
  Mutant of subtilisin BPN'
gcgcagtccgtgccttacggcgtatcacaaattaaagcccctgctctgcactctcaaggctacactggatcaaatgttaaagtagcggttatcgacagcggtatcgactcgagccatctggatcttaaagtcgctggaggggcttctatggtgccgggagaaacaaacccgtttgtcgatgcacaaacacatggcacacacgtcgcaggaacggttgcggcgttaaacaataatattggcgtgcttggtgtagccccggaagcttcgctctacgccgttaaagttcttgcagcagacaacgcagcacaatactcatggattgtcaacggcatcgaatgggccatcgcgaataacatggatgtaatcaacatgagcctgggagcaccaagcggcagtgcggcacttaaagcagcagttgataaagctgttgcatctggtgtcgtcgtagtagcggcagctgggaatgagggaacatccggatcatcgagtaccgtcggttatccaggcaagtacccttcagtgattgcagtgggcgctgtagactcttcaaatcaacgtgcctctttttcctccgtgggaccggagctggatgtcatggcccctggcgtttctattcaatcgacgcttccagggaacaagtatggtgcgcaaaacgggacttccatggcctcgccgcatgtagctggggcggccgcattgattctttctaagcacccgaactggacaaacactcaagtccgcagcagtttagaaaacaccactacaaaacttggtgattctttctactatggaaaagggctgatcaacgtacaggcggcagctcagtaa

SEQ ID NO: 20 - protein, 275 aa, Artificial Sequence
  Mutant of subtilisin BPN'
AQSVPYGVSQIKAPALHSQGYTGSNVKVAVIDSGIDSSHLDLKVAGGASMVPGETNPFVDAQTHGTHVAGTVAALNNNIGVLGVAPEASLYAVKVLAADNAAQYSWIVNGIEWAIANNMDVINMSLGAPSGSAALKAAVDKAVASGVVVVAAAGNEGTSGSSSTVGYPGKYPSVIAVGAVDSSNQRASFSSVGPELDVMAPGVSIQSTLPGNKYGAQNGTSMASPHVAGAAALILSKHPNWTNTQVRSSLENTTTKLGDSFYYGKGLINVQAAAQ

SEQ ID NO: 21 - DNA, 828 bp, Artificial Sequence
  Mutant of subtilisin BPN'
gcgcagtccgtgccttacggcgtatcacaaattaaagcccctgctctgcactctcaaggctacactggatcaaatgttaaagtagcggttatcgacagcggtatcgactcgagccatccagatcttaaagtcgctggaggggcttctatggtgccgtccgaaacaaacccgtttcaagataacaattctcatggcacacacgtcgcaggaacggttgcggcgttaaacaataatattggcgtgcttggtgtagccccgtctgcttcgctctacgccgttaaagttcttgcagcagacggatcaggccaatactcatggattatcaacggcatcgaatgggccatcgcgaataacatggatgtaatcaacatgagcctgggagcaacaagcggcagtgcggcacttaaagcagcagttgataaagctgttgcatctggtcaagtcgtagtagcggcagctgggaatgagggaacagatggaccttcgagtaccgtcggttatccaggcaagtacccttcagtgattgcagtgggcgctgtagactctacaaatacacgtgcctctttttcctccgtgggaccggagctggatgtcatggcccctggcgtttctattcaatcgacgcttccagcaaacaagtatggtgcgcaaaacgggacttccatggccgcaccgcatgtagctggggcggccgcattgattctttctaagcacccgtcatggacaaacaaccaagtccgcagcagtttagaacaaaccactacaaaacttggtgattctttctactatggaaaagggctgatcaacgtacaggcggcagctcagtaa

SEQ ID NO: 22 - protein, 275 aa, Artificial Sequence
  Mutant of subtilisin BPN'
AQSVPYGVSQIKAPALHSQGYTGSNVKVAVIDSGIDSSHPDLKVAGGASMVPSETNPFQDNNSHGTHVAGTVAALNNNIGVLGVAPSASLYAVKVLAADGSGQYSWIINGIEWAIANNMDVINMSLGATSGSAALKAAVDKAVASGQVVVAAAGNEGTDGPSSTVGYPGKYPSVIAVGAVDSTNTRASFSSVGPELDVMAPGVSIQSTLPANKYGAQNGTSMAAPHVAGAAALILSKHPSWTNNQVRSSLEQTTTKLGDSFYYGKGLINVQAAAQ

SEQ ID NO: 23 - DNA, 828 bp, Artificial Sequence
  Mutant of subtilisin BPN'
gcgcagtccgtgccttacggcgtatcacaaattaaagcccctgctctgcactctcaaggctacactggatcaaatgttaaagtagcggttatcgacagcggtatcgactcgagccatccagatcttaaagtcgctggaggggcttctatggtgccgtccgaaacaaacccgtttcaagataacaattctcatggcacacacgcagcaggaacggttgcggcgttaaacaataatattggcgtgcttggtgtagccccgtctgcttcgctctacgccgttaaagttcttgcagcagacggatcagcacaatactcatggattatcaacggcatcgaatgggccatcgcgaataacatggatgtaatcaacatggcactgggagcaccaagcggcagtgcggcacttaaagcagcagttgataaagctgttgcatctggtgtcgtcgtagtagcggcagctgggaatgagggaacatccggatcatcgagtaccgtcggttatccaggcaagtacccttcagtgattgcagtgggcgctgtagactcttcaaatcaacgtgcctctttttcctccgtgggaccggagctggatgtcatggcccctggcgtttctattcaatcgacgcttccagcaaacaagtatggtgcgcaaaacgggacttccatggcctcgccgcatgtagctggggcggccgcattgattctttctaagcacccgaactggacaaacactcaagtccgcagcagtttagaaaacaccactacaaaacttggtgattctttctactatggaaaagggctgatcaacgtacaggcggcagctcagtaa

SEQ ID NO: 24 - protein, 275 aa, Artificial Sequence
  Mutant of subtilisin BPN'
AQSVPYGVSQIKAPALHSQGYTGSNVKVAVIDSGIDSSHPDLKVAGGASMVPSETNPFQDNNSHGTHAAGTVAALNNNIGVLGVAPSASLYAVKVLAADGSAQYSWIINGIEWAIANNMDVINMALGAPSGSAALKAAVDKAVASGVVVVAAAGNEGTSGSSSTVGYPGKYPSVIAVGAVDSSNQRASFSSVGPELDVMAPGVSIQSTLPANKYGAQNGTSMASPHVAGAAALILSKHPNWTNTQVRSSLENTTTKLGDSFYYGKGLINVQAAAQ

SEQ ID NO: 25 - DNA, 36 bp, Artificial Sequence
  Primer
cttctatggtgccgtccgaaacaaacccgtttcaag

SEQ ID NO: 26 - DNA, 34 bp, Artificial Sequence
  Primer
tcatggcacacacgtcgcaggaacggttgcggcg

SEQ ID NO: 27 - DNA, 37 bp, Artificial Sequence
  Primer
agcagacggatcaggccaatactcatggattatcaac

SEQ ID NO: 28 - DNA, 39 bp, Artificial Sequence
  Primer
tgagcctgggagcaccaagcggcagtgcggcacttaaag

SEQ ID NO: 29 - DNA, 38 bp, Artificial Sequence
  Primer
tagactcttcaaatcaacgtgcctctttttcctccgtg

SEQ ID NO: 30 - DNA, 34 bp, Artificial Sequence
  Primer
gaaacaaacccgtttcaagataacaattctcatg

SEQ ID NO: 31 - DNA, 37 bp, Artificial Sequence
  Primer
atactcatggattatcaacggcatcgaatgggccatc

SEQ ID NO: 32 - DNA, 36 bp, Artificial Sequence
  Primer
tgttgcatctggtgtcgtcgtagtagcggcagctgg

SEQ ID NO: 33 - DNA, 37 bp, Artificial Sequence
  Primer
atcgacgcttccagggaacaagtatggtgcgcaaaac

SEQ ID NO: 34 - DNA, 35 bp, Artificial Sequence
  Primer
cagcagtttagaaaacaccactacaaaacttggtg

SEQ ID NO: 35 - DNA, 38 bp, Artificial Sequence
  Primer
caaacccgtttcaagataacaattctcatggcacacac

SEQ ID NO: 36 - DNA, 39 bp, Artificial Sequence
  Primer
ttggtgtagccccgtctgcttcgctctacgccgttaaag

SEQ ID NO: 37 - DNA, 36 bp, Artificial Sequence
  Primer
tggatgtaatcaacatgagcctgggagcaccaagcg

SEQ ID NO: 38 - DNA, 39 bp, Artificial Sequence
  Primer
agggaacatccggatcatcgagtaccgtcggttatccag

SEQ ID NO: 39 - DNA, 36 bp, Artificial Sequence
  Primer
gacttccatggcctcgccgcatgtagctggggcggc

SEQ ID NO: 40 - DNA, 36 bp, Artificial Sequence
  Primer
gtttcaagataacaattctcatggcacacacgtcgc

SEQ ID NO: 41 - DNA, 35 bp, Artificial Sequence
  Primer
gttcttgcagcagacggatcaggccaatactcatg

SEQ ID NO: 42 - DNA, 37 bp, Artificial Sequence
  Primer
atgtaatcaacatgagcctgggagcaccaagcggcag

SEQ ID NO: 43 - DNA, 37 bp, Artificial Sequence
  Primer
ggaatgagggaacatccggatcatcgagtaccgtcgg

SEQ ID NO: 44 - DNA, 38 bp, Artificial Sequence
  Primer
ctttctaagcacccgaactggacaaacactcaagtccg

SEQ ID NO: 45 - DNA, 36 bp, Artificial Sequence
  Primer
tcaagataacaattctcatggcacacacgtcgcagg

SEQ ID NO: 46 - DNA, 37 bp, Artificial Sequence
  Primer
tgcagcagacggatcaggccaatactcatggattatc

SEQ ID NO: 47 - DNA, 35 bp, Artificial Sequence
  Primer
aatcaacatgagcctgggagcaccaagcggcagtg

SEQ ID NO: 48 - DNA, 37 bp, Artificial Sequence
  Primer
cgctgtagactcttcaaatcaacgtgcctctttttcc

SEQ ID NO: 49 - DNA, 35 bp, Artificial Sequence
  Primer
gaactggacaaacactcaagtccgcagcagtttag

SEQ ID NO: 50 - DNA, 34 bp, Artificial Sequence; identical to SEQ ID NO: 26
  Primer

SEQ ID NO: 51 - DNA, 37 bp, Artificial Sequence; identical to SEQ ID NO: 27
  Primer

SEQ ID NO: 52 - DNA, 37 bp, Artificial Sequence; identical to SEQ ID NO: 33
  Primer

SEQ ID NO: 53 - DNA, 37 bp, Artificial Sequence; identical to SEQ ID NO: 42
  Primer

SEQ ID NO: 54 - DNA, 22 bp, Artificial Sequence
  Primer
tacatatgagttatgcagtttg

SEQ ID NO: 55 - DNA, 19 bp, Artificial Sequence
  Primer
ttatcctttaccttgtctc

SEQ ID NO: 56 - DNA, 35 bp, Artificial Sequence
  Primer
caacatgagcctgggatcaccaagcggcagtgcgg

SEQ ID NO: 57 - DNA, 35 bp, Artificial Sequence
  Primer
ccgcactgccgcttggtgatcccaggctcatgttg

SEQ ID NO: 58 - DNA, 38 bp, Artificial Sequence
  Primer
ctatggtgccgggcgaaacaaacccgtttcaagatccg

SEQ ID NO: 59 - DNA, 38 bp, Artificial Sequence
  Primer
cggatcttgaaacgggtttgtttcgcccggcaccatag

SEQ ID NO: 60 - DNA, 21 bp, Artificial Sequence
  Primer
gcctcacatttgtgccaccta

SEQ ID NO: 61 - DNA, 22 bp, Artificial Sequence
  Primer
cctctcggttatgagttagttc

SEQ ID NO: 62 - DNA, 24 bp, Artificial Sequence
  Primer
aaaggatcctaatcggcgcttttc

SEQ ID NO: 63 - DNA, 24 bp, Artificial Sequence
  Primer
cttgtctccaagcttaaaataaaa

SEQ ID NO: 64 - DNA, 36 bp, Artificial Sequence
  Primer
cagatcttaaagtctctggaggggcttctatggtgc

SEQ ID NO: 65 - DNA, 40 bp, Artificial Sequence
  Primer
catagaagcccctccagagactttaagatctggatggctc

SEQ ID NO: 66 - DNA, 36 bp, Artificial Sequence
  Primer
gcattgattctttacaagcacccgaactggacaaac

SEQ ID NO: 67 - DNA, 39 bp, Artificial Sequence
  Primer
cagttcgggtgcttgtaaagaatcaatgcggccgcccca

SEQ ID NO: 68 - DNA, 36 bp, Artificial Sequence
  Primer
gcattgattcttggtaagcacccgaactggacaaac

SEQ ID NO: 69 - DNA, 40 bp, Artificial Sequence
  Primer
ccagttcgggtgcttaccaagaatcaatgcggccgcccca

SEQ ID NO: 70 - DNA, 40 bp, Artificial Sequence
  Primer
catcgaatgggccacagcgaataacatggatgtaatcaac

SEQ ID NO: 71 - DNA, 40 bp, Artificial Sequence
  Primer
catccatgttattcgctgtggcccattcgatgccgttgat

SEQ ID NO: 72 - DNA, 40 bp, Artificial Sequence
  Primer
catcgaatgggccgtagcgaataacatggatgtaatcaac

SEQ ID NO: 73 - DNA, 40 bp, Artificial Sequence
  Primer
catccatgttattcgctacggcccattcgatgccgttgat

SEQ ID NO: 74 - DNA, 36 bp, Artificial Sequence
  Primer
ctgtagactctacaaatcaacgtgcctctttttcct

SEQ ID NO: 75 - DNA, 40 bp, Artificial Sequence
  Primer
aaagaggcacgttgatttgtagagtctacagcgcccactg

SEQ ID NO: 76 - DNA, 38 bp, Artificial Sequence
  Primer
ctgtagactcttcataccaacgtgcctctttttcctcc

SEQ ID NO: 77 - DNA, 40 bp, Artificial Sequence
  Primer
gaaaaagaggcacgttggtatgaagagtctacagcgccca

SEQ ID NO: 78 - DNA, 51 bp, Artificial Sequence
  Primer
tagcggttacagacagcggtatcgacccaagccatccagatcttaaagtcg

SEQ ID NO: 79 - DNA, 50 bp, Artificial Sequence
  Primer
atggcttgggtcgataccgctgtctgtaaccgctactttaacattgcctc

SEQ ID NO: 80 - DNA, 49 bp, Artificial Sequence
  Primer
taaagtagcggttacagacagcggtttagactcgagccatccagatctt

SEQ ID NO: 81 - DNA, 50 bp, Artificial Sequence
  Primer
atggctcgagtctaaaccgctgtctgtaaccgctactttaacattgcctc

SEQ ID NO: 82 - DNA, 50 bp, Artificial Sequence
  Primer
ggttgtagacagcggtatcgactcgtggcatccagatcttaaagtcgctg

SEQ ID NO: 83 - DNA, 50 bp, Artificial Sequence
  Primer
atgccacgagtcgataccgctgtctacaaccgctactttaacattgcctc

SEQ ID NO: 84 - DNA, 38 bp, Artificial Sequence
  Primer
ctacactggaggcaaagttaaagtagcggttatcgaca

SEQ ID NO: 85 - DNA, 40 bp, Artificial Sequence
  Primer
ataaccgctactttaactttgcctccagtgtagccttgag

SEQ ID NO: 86 - DNA, 37 bp, Artificial Sequence
  Primer
gagcctgggagcacgtagcggcagtgcggcacttaaa

SEQ ID NO: 87 - DNA, 40 bp, Artificial Sequence
  Primer
gtgccgcactgccgctacgtgctcccaggctcatgttgat

SEQ ID NO: 88 - DNA, 38 bp, Artificial Sequence
  Primer
tgagcctgggagcaaagagcggcagtgcggcacttaaa

SEQ ID NO: 89 - DNA, 38 bp, Artificial Sequence; identical to SEQ ID NO: 88
  Primer

SEQ ID NO: 90 - DNA, 40 bp, Artificial Sequence
  Primer
atcacaaattaaagccacagctctgcactctcaaggctac

SEQ ID NO: 91 - DNA, 40 bp, Artificial Sequence
  Primer
agagtgcagagctgtggctttaatttgtgatacgccgtaa

SEQ ID NO: 92 - DNA, 40 bp, Artificial Sequence; identical to SEQ ID NO: 91
  Primer

SEQ ID NO: 93 - DNA, 40 bp, Artificial Sequence
  Primer
taagatctggatggcttgtgtcgataccgctgtcgataac

SEQ ID NO: 94 - DNA, 40 bp, Artificial Sequence
  Primer
gacagcggtatcgacccaagccatccagatcttaaagtcg

SEQ ID NO: 95 - DNA, 40 bp, Artificial Sequence
  Primer
taagatctggatggcttgggtcgataccgctgtcgataac

SEQ ID NO: 96 - DNA, 40 bp, Artificial Sequence
  Primer
gacagcggtatcgactggagccatccagatcttaaagtcg

SEQ ID NO: 97 - DNA, 40 bp, Artificial Sequence
  Primer
taagatctggatggctccagtcgataccgctgtcgataac

SEQ ID NO: 98 - DNA, 40 bp, Artificial Sequence
  Primer
acgcgcagtccgtgttatacggcgtatcacaaattaaagc

SEQ ID NO: 99 - DNA, 40 bp, Artificial Sequence
  Primer
atttgtgatacgccgtataacacggactgcgcgtacgcat

SEQ ID NO: 100 - DNA, 37 bp, Artificial Sequence
  Primer
acaagtatggtgcgaaaaacgggacttccatggcctc

SEQ ID NO: 101 - DNA, 38 bp, Artificial Sequence
  Primer
catggaagtcccgtttttcgcaccatacttgttccctg

SEQ ID NO: 102 - DNA, 37 bp, Artificial Sequence
  Primer
acaagtatggtgcgggaaacgggacttccatggcctc

SEQ ID NO: 103 - DNA, 39 bp, Artificial Sequence
  Primer
ccatggaagtcccgtttcccgcaccatacttgttccctg

SEQ ID NO: 104 - DNA, 38 bp, Artificial Sequence
  Primer
cttacggcgtatcattaattaaagcccctgctctgcac

SEQ ID NO: 105 - DNA, 40 bp, Artificial Sequence
  Primer
gagcaggggctttaattaatgatacgccgtaaggcacgga

SEQ ID NO: 106 - DNA, 38 bp, Artificial Sequence
  Primer
cttacggcgtatcacgtattaaagcccctgctctgcac

SEQ ID NO: 107 - DNA, 40 bp, Artificial Sequence
  Primer
gagcaggggctttaatacgtgatacgccgtaaggcacgga

SEQ ID NO: 108 - DNA, 40 bp, Artificial Sequence
  Primer
tttagaaaacacctctacaaaacttggtgattctttctac

SEQ ID NO: 109 - DNA, 40 bp, Artificial Sequence
  Primer
tcaccaagttttgtagaggtgttttctaaactgctgcgga

SEQ ID NO: 110 - DNA, 40 bp, Artificial Sequence
  Primer
aggctacactggagcaaatgttaaagtagcggttatcgac

SEQ ID NO: 111 - DNA, 38 bp, Artificial Sequence
  Primer
gctactttaacatttgctccagtgtagccttgagagtg

SEQ ID NO: 112 - DNA, 39 bp, Artificial Sequence
  Primer
gagggaacatccggaccatcgagtaccgtcggttatcca

SEQ ID NO: 113 - DNA, 40 bp, Artificial Sequence
  Primer
accgacggtactcgatggtccggatgttccctcattccca

SEQ ID NO: 114 - DNA, 40 bp, Artificial Sequence
  Primer
agggaacatccggaccattaagtaccgtcggttatccagg

SEQ ID NO: 115 - DNA, 40 bp, Artificial Sequence
  Primer
accgacggtacttaatggtccggatgttccctcattccca

SEQ ID NO: 116 - DNA, 39 bp, Artificial Sequence
  Primer
gaacatccggatcattaagtaccgtcggttatccaggca

SEQ ID NO: 117 - DNA, 40 bp, Artificial Sequence
  Primer
ataaccgacggtacttaatgatccggatgttccctcattc

SEQ ID NO: 118 - DNA, 39 bp, Artificial Sequence
  Primer
gaacatccggatcaccaagtaccgtcggttatccaggca

SEQ ID NO: 119 - DNA, 40 bp, Artificial Sequence
  Primer
ataaccgacggtacttggtgatccggatgttccctcattc

SEQ ID NO: 120 - DNA, 38 bp, Artificial Sequence
  Primer
gtttagaaaacgcaactacaaaacttggtgattctttc

SEQ ID NO: 121 - DNA, 40 bp, Artificial Sequence
  Primer
caccaagttttgtagttgcgttttctaaactgctgcggac

SEQ ID NO: 122 - DNA, 40 bp, Artificial Sequence
  Primer
caaaacttggtgatccattctactatggaaaagggctgat

SEQ ID NO: 123 - DNA, 40 bp, Artificial Sequence
  Primer
tttccatagtagaatggatcaccaagttttgtagtggtgt

SEQ ID NO: 124 - DNA, 40 bp, Artificial Sequence
  Primer
caaaacttggtgataacttctactatggaaaagggctgat

SEQ ID NO: 125 - DNA, 40 bp, Artificial Sequence
  Primer
tttccatagtagaagttatcaccaagttttgtagtggtgt

SEQ ID NO: 126 - DNA, 40 bp, Artificial Sequence
  Primer
caaaacttggtgatatcttctactatggaaaagggctgat

SEQ ID NO: 127 - DNA, 40 bp, Artificial Sequence
  Primer
tttccatagtagaagatatcaccaagttttgtagtggtgt

SEQ ID NO: 128 - DNA, 40 bp, Artificial Sequence
  Primer
caaaacttggtgatggattctactatggaaaagggctgat

SEQ ID NO: 129 - DNA, 40 bp, Artificial Sequence
  Primer
tttccatagtagaatccatcaccaagttttgtagtggtgt

SEQ ID NO: 130 - DNA, 37 bp, Artificial Sequence
  Primer
gtgggcgctgtacactcttcaaatcaacgtgcctctt

SEQ ID NO: 131 - DNA, 40 bp, Artificial Sequence
  Primer
cacgttgatttgaagagtgtacagcgcccactgcaatcac

SEQ ID NO: 132 - DNA, 37 bp, Artificial Sequence
  Primer
gtgggcgctgtaggatcttcaaatcaacgtgcctctt

SEQ ID NO: 133 - DNA, 40 bp, Artificial Sequence
  Primer
cacgttgatttgaagatcctacagcgcccactgcaatcac

SEQ ID NO: 134 - DNA, 37 bp, Artificial Sequence
  Primer
cctgctctgcacttccaaggctacactggaggcaatg

SEQ ID NO: 135 - DNA, 40 bp, Artificial Sequence
  Primer
ctccagtgtagccttggaagtgcagagcaggggctttaat

SEQ ID NO: 136 - DNA, 37 bp, Artificial Sequence
  Primer
cctgctctgcacacacaaggctacactggaggcaatg

SEQ ID NO: 137 - DNA, 40 bp, Artificial Sequence
  Primer
ctccagtgtagccttgtgtgtgcagagcaggggctttaat

SEQ ID NO: 138 - DNA, 37 bp, Artificial Sequence
  Primer
cctgctctgcacccacaaggctacactggaggcaatg

SEQ ID NO: 139 - DNA, 40 bp, Artificial Sequence
  Primer
ctccagtgtagccttgtgggtgcagagcaggggctttaat

SEQ ID NO: 140 - DNA, 37 bp, Artificial Sequence
  Primer
cctgctctgcactaccaaggctacactggaggcaatg

SEQ ID NO: 141 - DNA, 40 bp, Artificial Sequence
  Primer
ctccagtgtagccttggtagtgcagagcaggggctttaat

SEQ ID NO: 142 - DNA, 37 bp, Artificial Sequence
  Primer
cctgctctgcacttacaaggctacactggaggcaatg

SEQ ID NO: 143 - DNA, 40 bp, Artificial Sequence
  Primer
ctccagtgtagccttgtaagtgcagagcaggggctttaat

SEQ ID NO: 144 - DNA, 38 bp, Artificial Sequence
  Primer
tgctctgcactctttaggctacactggaggcaatgtta

SEQ ID NO: 145 - DNA, 40 bp, Artificial Sequence
  Primer
ttgcctccagtgtagcctaaagagtgcagagcaggggctt

SEQ ID NO: 146 - DNA, 39 bp, Artificial Sequence
  Primer
atcgcgaataacatgaacgtaatcaacatgagcctggga

SEQ ID NO: 147 - DNA, 39 bp, Artificial Sequence
  Primer
ctcatgttgattacgttcatgttattcgcgatggcccat

SEQ ID NO: 148 - DNA, 37 bp, Artificial Sequence
  Primer
cttccagggaaccgttatggtgcgcaaaacgggactt

SEQ ID NO: 149 - DNA, 39 bp, Artificial Sequence
  Primer
gttttgcgcaccataacggttccctggaagcgtcgattg

SEQ ID NO: 150 - DNA, 40 bp, Artificial Sequence
  Primer
ctgcacttacaaggctctactggaggcaatgttaaagtag

SEQ ID NO: 151 - DNA, 49 bp, Artificial Sequence
  Primer
taacattgcctccagtagagccttgtaagtgcagagcaggggctttaat

SEQ ID NO: 152 - DNA, 43 bp, Artificial Sequence
  Primer
gctctgcacttacaaggcaacactggaggcaatgttaaagtag

SEQ ID NO: 153 - DNA, 48 bp, Artificial Sequence
  Primer
aacattgcctccagtgttgccttgtaagtgcagagcaggggctttaat

SEQ ID NO: 154 - DNA, 35 bp, Artificial Sequence
  Primer
cttacggcgtaacacaaattaaagcccctgctctg

SEQ ID NO: 155 - DNA, 38 bp, Artificial Sequence
  Primer
aggggctttaatttgtgttacgccgtaaggcacggact

SEQ ID NO: 156 - DNA, 40 bp, Artificial Sequence
  Primer
ttaaagcagcagttgatttcgctgttgcatctggtgtcgt

SEQ ID NO: 157 - DNA, 40 bp, Artificial Sequence
  Primer
agatgcaacagcgaaatcaactgctgctttaagtgccgca

SEQ ID NO: 158 - DNA, 40 bp, Artificial Sequence
  Primer
ttaaagcagcagttgatcgtgctgttgcatctggtgtcgt

SEQ ID NO: 159 - DNA, 40 bp, Artificial Sequence
  Primer
agatgcaacagcacgatcaactgctgctttaagtgccgca

SEQ ID NO: 160 - DNA, 40 bp, Artificial Sequence
  Primer
aaacccgtttcaagattctaattctcatggcacacacgtc

SEQ ID NO: 161 - DNA, 40 bp, Artificial Sequence
  Primer
tgtgccatgagaattagaatcttgaaacgggtttgtttcg

SEQ ID NO: 162 - DNA, 40 bp, Artificial Sequence
  Primer
aaacccgtttcaagatgataattctcatggcacacacgtc

SEQ ID NO: 163 - DNA, 40 bp, Artificial Sequence
  Primer
tgtgccatgagaattatcatcttgaaacgggtttgtttcg

SEQ ID NO: 164 - DNA, 39 bp, Artificial Sequence
  Primer
aagcggcagtgcgacacttaaagcagcagttgataaagc

SEQ ID NO: 165 - DNA, 40 bp, Artificial Sequence
  Primer
tcaactgctgctttaagtgtcgcactgccgcttggtgctc

SEQ ID NO: 166 - DNA, 37 bp, Artificial Sequence
  Primer
caagcggcagtgttgcacttaaagcagcagttgataa

SEQ ID NO: 167 - DNA, 40 bp, Artificial Sequence
  Primer
actgctgctttaagtgcaacactgccgcttggtgctccca

SEQ ID NO: 168 - protein, 382 aa, Bacillus Amyloliquefaciens
VRSKKLWISLLFALALIFTMAFGSTSSAQAAGKSNGEKKYIVGFKQTMSTMSAAKKKDVISEKGGKVQKQFKYVDAASATLNEKAVKELKKDPSVAYVEEDHVAHAYAQSVPYGVSQIKAPALHSQGYTGSNVKVAVIDSGIDSSHPDLKVAGGASMVPSETNPFQDNNSHGTHVAGTVAALNNSIGVLGVAPSASLYAVKVLGADGSGQYSWIINGIEWAIANNMDVINMSLGGPSGSAALKAAVDKAVASGVVVVAAAGNEGTSGSSSTVGYPGKYPSVIAVGAVDSSNQRASFSSVGPELDVMAPGVSIQSTLPGNKYGAYNGTSMASPHVAGAAALILSKHPNWTNTQVRSSLENTTTKLGDSFYYGKGLINVQAAAQ

SEQ ID NO: 169 - DNA, 36 bp, Artificial Sequence
  Primer
cggcgttaaacaataacattggcgtgcttggtgtag

SEQ ID NO: 170 - DNA, 37 bp, Artificial Sequence
  Primer
accaagcacgccaatgttattgtttaacgccgcaacc

SEQ ID NO: 171 - DNA, 39 bp, Artificial Sequence
  Primer
gtatcgactcgagccatgaagatcttaaagtcgctggag

SEQ ID NO: 172 - DNA, 38 bp, Artificial Sequence
  Primer
cagcgactttaagatcttcatggctcgagtcgataccg

SEQ ID NO: 173 - DNA, 39 bp, Artificial Sequence
  Primer
ttggtgtagccccggatgcttcgctctacgccgttaaag

SEQ ID NO: 174 - DNA, 35 bp, Artificial Sequence
  Primer
cgtagagcgaagcatccggggctacaccaagcacg

SEQ ID NO: 175 - DNA, 39 bp, Artificial Sequence
  Primer
gaacggttgcggcgttagataattctattggcgtgcttg

SEQ ID NO: 176 - DNA, 37 bp, Artificial Sequence
  Primer
agcacgccaatagaattatctaacgccgcaaccgttc

SEQ ID NO: 177 - DNA, 44 bp, Artificial Sequence
  Primer
aacggttgcggcgttagataataacattggcgtgcttggtgtag

SEQ ID NO: 178 - DNA, 46 bp, Artificial Sequence
  Primer
acaccaagcacgccaatgttattatctaacgccgcaaccgttcctg

SEQ ID NO: 179 - DNA, 31 bp, Artificial Sequence
  Primer
cggcgttaaacaataatattggcgtgcttgg

SEQ ID NO: 180 - DNA, 31 bp, Artificial Sequence
  Primer
ccaagcacgccaatattattgtttaacgccg

SEQ ID NO: 181 - DNA, 28 bp, Artificial Sequence
  Primer
ggtgtagccccggatgcttcgctctacg

SEQ ID NO: 182 - DNA, 28 bp, Artificial Sequence
  Primer
cgtagagcgaagcatccggggctacacc

SEQ ID NO: 183 - DNA, 30 bp, Artificial Sequence
  Primer
gtatcgactcgagccatgaagatcttaaag

SEQ ID NO: 184 - DNA, 30 bp, Artificial Sequence
  Primer
ctttaagatcttcatggctcgagtcgatac

SEQ ID NO: 185 - DNA, 28 bp, Artificial Sequence
  Primer
cgcttccagggaacaactatggtgcgta

SEQ ID NO: 186 - DNA, 28 bp, Artificial Sequence
  Primer
tacgcaccatagttgttccctggaagcg

SEQ ID NO: 187 - DNA, 31 bp, Artificial Sequence
  Primer
cactctcaaggctacgttggatcaaatgtta

SEQ ID NO: 188 - DNA, 31 bp, Artificial Sequence
  Primer
taacatttgatccaacgtagccttgagagtg

SEQ ID NO: 189 - DNA, 29 bp, Artificial Sequence
  Primer
tggcgtttctattgaatcgacgcttccag

SEQ ID NO: 190 - DNA, 29 bp, Artificial Sequence
  Primer
ctggaagcgtcgattcaatagaaacgcca

SEQ ID NO: 191 - DNA, 39 bp, Artificial Sequence; identical to SEQ ID NO: 175
  Primer

SEQ ID NO: 192 - DNA, 37 bp, Artificial Sequence; identical to SEQ ID NO: 176
  Primer

SEQ ID NO: 193 - DNA, 39 bp, Artificial Sequence; identical to SEQ ID NO: 173
  Primer

SEQ ID NO: 194 - DNA, 35 bp, Artificial Sequence; identical to SEQ ID NO: 174
  Primer

SEQ ID NO: 195 - DNA, 35 bp, Artificial Sequence
  Primer
gcagcagacggatcagcacaatactcatggattat

SEQ ID NO: 196 - DNA, 35 bp, Artificial Sequence
  Primer
ataatccatgagtattgtgctgatccgtctgctgc

SEQ ID NO: 197 - DNA, 45 bp, Artificial Sequence
  Primer
caacatgagcctgggagcaccaccgggcagtgcggcacttaaagc

SEQ ID NO: 198 - DNA, 45 bp, Artificial Sequence
  Primer
gctttaagtgccgcactgcccggtggtgctcccaggctcatgttg

SEQ ID NO: 199 - DNA, 39 bp, Artificial Sequence
  Primer
gttcttgcagcagacggaaatggccaatactcatggatt

SEQ ID NO: 200 - DNA, 39 bp, Artificial Sequence
  Primer
aatccatgagtattggccatttccgtctgctgcaagaac

SEQ ID NO: 201 - DNA, 42 bp, Artificial Sequence
  Primer
ttaaagttcttgcagcagacaattcaggccaatactcatgga

SEQ ID NO: 202 - DNA, 42 bp, Artificial Sequence
  Primer
tccatgagtattggcctgaattgtctgctgcaagaactttaa

SEQ ID NO: 203 - DNA, 36 bp, Artificial Sequence
  Primer
ccgtttcaagatccgaattctcatggcacacacgtc

SEQ ID NO: 204 - DNA, 38 bp, Artificial Sequence
  Primer
tgccatgagaattcggatcttgaaacgggtttgtttcg

SEQ ID NO: 205 - DNA, 40 bp, Artificial Sequence
  Primer
ttcaaatcaacgtgattctttttcctccgtgggaccggag

SEQ ID NO: 206 - DNA, 40 bp, Artificial Sequence
  Primer
acggaggaaaaagaatcacgttgatttgaagagtctacag

SEQ ID NO: 207 - DNA, 38 bp, Artificial Sequence
  Primer
caaatcaacgtgcctctgattcctccgtgggaccggag

SEQ ID NO: 208 - DNA, 38 bp, Artificial Sequence
  Primer
ctccggtcccacggaggaatcagaggcacgttgatttg

SEQ ID NO: 209 - DNA, 44 bp, Artificial Sequence
  Primer
agcggcagtgcggcacttaaagttgcagttgataaagctgttgc

SEQ ID NO: 210 - DNA, 44 bp, Artificial Sequence
  Primer
gcaacagctttatcaactgcaactttaagtgccgcactgccgct

SEQ ID NO: 211 - DNA, 39 bp, Artificial Sequence
  Primer
tcaagataacaatacacatggcacacacgtcgcaggaac

SEQ ID NO: 212 - DNA, 40 bp, Artificial Sequence
  Primer
acgtgtgtgccatgtgtattgttatcttgaaacgggtttg

SEQ ID NO: 213 - DNA, 40 bp, Artificial Sequence
  Primer
agacggatcaggcaattactcatggattatcaacggcatc

SEQ ID NO: 214 - DNA, 37 bp, Artificial Sequence
  Primer
taatccatgagtaattgcctgatccgtctgctgcaag

SEQ ID NO: 215 - DNA, 38 bp, Artificial Sequence
  Primer
acccgtttcaagataacgattctcatggcacacacgtc

SEQ ID NO: 216 - DNA, 38 bp, Artificial Sequence
  Primer
gacgtgtgtgccatgagaatcgttatcttgaaacgggt

SEQ ID NO: 217 - DNA, 37 bp, Artificial Sequence
  Primer
caatactcatggattatcgatggcatcgaatgggcca

SEQ ID NO: 218 - DNA, 37 bp, Artificial Sequence
  Primer
tggcccattcgatgccatcgataatccatgagtattg

SEQ ID NO: 219 - DNA, 39 bp, Artificial Sequence
  Primer
ctcttcaaatcaacgtgccgatttttcctccgtgggacc

SEQ ID NO: 220 - DNA, 39 bp, Artificial Sequence
  Primer
ggtcccacggaggaaaaatcggcacgttgatttgaagag

SEQ ID NO: 221 - DNA, 37 bp, Artificial Sequence
  Primer
caaacactcaagtccgcagaagtttagaaaacaccac

SEQ ID NO: 222 - DNA, 38 bp, Artificial Sequence
  Primer
gtgcttggtgtagccccgagagcttcgctctacgccgt

SEQ ID NO: 223 - DNA, 38 bp, Artificial Sequence
  Primer
acggcgtagagcgaagctctcggggctacaccaagcac

SEQ ID NO: 224 - DNA, 37 bp, Artificial Sequence
  Primer
caaacactcaagtccgcgatagtttagaaaacaccac

SEQ ID NO: 225 - DNA, 37 bp, Artificial Sequence
  Primer
gtggtgttttctaaactatcgcggacttgagtgtttg

SEQ ID NO: 226 - DNA, 38 bp, Artificial Sequence
  Primer
gtgcttggtgtagccccgtctgcttcgctctacgccgt

SEQ ID NO: 227 - DNA, 38 bp, Artificial Sequence
  Primer
acggcgtagagcgaagcagacggggctacaccaagcac

SEQ ID NO: 228 - DNA, 37 bp, Artificial Sequence
  Primer
caatactcatggattatcaacggcatcgaatgggcca

SEQ ID NO: 229 - DNA, 37 bp, Artificial Sequence
  Primer
tggcccattcgatgccgttgataatccatgagtattg

SEQ ID NO: 230 - DNA, 37 bp, Artificial Sequence
  Primer
actcatggattatcgatggcatcgaatgggccatcgc

SEQ ID NO: 231 - DNA, 36 bp, Artificial Sequence
  Primer
cactcaagtccgcagaagtttagaaaacaccactac

SEQ ID NO: 232 - DNA, 36 bp, Artificial Sequence
  Primer
cactcaagtccgcgatagtttagaaaacaccactac

SEQ ID NO: 233 - DNA, 38 bp, Artificial Sequence
  Primer
caaatcaacgtgccagattttcctccgtgggaccggag

SEQ ID NO: 234 - DNA, 24 bp, Artificial Sequence
  Primer
aaaggggaggaaaatcgtgaaaca

SEQ ID NO: 235 - DNA, 22 bp, Artificial Sequence
  Primer
gttctaaatcgtgtttttcttg

SEQ ID NO: 236 - DNA, 48 bp, Artificial Sequence
  Primer
gaactggacaaacactcaagtccgcgatagtttagaaaacaccactac

SEQ ID NO: 237 - DNA, 36 bp, Artificial Sequence
  Primer
gacttgagtgtttgtccagttcgggtgcttagaaag

SEQ ID NO: 238 - DNA, 37 bp, Artificial Sequence
  Primer
caaacactcaagtccgcagcagtttagaaaacaccac

SEQ ID NO: 239 - DNA, 37 bp, Artificial Sequence
  Primer
gtggtgttttctaaactgctgcggacttgagtgtttg

SEQ ID NO: 240 - DNA, 49 bp, Artificial Sequence
  Primer
acgccgttaaagttcttgcagcagacgaatcaggccaatactcatggat

SEQ ID NO: 241 - DNA, 36 bp, Artificial Sequence
  Primer
tgctgcaagaactttaacggcgtagagcgaagcaga

SEQ ID NO: 242 - DNA, 37 bp, Artificial Sequence
  Primer
acatggatgtaatctgcatgagcctgggaggaccaag

SEQ ID NO: 243 - DNA, 38 bp, Artificial Sequence
  Primer
tcctcccaggctcatgcagattacatccatgttattcg

SEQ ID NO: 244 - DNA, 22 bp, Artificial Sequence
  Primer
gttatgagttagttcaaattcg

SEQ ID NO: 245 - DNA, 46 bp, Artificial Sequence
  Primer
  misc_feature (16)..(17): n is a, c, g, or t
  misc_feature (19)..(20): n is a, c, g, or t
  misc_feature (22)..(23): n is a, c, g, or t
tacgcgcagtccgtgnntnncnncgtatcacaaattaaagcccctg

SEQ ID NO: 246 - DNA, 44 bp, Artificial Sequence
  Primer
  misc_feature (17)..(18): n is a, c, g, or t
  misc_feature (20)..(21): n is a, c, g, or t
  misc_feature (23)..(24): n is a, c, g, or t
tttaatttgtgatacgnngnnanncacggactgcgcgtacgcat

SEQ ID NO: 247 - DNA, 43 bp, Artificial Sequence
  Primer
  misc_feature (16)..(17): n is a, c, g, or t
  misc_feature (19)..(20): n is a, c, g, or t
  misc_feature (22)..(23): n is a, c, g, or t
tacggcgtatcacaanntnnannccctgctctgcactctcaag

SEQ ID NO: 248 - DNA, 45 bp, Artificial Sequence
  Primer
  misc_feature (17)..(18): n is a, c, g, or t
  misc_feature (20)..(21): n is a, c, g, or t
  misc_feature (23)..(24): n is a, c, g, or t
agagtgcagagcagggnntnnannttgtgatacgccgtaaggcac

SEQ ID NO: 249 - DNA, 47 bp, Artificial Sequence
  Primer
  misc_feature (16)..(17): n is a, c, g, or t
  misc_feature (19)..(20): n is a, c, g, or t
  misc_feature (22)..(23): n is a, c, g, or t
gctctgcactctcaanncnncnntggatcaaatgttaaagtagcggt

SEQ ID NO: 250 - DNA, 47 bp, Artificial Sequence
  Primer
  misc_feature (17)..(18): n is a, c, g, or t
  misc_feature (20)..(21): n is a, c, g, or t
  misc_feature (23)..(24): n is a, c, g, or t
tttaacatttgatccanngnngnnttgagagtgcagagcaggggctt

SEQ ID NO: 251 - DNA, 48 bp, Artificial Sequence
  Primer
  misc_feature (16)..(17): n is a, c, g, or t
  misc_feature (19)..(20): n is a, c, g, or t
  misc_feature (22)..(23): n is a, c, g, or t
ctgcactctcaaggcnncnntnnatcaaatgttaaagtagcggttatc

SEQ ID NO: 252 - DNA, 44 bp, Artificial Sequence
  Primer
  misc_feature (17)..(18): n is a, c, g, or t
  misc_feature (20)..(21): n is a, c, g, or t
  misc_feature (23)..(24): n is a, c, g, or t
tactttaacatttgatnnanngnngccttgagagtgcagagcag

SEQ ID NO: 253 - DNA, 47 bp, Artificial Sequence
  Primer
  misc_feature (16)..(17): n is a, c, g, or t
  misc_feature (19)..(20): n is a, c, g, or t
  misc_feature (22)..(23): n is a, c, g, or t
cactctcaaggctacnntnnannaaatgttaaagtagcggttatcga

SEQ ID NO: 254 - DNA, 44 bp, Artificial Sequence
  Primer
  misc_feature (17)..(18): n is a, c, g, or t
  misc_feature (20)..(21): n is a, c, g, or t
  misc_feature (23)..(24): n is a, c, g, or t
cgctactttaacatttnntnnanngtagccttgagagtgcagag

SEQ ID NO: 255 - DNA, 46 bp, Artificial Sequence
  Primer
  misc_feature (16)..(17): n is a, c, g, or t
  misc_feature (19)..(20): n is a, c, g, or t
  misc_feature (22)..(23): n is a, c, g, or t
tctcaaggctacactnnannanntgttaaagtagcggttatcgaca

SEQ ID NO: 256 - DNA, 45 bp, Artificial Sequence
  Primer
  misc_feature (17)..(18): n is a, c, g, or t
  misc_feature (20)..(21): n is a, c, g, or t
  misc_feature (23)..(24): n is a, c, g, or t
aaccgctactttaacanntnntnnagtgtagccttgagagtgcag

SEQ ID NO: 257 - DNA, 45 bp, Artificial Sequence
  Primer
  misc_feature (16)..(17): n is a, c, g, or t
  misc_feature (19)..(20): n is a, c, g, or t
  misc_feature (22)..(23): n is a, c, g, or t
caaggctacactggannanntnntaaagtagcggttatcgacagc

SEQ ID NO: 258 - DNA, 45 bp, Artificial Sequence
  Primer
  misc_feature (17)..(18): n is a, c, g, or t
  misc_feature (20)..(21): n is a, c, g, or t
  misc_feature (23)..(24): n is a, c, g, or t
gataaccgctactttannanntnntccagtgtagccttgagagtg

SEQ ID NO: 259 - DNA, 45 bp, Artificial Sequence
  Primer
  misc_feature (16)..(17): n is a, c, g, or t
  misc_feature (19)..(20): n is a, c, g, or t
  misc_feature (22)..(23): n is a, c, g, or t
ggctacactggatcanntnntnnagtagcggttatcgacagcggt

SEQ ID NO: 260 - DNA, 45 bp, Artificial Sequence
  Primer
  misc_feature (17)..(18): n is a, c, g, or t
  misc_feature (20)..(21): n is a, c, g, or t
  misc_feature (23)..(24): n is a, c, g, or t
gtcgataaccgctactnnannanntgatccagtgtagccttgaga

SEQ ID NO: 261 - DNA, 44 bp, Artificial Sequence
  Primer
  misc_feature (16)..(17): n is a, c, g, or t
  misc_feature (19)..(20): n is a, c, g, or t
  misc_feature (22)..(23): n is a, c, g, or t
tacactggatcaaatnntnnannagcggttatcgacagcggtat

SEQ ID NO: 262 - DNA, 46 bp, Artificial Sequence
  Primer
  misc_feature (17)..(18): n is a, c, g, or t
  misc_feature (20)..(21): n is a, c, g, or t
  misc_feature (23)..(24): n is a, c, g, or t
gctgtcgataaccgctnntnnannatttgatccagtgtagccttga

SEQ ID NO: 263 - DNA, 45 bp, Artificial Sequence
  Primer
  misc_feature (16)..(17): n is a, c, g, or t
  misc_feature (19)..(20): n is a, c, g, or t
  misc_feature (22)..(23): n is a, c, g, or t
actggatcaaatgttnnannannggttatcgacagcggtatcgac

SEQ ID NO: 264 - DNA, 46 bp, Artificial Sequence
  Primer
  misc_feature (17)..(18): n is a, c, g, or t
  misc_feature (20)..(21): n is a, c, g, or t
  misc_feature (23)..(24): n is a, c, g, or t
accgctgtcgataaccnntnntnnaacatttgatccagtgtagcct

SEQ ID NO: 265 - DNA, 44 bp, Artificial Sequence
  Primer
  misc_feature (16)..(17): n is a, c, g, or t
  misc_feature (19)..(20): n is a, c, g, or t
  misc_feature (22)..(23): n is a, c, g, or t
ggatcaaatgttaaannanngnntatcgacagcggtatcgactc

SEQ ID NO: 266 - DNA, 47 bp, Artificial Sequence
  Primer
  misc_feature (17)..(18): n is a, c, g, or t
  misc_feature (20)..(21): n is a, c, g, or t
  misc_feature (23)..(24): n is a, c, g, or t
gataccgctgtcgatanncnntnntttaacatttgatccagtgtagc

SEQ ID NO: 267 - DNA, 48 bp, Artificial Sequence
  Primer
  misc_feature (16)..(17): n is a, c, g, or t
  misc_feature (19)..(20): n is a, c, g, or t
  misc_feature (22)..(23): n is a, c, g, or t
tcaaatgttaaagtanngnntnncgacagcggtatcgactcgagccat

SEQ ID NO: 268 - DNA, 48 bp, Artificial Sequence
  Primer
  misc_feature (17)..(18): n is a, c, g, or t
  misc_feature (20)..(21): n is a, c, g, or t
  misc_feature (23)..(24): n is a, c, g, or t
gtcgataccgctgtcgnnanncnntactttaacatttgatccagtgta

SEQ ID NO: 269 - DNA, 45 bp, Artificial Sequence
  Primer
  misc_feature (16)..(17): n is a, c, g, or t
  misc_feature (19)..(20): n is a, c, g, or t
  misc_feature (22)..(23): n is a, c, g, or t
aatgttaaagtagcgnntnncnncagcggtatcgactcgagccat

SEQ ID NO: 270 - DNA, 47 bp, Artificial Sequence
  Primer
  misc_feature (17)..(18): n is a, c, g, or t
  misc_feature (20)..(21): n is a, c, g, or t
  misc_feature (23)..(24): n is a, c, g, or t
cgagtcgataccgctgnngnnanncgctactttaacatttgatccag

SEQ ID NO: 271 - DNA, 45 bp, Artificial Sequence
  Primer
  misc_feature (16)..(17): n is a, c, g, or t
  misc_feature (19)..(20): n is a, c, g, or t
  misc_feature (22)..(23): n is a, c, g, or t
gttaaagtagcggttnncnncnncggtatcgactcgagccatcca

SEQ ID NO: 272 - DNA, 47 bp, Artificial Sequence
  Primer
  misc_feature (17)..(18): n is a, c, g, or t
  misc_feature (20)..(21): n is a, c, g, or t
  misc_feature (23)..(24): n is a, c, g, or t
gctcgagtcgataccgnngnngnnaaccgctactttaacatttgatc

SEQ ID NO: 273 - DNA, 45 bp, Artificial Sequence
  Primer
  misc_feature (16)..(17): n is a, c, g, or t
  misc_feature (19)..(20): n is a, c, g, or t
  misc_feature (22)..(23): n is a, c, g, or t
aaagtagcggttatcnncnncnntatcgactcgagccatccagat

SEQ ID NO: 274 - DNA, 47 bp, Artificial Sequence
  Primer
  misc_feature (17)..(18): n is a, c, g, or t
  misc_feature (20)..(21): n is a, c, g, or t
  misc_feature (23)..(24): n is a, c, g, or t
atggctcgagtcgatanngnngnngataaccgctactttaacatttg

SEQ ID NO: 275 - DNA, 44 bp, Artificial Sequence
  Primer
  misc_feature (16)..(17): n is a, c, g, or t
  misc_feature (19)..(20): n is a, c, g, or t
  misc_feature (22)..(23): n is a, c, g, or t
gtagcggttatcgacnncnntnncgactcgagccatccagatct

SEQ ID NO: 276 - DNA, 46 bp, Artificial Sequence
  Primer
  misc_feature (17)..(18): n is a, c, g, or t
  misc_feature (20)..(21): n is a, c, g, or t
  misc_feature (23)..(24): n is a, c, g, or t
tggatggctcgagtcgnnanngnngtcgataaccgctactttaaca

SEQ ID NO: 277 - DNA, 46 bp, Artificial Sequence
  Primer
  misc_feature (16)..(17): n is a, c, g, or t
  misc_feature (19)..(20): n is a, c, g, or t
  misc_feature (22)..(23): n is a, c, g, or t
gcggttatcgacagcnntnncnnctcgagccatccagatcttaaag

SEQ ID NO: 278 - DNA, 45 bp, Artificial Sequence
  Primer
  misc_feature (17)..(18): n is a, c, g, or t
  misc_feature (20)..(21): n is a, c, g, or t
  misc_feature (23)..(24): n is a, c, g, or t
atctggatggctcgagnngnnanngctgtcgataaccgctacttt

SEQ ID NO: 279 - DNA, 45 bp, Artificial Sequence
  Primer
  misc_feature (16)..(17): n is a, c, g, or t
  misc_feature (19)..(20): n is a, c, g, or t
  misc_feature (22)..(23): n is a, c, g, or t
gttatcgacagcggtnncnncnngagccatccagatcttaaagtc

SEQ ID NO: 280 - DNA, 44 bp, Artificial Sequence
  Primer
  misc_feature (17)..(18): n is a, c, g, or t
  misc_feature (20)..(21): n is a, c, g, or t
  misc_feature (23)..(24): n is a, c, g, or t
aagatctggatggctcnngnngnnaccgctgtcgataaccgcta

SEQ ID NO: 281 - DNA, 46 bp, Artificial Sequence
  Primer
  misc_feature (16)..(17): n is a, c, g, or t
  misc_feature (19)..(20): n is a, c, g, or t
  misc_feature (22)..(23): n is a, c, g, or t
atcgacagcggtatcnncnngnnccatccagatcttaaagtcgctg

SEQ ID NO: 282 - DNA, 47 bp, Artificial Sequence
  Primer
  misc_feature (17)..(18): n is a, c, g, or t
  misc_feature (20)..(21): n is a, c, g, or t
  misc_feature (23)..(24): n is a, c, g, or t
tttaagatctggatggnncnngnngataccgctgtcgataaccgcta

SEQ ID NO: 283 - DNA, 45 bp, Artificial Sequence
  Primer
  misc_feature (16)..(17): n is a, c, g, or t
  misc_feature (19)..(20): n is a, c, g, or t
  misc_feature (22)..(23): n is a, c, g, or t
gacagcggtatcgacnngnncnntccagatcttaaagtcgctgga

SEQ ID NO: 284 - DNA, 45 bp, Artificial Sequence
  Primer
  misc_feature (17)..(18): n is a, c, g, or t
  misc_feature (20)..(21): n is a, c, g, or t
  misc_feature (23)..(24): n is a, c, g, or t
gactttaagatctgganngnncnngtcgataccgctgtcgataac

SEQ ID NO: 285 - DNA, 44 bp, Artificial Sequence
  Primer
  misc_feature (16)..(17): n is a, c, g, or t
  misc_feature (19)..(20): n is a, c, g, or t
  misc_feature (22)..(23): n is a, c, g, or t
agcggtatcgactcgnncnntnnagatcttaaagtcgctggagg

SEQ ID NO: 286 - DNA, 44 bp, Artificial Sequence
  Primer
  misc_feature (17)..(18): n is a, c, g, or t
  misc_feature (20)..(21): n is a, c, g, or t
  misc_feature (23)..(24): n is a, c, g, or t
agcgactttaagatctnnanngnncgagtcgataccgctgtcga

SEQ ID NO: 287 - DNA, 44 bp, Artificial Sequence
  Primer
  misc_feature (16)..(17): n is a, c, g, or t
  misc_feature (19)..(20): n is a, c, g, or t
  misc_feature (22)..(23): n is a, c, g, or t
gactcgagccatccanntnntnnagtcgctggaggggcttctat

SEQ ID NO: 288 - DNA, 44 bp, Artificial Sequence
  Primer
  misc_feature (17)..(18): n is a, c, g, or t
  misc_feature (20)..(21): n is a, c, g, or t
  misc_feature (23)..(24): n is a, c, g, or t
agcccctccagcgactnnannanntggatggctcgagtcgatac

SEQ ID NO: 289 - DNA, 46 bp, Artificial Sequence
  Primer
  misc_feature (16)..(17): n is a, c, g, or t
  misc_feature (19)..(20): n is a, c, g, or t
  misc_feature (22)..(23): n is a, c, g, or t
agccatccagatcttnnanncnntggaggggcttctatggtgccgt

SEQ ID NO: 290 - DNA, 47 bp, Artificial Sequence
  Primer
  misc_feature (16)..(16): n is a, c, g, or t
  misc_feature (26)..(26): n is a, c, g, or t
catagaagcccctccnagcgactttnaagatctggatggctcgagtc

SEQ ID NO: 291 - DNA, 43 bp, Artificial Sequence
  Primer
  misc_feature (16)..(17): n is a, c, g, or t
  misc_feature (19)..(20): n is a, c, g, or t
  misc_feature (22)..(23): n is a, c, g, or t
catccagatcttaaanncnntnnaggggcttctatggtgccgt

SEQ ID NO: 292 - DNA, 46 bp, Artificial Sequence
  Primer
  misc_feature (17)..(18): n is a, c, g, or t
  misc_feature (20)..(21): n is a, c, g, or t
  misc_feature (23)..(24): n is a, c, g, or t
caccatagaagcccctnnanngnntttaagatctggatggctcgag

SEQ ID NO: 293 - DNA, 47 bp, Artificial Sequence
  Primer
  misc_feature (16)..(17): n is a, c, g, or t
  misc_feature (19)..(20): n is a, c, g, or t
  misc_feature (22)..(23): n is a, c, g, or t
ggaggggcttctatgnngnngnncgaaacaaacccgtttcaagataa

SEQ ID NO: 294 - DNA, 44 bp, Artificial Sequence
  Primer
  misc_feature (17)..(18): n is a, c, g, or t
  misc_feature (20)..(21): n is a, c, g, or t
  misc_feature (23)..(24): n is a, c, g, or t
aaacgggtttgtttcgnncnncnncatagaagcccctccagcga

SEQ ID NO: 295 - DNA, 47 bp, Artificial Sequence
  Primer
  misc_feature (16)..(17): n is a, c, g, or t
  misc_feature (19)..(20): n is a, c, g, or t
  misc_feature (22)..(23): n is a, c, g, or t
ggggcttctatggtgnngnncnnaacaaacccgtttcaagataacaa

SEQ ID NO: 296 - DNA, 44 bp, Artificial Sequence
  Primer
  misc_feature (17)..(18): n is a, c, g, or t
  misc_feature (20)..(21): n is a, c, g, or t
  misc_feature (23)..(24): n is a, c, g, or t
ttgaaacgggtttgttnngnncnncaccatagaagcccctccag

SEQ ID NO: 297 - DNA, 47 bp, Artificial Sequence
  Primer
  misc_feature (16)..(17): n is a, c, g, or t
  misc_feature (19)..(20): n is a, c, g, or t
  misc_feature (22)..(23): n is a, c, g, or t
gcttctatggtgccgnncnnannaaacccgtttcaagataacaattc

SEQ ID NO: 298 - DNA, 44 bp, Artificial Sequence
  Primer
  misc_feature (17)..(18): n is a, c, g, or t
  misc_feature (20)..(21): n is a, c, g, or t
  misc_feature (23)..(24): n is a, c, g, or t
atcttgaaacgggtttnntnngnncggcaccatagaagcccctc

SEQ ID NO: 299 - DNA, 47 bp, Artificial Sequence
  Primer
  misc_feature (16)..(17): n is a, c, g, or t
  misc_feature (19)..(20): n is a, c, g, or t
  misc_feature (22)..(23): n is a, c, g, or t
tctatggtgccgtccnnannanncccgtttcaagataacaattctca

SEQ ID NO: 300 - DNA, 46 bp, Artificial Sequence
  Primer
  misc_feature (17)..(18): n is a, c, g, or t
  misc_feature (20)..(21): n is a, c, g, or t
  misc_feature (23)..(24): n is a, c, g, or t
gttatcttgaaacgggnntnntnnggacggcaccatagaagcccct

SEQ ID NO: 301 - DNA, 47 bp, Artificial Sequence
  Primer
  misc_feature (16)..(17): n is a, c, g, or t
  misc_feature (19)..(20): n is a, c, g, or t
  misc_feature (22)..(23): n is a, c, g, or t
atggtgccgtccgaannanncnngtttcaagataacaattctcatgg

SEQ ID NO: 302 - DNA, 44 bp, Artificial Sequence
  Primer
  misc_feature (17)..(18): n is a, c, g, or t
  misc_feature (20)..(21): n is a, c, g, or t
  misc_feature (23)..(24): n is a, c, g, or t
attgttatcttgaaacnngnntnnttcggacggcaccatagaag

SEQ ID NO: 303 - DNA, 47 bp, Artificial Sequence
  Primer
  misc_feature (16)..(17): n is a, c, g, or t
  misc_feature (19)..(20): n is a, c, g, or t
  misc_feature (22)..(23): n is a, c, g, or t
gtgccgtccgaaacanncnngnntcaagataacaattctcatggcac

SEQ ID NO: 304 - DNA, 45 bp, Artificial Sequence
  Primer
  misc_feature (17)..(18): n is a, c, g, or t
  misc_feature (20)..(21): n is a, c, g, or t
  misc_feature (23)..(24): n is a, c, g, or t
agaattgttatcttganncnngnntgtttcggacggcaccataga

SEQ ID NO: 305 - DNA, 46 bp, Artificial Sequence
  Primer
  misc_feature (16)..(17): n is a, c, g, or t
  misc_feature (19)..(20): n is a, c, g, or t
  misc_feature (22)..(23): n is a, c, g, or t
ccgtccgaaacaaacnngnntnnagataacaattctcatggcacac

SEQ ID NO: 306 - DNA, 44 bp, Artificial Sequence
  Primer
  misc_feature (17)..(18): n is a, c, g, or t
  misc_feature (20)..(21): n is a, c, g, or t
  misc_feature (23)..(24): n is a, c, g, or t
atgagaattgttatctnnanncnngtttgtttcggacggcacca

SEQ ID NO: 307 - DNA, 45 bp, Artificial Sequence
  Primer
  misc_feature (16)..(17): n is a, c, g, or t
  misc_feature (19)..(20): n is a, c, g, or t
  misc_feature (22)..(23): n is a, c, g, or t
tccgaaacaaacccgnntnnanntaacaattctcatggcacacac

SEQ ID NO: 308 - DNA, 44 bp, Artificial Sequence
  Primer
  misc_feature (17)..(18): n is a, c, g, or t
  misc_feature (20)..(21): n is a, c, g, or t
  misc_feature (23)..(24): n is a, c, g, or t
gccatgagaattgttanntnnanncgggtttgtttcggacggca

SEQ ID NO: 309 - DNA, 45 bp, Artificial Sequence
  Primer
  misc_feature (16)..(17): n is a, c, g, or t
  misc_feature (19)..(20): n is a, c, g, or t
  misc_feature (22)..(23): n is a, c, g, or t
gaaacaaacccgtttnnanntnncaattctcatggcacacacgtc

SEQ ID NO: 310 - DNA, 44 bp, Artificial Sequence
  Primer
  misc_feature (17)..(18): n is a, c, g, or t
  misc_feature (20)..(21): n is a, c, g, or t
  misc_feature (23)..(24): n is a, c, g, or t
tgtgccatgagaattgnnanntnnaaacgggtttgtttcggacg

SEQ ID NO: 311 - DNA, 43 bp, Artificial Sequence
  Primer
  misc_feature (16)..(17): n is a, c, g, or t
  misc_feature (19)..(20): n is a, c, g, or t
  misc_feature (22)..(23): n is a, c, g, or t
acaaacccgtttcaanntnncnnttctcatggcacacacgtcg

SEQ ID NO: 312 - DNA, 46 bp, Artificial Sequence
  Primer
  misc_feature (17)..(18): n is a, c, g, or t
  misc_feature (20)..(21): n is a, c, g, or t
  misc_feature (23)..(24): n is a, c, g, or t
gtgtgtgccatgagaanngnnannttgaaacgggtttgtttcggac

SEQ ID NO: 313 - DNA, 43 bp, Artificial Sequence
  Primer
  misc_feature (16)..(17): n is a, c, g, or t
  misc_feature (19)..(20): n is a, c, g, or t
  misc_feature (22)..(23): n is a, c, g, or t
aacccgtttcaagatnncnntnntcatggcacacacgtcgcag

SEQ ID NO: 314 - DNA, 46 bp, Artificial Sequence
  Primer
  misc_feature (17)..(18): n is a, c, g, or t
  misc_feature (20)..(21): n is a, c, g, or t
  misc_feature (23)..(24): n is a, c, g, or t
gacgtgtgtgccatgannanngnnatcttgaaacgggtttgtttcg

SEQ ID NO: 315 - DNA, 43 bp, Artificial Sequence
  Primer
  misc_feature (16)..(17): n is a, c, g, or t
  misc_feature (19)..(20): n is a, c, g, or t
  misc_feature (22)..(23): n is a, c, g, or t
ccgtttcaagataacnntnntnntggcacacacgtcgcaggaa

SEQ ID NO: 316 - DNA, 47 bp, Artificial Sequence
  Primer
  misc_feature (17)..(18): n is a, c, g, or t
  misc_feature (20)..(21): n is a, c, g, or t
  misc_feature (23)..(24): n is a, c, g, or t
tgcgacgtgtgtgccannannanngttatcttgaaacgggtttgttt

SEQ ID NO: 317 - DNA, 44 bp, Artificial Sequence
  Primer
  misc_feature (16)..(17): n is a, c, g, or t
  misc_feature (19)..(20): n is a, c, g, or t
  misc_feature (22)..(23): n is a, c, g, or t
aattctcatggcacanncnncnnaggaacggttgcggcgttaaa

SEQ ID NO: 318 - DNA, 47 bp, Artificial Sequence
  Primer
  misc_feature (17)..(18): n is a, c, g, or t
  misc_feature (20)..(21): n is a, c, g, or t
  misc_feature (23)..(24): n is a, c, g, or t
cgccgcaaccgttcctnngnngnntgtgccatgagaattgttatctt

SEQ ID NO: 319 - DNA, 45 bp, Artificial Sequence
  Primer
  misc_feature (16)..(17): n is a, c, g, or t
  misc_feature (19)..(20): n is a, c, g, or t
  misc_feature (22)..(23): n is a, c, g, or t
tctcatggcacacacnncnnannaacggttgcggcgttaaacaat

SEQ ID NO: 320 - DNA, 46 bp, Artificial Sequence
  Primer
  misc_feature (17)..(18): n is a, c, g, or t
  misc_feature (20)..(21): n is a, c, g, or t
  misc_feature (23)..(24): n is a, c, g, or t
taacgccgcaaccgttnntnngnngtgtgtgccatgagaattgtta

SEQ ID NO: 321 - DNA, 47 bp, Artificial Sequence
  Primer
  misc_feature (16)..(17): n is a, c, g, or t
  misc_feature (19)..(20): n is a, c, g, or t
  misc_feature (22)..(23): n is a, c, g, or t
acacacgtcgcagganngnntnnggcgttaaacaattctattggcgt

SEQ ID NO: 322 - DNA, 44 bp, Artificial Sequence
  Primer
  misc_feature (17)..(18): n is a, c, g, or t
  misc_feature (20)..(21): n is a, c, g, or t
  misc_feature (23)..(24): n is a, c, g, or t
agaattgtttaacgccnnanncnntcctgcgacgtgtgtgccat

SEQ ID NO: 323 - DNA, 46 bp, Artificial Sequence
  Primer
  misc_feature (16)..(17): n is a, c, g, or t
  misc_feature (19)..(20): n is a, c, g, or t
  misc_feature (22)..(23): n is a, c, g, or t
gcaggaacggttgcgnngnnanncaattctattggcgtgcttggtg

SEQ ID NO: 324 - DNA, 44 bp, Artificial Sequence
  Primer
  misc_feature (17)..(18): n is a, c, g, or t
  misc_feature (20)..(21): n is a, c, g, or t
  misc_feature (23)..(24): n is a, c, g, or t
cacgccaatagaattgnntnncnncgcaaccgttcctgcgacgt

SEQ ID NO: 325 - DNA, 44 bp, Artificial Sequence
  Primer
  misc_feature (16)..(17): n is a, c, g, or t
  misc_feature (19)..(20): n is a, c, g, or t
  misc_feature (22)..(23): n is a, c, g, or t
acggttgcggcgttanncnntnntattggcgtgcttggtgtagc

SEQ ID NO: 326 - DNA, 44 bp, Artificial Sequence
  Primer
  misc_feature (17)..(18): n is a, c, g, or t
  misc_feature (20)..(21): n is a, c, g, or t
  misc_feature (23)..(24): n is a, c, g, or t
accaagcacgccaatannanngnntaacgccgcaaccgttcctg

SEQ ID NO: 327 - DNA, 44 bp, Artificial Sequence
  Primer
  misc_feature (16)..(17): n is a, c, g, or t
  misc_feature (19)..(20): n is a, c, g, or t
  misc_feature (22)..(23): n is a, c, g, or t
aacaattctattggcnngnntnntgtagccccgtctgcttcgct

SEQ ID NO: 328 - DNA, 50 bp, Artificial Sequence
  Primer
  misc_feature (17)..(18): n is a, c, g, or t
  misc_feature (20)..(21): n is a, c, g, or t
  misc_feature (23)..(24): n is a, c, g, or t
agcagacggggctacannanncnngccaatagaattgtttaacgccgcaa

SEQ ID NO: 329 - DNA, 43 bp, Artificial Sequence
  Primer
  misc_feature (16)..(17): n is a, c, g, or t
  misc_feature (19)..(20): n is a, c, g, or t
  misc_feature (22)..(23): n is a, c, g, or t
tctattggcgtgcttnntnnanncccgtctgcttcgctctacg

SEQ ID NO: 330 - DNA, 47 bp, Artificial Sequence
  Primer
  misc_feature (17)..(18): n is a, c, g, or t
  misc_feature (20)..(21): n is a, c, g, or t
  misc_feature (23)..(24): n is a, c, g, or t
gagcgaagcagacgggnntnnannaagcacgccaatagaattgttta

SEQ ID NO: 331 - DNA, 44 bp, Artificial Sequence
  Primer
  misc_feature (16)..(17): n is a, c, g, or t
  misc_feature (19)..(20): n is a, c, g, or t
  misc_feature (22)..(23): n is a, c, g, or t
attggcgtgcttggtnnanncnngtctgcttcgctctacgccgt

SEQ ID NO: 332 - DNA, 46 bp, Artificial Sequence
  Primer
  misc_feature (17)..(18): n is a, c, g, or t
  misc_feature (20)..(21): n is a, c, g, or t
  misc_feature (23)..(24): n is a, c, g, or t
gtagagcgaagcagacnngnntnnaccaagcacgccaatagaattg

SEQ ID NO: 333 - DNA, 45 bp, Artificial Sequence
  Primer
  misc_feature (17)..(18): n is a, c, g, or t
  misc_feature (20)..(21): n is a, c, g, or t
  misc_feature (23)..(24): n is a, c, g, or t
tggcgtgcttggtgtanncnngnntgcttcgctctacgccgttaa

SEQ ID NO: 334 - DNA, 45 bp, Artificial Sequence
  Primer
  misc_feature (17)..(18): n is a, c, g, or t
  misc_feature (20)..(21): n is a, c, g, or t
  misc_feature (23)..(24): n is a, c, g, or t
ggcgtagagcgaagcanncnngnntacaccaagcacgccaataga

SEQ ID NO: 335 - DNA, 45 bp, Artificial Sequence
  Primer
  misc_feature (16)..(17): n is a, c, g, or t
  misc_feature (19)..(20): n is a, c, g, or t
  misc_feature (22)..(23): n is a, c, g, or t
gtgcttggtgtagccnngnntnnttcgctctacgccgttaaagtt

SEQ ID NO: 336 - DNA, 44 bp, Artificial Sequence
  Primer
  misc_feature (17)..(18): n is a, c, g, or t
  misc_feature (20)..(21): n is a, c, g, or t
  misc_feature (23)..(24): n is a, c, g, or t
aacggcgtagagcgaannanncnnggctacaccaagcacgccaa

SEQ ID NO: 337 - DNA, 45 bp, Artificial Sequence
  Primer
  misc_feature (16)..(17): n is a, c, g, or t
  misc_feature (19)..(20): n is a, c, g, or t
  misc_feature (22)..(23): n is a, c, g, or t
cttggtgtagccccgnntnntnngctctacgccgttaaagttctt

SEQ ID NO: 338 - DNA, 48 bp, Artificial Sequence
  Primer
  misc_feature (17)..(18): n is a, c, g, or t
  misc_feature (20)..(21): n is a, c, g, or t
  misc_feature (23)..(24): n is a, c, g, or t
tttaacggcgtagagcnnannanncggggctacaccaagcacgccaat

SEQ ID NO: 339 - DNA, 46 bp, Artificial Sequence
  Primer
  misc_feature (16)..(17): n is a, c, g, or t
  misc_feature (19)..(20): n is a, c, g, or t
  misc_feature (22)..(23): n is a, c, g, or t
ggtgtagccccgtctnntnngnnctacgccgttaaagttcttgcag

SEQ ID NO: 340 - DNA, 44 bp, Artificial Sequence
  Primer
  misc_feature (17)..(18): n is a, c, g, or t
  misc_feature (20)..(21): n is a, c, g, or t
  misc_feature (23)..(24): n is a, c, g, or t
aactttaacggcgtagnncnnannagacggggctacaccaagca

SEQ ID NO: 341 - DNA, 45 bp, Artificial Sequence
  Primer
  misc_feature (16)..(17): n is a, c, g, or t
  misc_feature (19)..(20): n is a, c, g, or t
  misc_feature (22)..(23): n is a, c, g, or t
gtagccccgtctgctnngnncnncgccgttaaagttcttgcagca

SEQ ID NO: 342 - DNA, 44 bp, Artificial Sequence
  Primer
  misc_feature (17)..(18): n is a, c, g, or t
  misc_feature (20)..(21): n is a, c, g, or t
  misc_feature (23)..(24): n is a, c, g, or t
aagaactttaacggcgnngnncnnagcagacggggctacaccaa

SEQ ID NO: 343 - DNA, 45 bp, Artificial Sequence
  Primer
  misc_feature (16)..(17): n is a, c, g, or t
  misc_feature (19)..(20): n is a, c, g, or t
  misc_feature (22)..(23): n is a, c, g, or t
gccccgtctgcttcgnncnncnncgttaaagttcttgcagcagac

SEQ ID NO: 344 - DNA, 44 bp, Artificial Sequence
  Primer
  misc_feature (17)..(18): n is a, c, g, or t
  misc_feature (20)..(21): n is a, c, g, or t
  misc_feature (23)..(24): n is a, c, g, or t
tgcaagaactttaacgnngnngnncgaagcagacggggctacac

SEQ ID NO: 345 - DNA, 45 bp, Artificial Sequence
  Primer
  misc_feature (16)..(17): n is a, c, g, or t
  misc_feature (19)..(20): n is a, c, g, or t
  misc_feature (22)..(23): n is a, c, g, or t
ccgtctgcttcgctcnncnncnntaaagttcttgcagcagacgga

SEQ ID NO: 346 - DNA, 43 bp, Artificial Sequence
  Primer
  misc_feature (17)..(18): n is a, c, g, or t
  misc_feature (20)..(21): n is a, c, g, or t
  misc_feature (23)..(24): n is a, c, g, or t
tgctgcaagaactttanngnngnngagcgaagcagacggggct

SEQ ID NO: 347 - DNA, 44 bp, Artificial Sequence
  Primer
  misc_feature (16)..(17): n is a, c, g, or t
  misc_feature (19)..(20): n is a, c, g, or t
  misc_feature (22)..(23): n is a, c, g, or t
tctgcttcgctctacnncnntnnagttcttgcagcagacggatc

SEQ ID NO: 348 - DNA, 47 bp, Artificial Sequence
  Primer
  misc_feature (17)..(18): n is a, c, g, or t
  misc_feature (20)..(21): n is a, c, g, or t
  misc_feature (23)..(24): n is a, c, g, or t
gtctgctgcaagaactnnanngnngtagagcgaagcagacggggcta

SEQ ID NO: 349 - DNA, 43 bp, Artificial Sequence
  Primer
  misc_feature (16)..(17): n is a, c, g, or t
  misc_feature (19)..(20): n is a, c, g, or t
  misc_feature (22)..(23): n is a, c, g, or t
gcttcgctctacgccnntnnanntcttgcagcagacggatcag

SEQ ID NO: 350 - DNA, 44 bp, Artificial Sequence
  Primer
  misc_feature (17)..(18): n is a, c, g, or t
  misc_feature (20)..(21): n is a, c, g, or t
  misc_feature (23)..(24): n is a, c, g, or t
tccgtctgctgcaaganntnnannggcgtagagcgaagcagacg

SEQ ID NO: 351 - DNA, 44 bp, Artificial Sequence
  Primer
  misc_feature (16)..(17): n is a, c, g, or t
  misc_feature (19)..(20): n is a, c, g, or t
  misc_feature (22)..(23): n is a, c, g, or t
tcgctctacgccgttnnanntnntgcagcagacggatcaggcca

SEQ ID NO: 352 - DNA, 44 bp, Artificial Sequence
  Primer
  misc_feature (17)..(18): n is a, c, g, or t
  misc_feature (20)..(21): n is a, c, g, or t
  misc_feature (23)..(24): n is a, c, g, or t
tgatccgtctgctgcannanntnnaacggcgtagagcgaagcag

SEQ ID NO: 353 - DNA, 44 bp, Artificial Sequence
  Primer
  misc_feature (16)..(17): n is a, c, g, or t
  misc_feature (19)..(20): n is a, c, g, or t
  misc_feature (22)..(23): n is a, c, g, or t
ctctacgccgttaaanntnntnnagcagacggatcaggccaata

SEQ ID NO: 354 - DNA, 44 bp, Artificial Sequence
  Primer
  misc_feature (17)..(18): n is a, c, g, or t
  misc_feature (20)..(21): n is a, c, g, or t
  misc_feature (23)..(24): n is a, c, g, or t
gcctgatccgtctgctnnannanntttaacggcgtagagcgaag

SEQ ID NO: 355 - DNA, 44 bp, Artificial Sequence
  Primer
  misc_feature (16)..(17): n is a, c, g, or t
  misc_feature (19)..(20): n is a, c, g, or t
  misc_feature (22)..(23): n is a, c, g, or t
tacgccgttaaagttnntnnannagacggatcaggccaatactc

SEQ ID NO: 356 - DNA, 45 bp, Artificial Sequence
  Primer
  misc_feature (17)..(18): n is a, c, g, or t
  misc_feature (20)..(21): n is a, c, g, or t
  misc_feature (23)..(24): n is a, c, g, or t
ttggcctgatccgtctnntnnannaactttaacggcgtagagcga

SEQ ID NO: 357 - DNA, 44 bp, Artificial Sequence
  Primer
  misc_feature (16)..(17): n is a, c, g, or t
  misc_feature (19)..(20): n is a, c, g, or t
  misc_feature (22)..(23): n is a, c, g, or t
gccgttaaagttcttnnannanncggatcaggccaatactcatg

SEQ ID NO: 358 - DNA, 45 bp, Artificial Sequence
  Primer
  misc_feature (17)..(18): n is a, c, g, or t
  misc_feature (20)..(21): n is a, c, g, or t
  misc_feature (23)..(24): n is a, c, g, or t
gtattggcctgatccgnntnntnnaagaactttaacggcgtagag

SEQ ID NO: 359 - DNA, 46 bp, Artificial Sequence
  Primer
  misc_feature (16)..(17): n is a, c, g, or t
  misc_feature (19)..(20): n is a, c, g, or t
  misc_feature (22)..(23): n is a, c, g, or t
gttaaagttcttgcannanncnnatcaggccaatactcatggatta

SEQ ID NO: 360 - DNA, 46 bp, Artificial Sequence
  Primer
  misc_feature (17)..(18): n is a, c, g, or t
  misc_feature (20)..(21): n is a, c, g, or t
  misc_feature (23)..(24): n is a, c, g, or t
tgagtattggcctgatnngnntnntgcaagaactttaacggcgtag

SEQ ID NO: 361 - DNA, 45 bp, Artificial Sequence
  Primer
  misc_feature (16)..(17): n is a, c, g, or t
  misc_feature (19)..(20): n is a, c, g, or t
  misc_feature (22)..(23): n is a, c, g, or t
aaagttcttgcagcanncnnannaggccaatactcatggattatc

SEQ ID NO: 362 - DNA, 48 bp, Artificial Sequence
  Primer
  misc_feature (17)..(18): n is a, c, g, or t
  misc_feature (20)..(21): n is a, c, g, or t
  misc_feature (23)..(24): n is a, c, g, or t
ccatgagtattggcctnntnngnntgctgcaagaactttaacggcgta

SEQ ID NO: 363 - DNA, 45 bp, Artificial Sequence
  Primer
  misc_feature (16)..(17): n is a, c, g, or t
  misc_feature (19)..(20): n is a, c, g, or t
  misc_feature (22)..(23): n is a, c, g, or t
gttcttgcagcagacnnannannccaatactcatggattatcaac

SEQ ID NO: 364 - DNA, 46 bp, Artificial Sequence
  Primer
  misc_feature (17)..(18): n is a, c, g, or t
  misc_feature (20)..(21): n is a, c, g, or t
  misc_feature (23)..(24): n is a, c, g, or t
aatccatgagtattggnntnntnngtctgctgcaagaactttaacg

SEQ ID NO: 365 - DNA, 46 bp, Artificial Sequence
  Primer
  misc_feature (16)..(17): n is a, c, g, or t
  misc_feature (19)..(20): n is a, c, g, or t
  misc_feature (22)..(23): n is a, c, g, or t
cttgcagcagacggannanncnnatactcatggattatcaacggca

SEQ ID NO: 366 - DNA, 45 bp, Artificial Sequence
  Primer
  misc_feature (17)..(18): n is a, c, g, or t
  misc_feature (20)..(21): n is a, c, g, or t
  misc_feature (23)..(24): n is a, c, g, or t
gataatccatgagtatnngnntnntccgtctgctgcaagaacttt

SEQ ID NO: 367 - DNA, 45 bp, Artificial Sequence
  Primer
  misc_feature (16)..(17): n is a, c, g, or t
  misc_feature (19)..(20): n is a, c, g, or t
  misc_feature (22)..(23): n is a, c, g, or t
gcagcagacggatcanncnnannctcatggattatcaacggcatc

SEQ ID NO: 368 - DNA, 44 bp, Artificial Sequence
  Primer
  misc_feature (16)..(17): n is a, c, g, or t
  misc_feature (19)..(20): n is a, c, g, or t
  misc_feature (22)..(23): n is a, c, g, or t
ttgataatccatgagnntnngnntgatccgtctgctgcaagaac

SEQ ID NO: 369 - DNA, 46 bp, Artificial Sequence
  Primer
  misc_feature (16)..(17): n is a, c, g, or t
  misc_feature (19)..(20): n is a, c, g, or t
  misc_feature (22)..(23): n is a, c, g, or t
gcagacggatcaggcnnanncnnatggattatcaacggcatcgaat

SEQ ID NO: 370 - DNA, 44 bp, Artificial Sequence
  Primer
  misc_feature (17)..(18): n is a, c, g, or t
  misc_feature (20)..(21): n is a, c, g, or t
  misc_feature (23)..(24): n is a, c, g, or t
gccgttgataatccatnngnntnngcctgatccgtctgctgcaa

SEQ ID NO: 371 - DNA, 45 bp, Artificial Sequence
  Primer
  misc_feature (16)..(17): n is a, c, g, or t
  misc_feature (19)..(20): n is a, c, g, or t
  misc_feature (22)..(23): n is a, c, g, or t
gacggatcaggccaanncnnanngattatcaacggcatcgaatgg

SEQ ID NO: 372 - DNA, 44 bp, Artificial Sequence
  Primer
  misc_feature (17)..(18): n is a, c, g, or t
  misc_feature (20)..(21): n is a, c, g, or t
  misc_feature (23)..(24): n is a, c, g, or t
gatgccgttgataatcnntnngnnttggcctgatccgtctgctg

SEQ ID NO: 373 - DNA, 47 bp, Artificial Sequence
  Primer
  misc_feature (16)..(17): n is a, c, g, or t
  misc_feature (19)..(20): n is a, c, g, or t
  misc_feature (22)..(23): n is a, c, g, or t
ggatcaggccaatacnnanngnntatcaacggcatcgaatgggccat

SEQ ID NO: 374 - DNA, 44 bp, Artificial Sequence
  Primer
  misc_feature (17)..(18): n is a, c, g, or t
  misc_feature (20)..(21): n is a, c, g, or t
  misc_feature (23)..(24): n is a, c, g, or t
ttcgatgccgttgatanncnntnngtattggcctgatccgtctg

SEQ ID NO: 375 - DNA, 44 bp, Artificial Sequence
  Primer
  misc_feature (16)..(17): n is a, c, g, or t
  misc_feature (19)..(20): n is a, c, g, or t
  misc_feature (22)..(23): n is a, c, g, or t
tcaggccaatactcanngnntnncaacggcatcgaatgggccat

SEQ ID NO: 376 - DNA, 45 bp, Artificial Sequence
  Primer
  misc_feature (17)..(18): n is a, c, g, or t
  misc_feature (20)..(21): n is a, c, g, or t
  misc_feature (23)..(24): n is a, c, g, or t
ccattcgatgccgttgnnanncnntgagtattggcctgatccgtc

SEQ ID NO: 377 - DNA, 48 bp, Artificial Sequence
  Primer
  misc_feature (16)..(17): n is a, c, g, or t
  misc_feature (19)..(20): n is a, c, g, or t
  misc_feature (22)..(23): n is a, c, g, or t
ggccaatactcatggnntnncnncggcatcgaatgggccatcgcgaat

SEQ ID NO: 378 - DNA, 45 bp, Artificial Sequence
  Primer
  misc_feature (17)..(18): n is a, c, g, or t
  misc_feature (20)..(21): n is a, c, g, or t
  misc_feature (23)..(24): n is a, c, g, or t
ggcccattcgatgccgnngnnannccatgagtattggcctgatcc

SEQ ID NO: 379 - DNA, 44 bp, Artificial Sequence
  Primer
  misc_feature (16)..(17): n is a, c, g, or t
  misc_feature (19)..(20): n is a, c, g, or t
  misc_feature (22)..(23): n is a, c, g, or t
caatactcatggattnncnncnncatcgaatgggccatcgcgaa

SEQ ID NO: 380 - DNA, 46 bp, Artificial Sequence
  Primer
  misc_feature (17)..(18): n is a, c, g, or t
  misc_feature (20)..(21): n is a, c, g, or t
  misc_feature (23)..(24): n is a, c, g, or t
gatggcccattcgatgnngnngnnaatccatgagtattggcctgat

SEQ ID NO: 381 - DNA, 44 bp, Artificial Sequence
  Primer
  misc_feature (16)..(17): n is a, c, g, or t
  misc_feature (19)..(20): n is a, c, g, or t
  misc_feature (22)..(23): n is a, c, g, or t
tactcatggattatcnncnncnncgaatgggccatcgcgaataa

SEQ ID NO: 382 - DNA, 46 bp, Artificial Sequence
  Primer
  misc_feature (17)..(18): n is a, c, g, or t
  misc_feature (20)..(21): n is a, c, g, or t
  misc_feature (23)..(24): n is a, c, g, or t
cgcgatggcccattcgnngnngnngataatccatgagtattggcct

SEQ ID NO: 383 - DNA, 45 bp, Artificial Sequence
  Primer
  misc_feature (16)..(17): n is a, c, g, or t
  misc_feature (19)..(20): n is a, c, g, or t
  misc_feature (22)..(23): n is a, c, g, or t
tcatggattatcaacnncnncnnatgggccatcgcgaataacatg

SEQ ID NO: 384 - DNA, 46 bp, Artificial Sequence
  Primer
  misc_feature (17)..(18): n is a, c, g, or t
  misc_feature (20)..(21): n is a, c, g, or t
  misc_feature (23)..(24): n is a, c, g, or t
attcgcgatggcccatnngnngnngttgataatccatgagtattgg

SEQ ID NO: 385 - DNA, 44 bp, Artificial Sequence
  Primer
  misc_feature (16)..(17): n is a, c, g, or t
  misc_feature (19)..(20): n is a, c, g, or t
  misc_feature (22)..(23): n is a, c, g, or t
tggattatcaacggcnncnnannggccatcgcgaataacatgga

SEQ ID NO: 386 - DNA, 46 bp, Artificial Sequence
  Primer
  misc_feature (17)..(18): n is a, c, g, or t
  misc_feature (20)..(21): n is a, c, g, or t
  misc_feature (23)..(24): n is a, c, g, or t
gttattcgcgatggccnntnngnngccgttgataatccatgagtat

SEQ ID NO: 387 - DNA, 46 bp, Artificial Sequence
  Primer
  misc_feature (16)..(17): n is a, c, g, or t
  misc_feature (19)..(20): n is a, c, g, or t
  misc_feature (22)..(23): n is a, c, g, or t
attatcaacggcatcnnanngnncatcgcgaataacatggatgtaa

SEQ ID NO: 388 - DNA, 46 bp, Artificial Sequence
  Primer
  misc_feature (17)..(18): n is a, c, g, or t
  misc_feature (20)..(21): n is a, c, g, or t
  misc_feature (23)..(24): n is a, c, g, or t
catgttattcgcgatgnncnntnngatgccgttgataatccatgag

SEQ ID NO: 389 - DNA, 47 bp, Artificial Sequence
  Primer
  misc_feature (16)..(17): n is a, c, g, or t
  misc_feature (19)..(20): n is a, c, g, or t
  misc_feature (22)..(23): n is a, c, g, or t
atcaacggcatcgaanngnncnncgcgaataacatggatgtaatcaa

SEQ ID NO: 390 - DNA, 46 bp, Artificial Sequence
  Primer
  misc_feature (17)..(18): n is a, c, g, or t
  misc_feature (20)..(21): n is a, c, g, or t
  misc_feature (23)..(24): n is a, c, g, or t
atccatgttattcgcgnngnncnnttcgatgccgttgataatccat

SEQ ID NO: 391 - DNA, 47 bp, Artificial Sequence
  Primer
  misc_feature (16)..(17): n is a, c, g, or t
  misc_feature (19)..(20): n is a, c, g, or t
  misc_feature (22)..(23): n is a, c, g, or t
aacggcatcgaatggnncnncnngaataacatggatgtaatcaacat

SEQ ID NO: 392 - DNA, 47 bp, Artificial Sequence; identical to SEQ ID NO: 391
  Primer
  misc_feature (16)..(17): n is a, c, g, or t
  misc_feature (19)..(20): n is a, c, g, or t
  misc_feature (22)..(23): n is a, c, g, or t

SEQ ID NO: 393 - DNA, 47 bp, Artificial Sequence
  Primer
  misc_feature (16)..(17): n is a, c, g, or t
  misc_feature (19)..(20): n is a, c, g, or t
  misc_feature (22)..(23): n is a, c, g, or t
ggcatcgaatgggccnncnngnntaacatggatgtaatcaacatgag

SEQ ID NO: 394 - DNA, 44 bp, Artificial Sequence
  Primer
  misc_feature (17)..(18): n is a, c, g, or t
  misc_feature (20)..(21): n is a, c, g, or t
  misc_feature (23)..(24): n is a, c, g, or t
gattacatccatgttanncnngnnggcccattcgatgccgttga

SEQ ID NO: 395 - DNA, 47 bp, Artificial Sequence
  Primer
  misc_feature (16)..(17): n is a, c, g, or t
  misc_feature (19)..(20): n is a, c, g, or t
  misc_feature (22)..(23): n is a, c, g, or t
atcgaatgggccatcnngnntnncatggatgtaatcaacatgagcct

SEQ ID NO: 396 - DNA, 44 bp, Artificial Sequence
  Primer
  misc_feature (17)..(18): n is a, c, g, or t
  misc_feature (20)..(21): n is a, c, g, or t
  misc_feature (23)..(24): n is a, c, g, or t
gttgattacatccatgnnanncnngatggcccattcgatgccgt

SEQ ID NO: 397 - DNA, 45 bp, Artificial Sequence
  Primer
  misc_feature (16)..(17): n is a, c, g, or t
  misc_feature (19)..(20): n is a, c, g, or t
  misc_feature (22)..(23): n is a, c, g, or t
gaatgggccatcgcgnntnncnnggatgtaatcaacatgagcctg

SEQ ID NO: 398 - DNA, 44 bp, Artificial Sequence
  Primer
  misc_feature (17)..(18): n is a, c, g, or t
  misc_feature (20)..(21): n is a, c, g, or t
  misc_feature (23)..(24): n is a, c, g, or t
catgttgattacatccnngnnanncgcgatggcccattcgatgc

SEQ ID NO: 399 - DNA, 45 bp, Artificial Sequence
  Primer
  misc_feature (16)..(17): n is a, c, g, or t
  misc_feature (19)..(20): n is a, c, g, or t
  misc_feature (22)..(23): n is a, c, g, or t
tgggccatcgcgaatnncnngnntgtaatcaacatgagcctggga

SEQ ID NO: 400 - DNA, 44 bp, Artificial Sequence
  Primer
  misc_feature (17)..(18): n is a, c, g, or t
  misc_feature (20)..(21): n is a, c, g, or t
  misc_feature (23)..(24): n is a, c, g, or t
gctcatgttgattacanncnngnnattcgcgatggcccattcga

SEQ ID NO: 401 - DNA, 45 bp, Artificial Sequence
  Primer
  misc_feature (16)..(17): n is a, c, g, or t
  misc_feature (19)..(20): n is a, c, g, or t
  misc_feature (22)..(23): n is a, c, g, or t
gccatcgcgaataacnngnntnnaatcaacatgagcctgggagca

SEQ ID NO: 402 - DNA, 45 bp, Artificial Sequence
  Primer
  misc_feature (17)..(18): n is a, c, g, or t
  misc_feature (20)..(21): n is a, c, g, or t
  misc_feature (23)..(24): n is a, c, g, or t
caggctcatgttgattnnanncnngttattcgcgatggcccattc

SEQ ID NO: 403 - DNA, 43 bp, Artificial Sequence
  Primer
  misc_feature (16)..(17): n is a, c, g, or t
  misc_feature (19)..(20): n is a, c, g, or t
  misc_feature (22)..(23): n is a, c, g, or t
atcgcgaataacatgnntnnanncaacatgagcctgggagcac

SEQ ID NO: 404 - DNA, 46 bp, Artificial Sequence
  Primer
  misc_feature (17)..(18): n is a, c, g, or t
  misc_feature (20)..(21): n is a, c, g, or t
  misc_feature (23)..(24): n is a, c, g, or t
tcccaggctcatgttgnntnnanncatgttattcgcgatggcccat

SEQ ID NO: 405 - DNA, 44 bp, Artificial Sequence
  Primer
  misc_feature (16)..(17): n is a, c, g, or t
  misc_feature (19)..(20): n is a, c, g, or t
  misc_feature (22)..(23): n is a, c, g, or t
gcgaataacatggatnnanncnncatgagcctgggagcaccaag

SEQ ID NO: 406 - DNA, 50 bp, Artificial Sequence
  Primer
  misc_feature (17)..(18): n is a, c, g, or t
  misc_feature (20)..(21): n is a, c, g, or t
  misc_feature (23)..(24): n is a, c, g, or t
tgctcccaggctcatgnngnntnnatccatgttattcgcgatggcccatt

SEQ ID NO: 407 - DNA, 46 bp, Artificial Sequence
  Primer
  misc_feature (16)..(17): n is a, c, g, or t
  misc_feature (19)..(20): n is a, c, g, or t
  misc_feature (22)..(23): n is a, c, g, or t
aataacatggatgtanncnncnngagcctgggagcaccaagcggca

SEQ ID NO: 408 - DNA, 46 bp, Artificial Sequence
  Primer
  misc_feature (17)..(18): n is a, c, g, or t
  misc_feature (20)..(21): n is a, c, g, or t
  misc_feature (23)..(24): n is a, c, g, or t
tggtgctcccaggctcnngnngnntacatccatgttattcgcgatg

SEQ ID NO: 409 - DNA, 43 bp, Artificial Sequence
  Primer
  misc_feature (16)..(17): n is a, c, g, or t
  misc_feature (19)..(20): n is a, c, g, or t
  misc_feature (22)..(23): n is a, c, g, or t
aacatggatgtaatcnncnngnncctgggagcaccaagcggca

SEQ ID NO: 410 - DNA, 47 bp, Artificial Sequence
  Primer
  misc_feature (17)..(18): n is a, c, g, or t
  misc_feature (20)..(21): n is a, c, g, or t
  misc_feature (23)..(24): n is a, c, g, or t
gcttggtgctcccaggnncnngnngattacatccatgttattcgcga

SEQ ID NO: 411 - DNA, 43 bp, Artificial Sequence
  Primer
  misc_feature (16)..(17): n is a, c, g, or t
  misc_feature (19)..(20): n is a, c, g, or t
  misc_feature (22)..(23): n is a, c, g, or t
atggatgtaatcaacnngnncnngggagcaccaagcggcagtg

SEQ ID NO: 412 - DNA, 47 bp, Artificial Sequence
  Primer
  misc_feature (17)..(18): n is a, c, g, or t
  misc_feature (20)..(21): n is a, c, g, or t
  misc_feature (23)..(24): n is a, c, g, or t
gccgcttggtgctcccnngnncnngttgattacatccatgttattcg

SEQ ID NO: 413 - DNA, 45 bp, Artificial Sequence
  Primer
  misc_feature (16)..(17): n is a, c, g, or t
  misc_feature (19)..(20): n is a, c, g, or t
  misc_feature (22)..(23): n is a, c, g, or t
gatgtaatcaacatgnncnngnnagcaccaagcggcagtgcggca

SEQ ID NO: 414 - DNA, 48 bp, Artificial Sequence
  Primer
  misc_feature (17)..(18): n is a, c, g, or t
  misc_feature (20)..(21): n is a, c, g, or t
  misc_feature (23)..(24): n is a, c, g, or t
actgccgcttggtgctnncnngnncatgttgattacatccatgttatt

SEQ ID NO: 415 - DNA, 44 bp, Artificial Sequence
  Primer
  misc_feature (16)..(17): n is a, c, g, or t
  misc_feature (19)..(20): n is a, c, g, or t
  misc_feature (22)..(23): n is a, c, g, or t
gtaatcaacatgagcnngnnannaccaagcggcagtgcggcact

SEQ ID NO: 416 - DNA, 46 bp, Artificial Sequence
  Primer
  misc_feature (17)..(18): n is a, c, g, or t
  misc_feature (20)..(21): n is a, c, g, or t
  misc_feature (23)..(24): n is a, c, g, or t
cgcactgccgcttggtnntnncnngctcatgttgattacatccatg

SEQ ID NO: 417 - DNA, 45 bp, Artificial Sequence
  Primer
  misc_feature (16)..(17): n is a, c, g, or t
  misc_feature (19)..(20): n is a, c, g, or t
  misc_feature (22)..(23): n is a, c, g, or t
atgagcctgggagcannanncnncagtgcggcacttaaagcagca

SEQ ID NO: 418 - DNA, 45 bp, Artificial Sequence
  Primer
  misc_feature (17)..(18): n is a, c, g, or t
  misc_feature (20)..(21): n is a, c, g, or t
  misc_feature (23)..(24): n is a, c, g, or t
tttaagtgccgcactgnngnntnntgctcccaggctcatgttgat

SEQ ID NO: 419 - DNA, 46 bp, Artificial Sequence
  Primer
  misc_feature (16)..(17): n is a, c, g, or t
  misc_feature (19)..(20): n is a, c, g, or t
  misc_feature (22)..(23): n is a, c, g, or t
ggagcaccaagcggcnntnngnnacttaaagcagcagttgataaag

SEQ ID NO: 420 - DNA, 45 bp, Artificial Sequence
  Primer
  misc_feature (17)..(18): n is a, c, g, or t
  misc_feature (20)..(21): n is a, c, g, or t
  misc_feature (23)..(24): n is a, c, g, or t
aactgctgctttaagtnncnnanngccgcttggtgctcccaggct

SEQ ID NO: 421 - DNA, 46 bp, Artificial Sequence
  Primer
  misc_feature (16)..(17): n is a, c, g, or t
  misc_feature (19)..(20): n is a, c, g, or t
  misc_feature (22)..(23): n is a, c, g, or t
gcaccaagcggcagtnngnnanntaaagcagcagttgataaagctg

SEQ ID NO: 422 - DNA, 44 bp, Artificial Sequence
  Primer
  misc_feature (17)..(18): n is a, c, g, or t
  misc_feature (20)..(21): n is a, c, g, or t
  misc_feature (23)..(24): n is a, c, g, or t
atcaactgctgctttanntnncnnactgccgcttggtgctccca

SEQ ID NO: 423 - DNA, 46 bp, Artificial Sequence
  Primer
  misc_feature (16)..(17): n is a, c, g, or t
  misc_feature (19)..(20): n is a, c, g, or t
  misc_feature (22)..(23): n is a, c, g, or t
ccaagcggcagtgcgnnanntnnagcagcagttgataaagctgttg

SEQ ID NO: 424 - DNA, 44 bp, Artificial Sequence
  Primer
  misc_feature (17)..(18): n is a, c, g, or t
  misc_feature (20)..(21): n is a, c, g, or t
  misc_feature (23)..(24): n is a, c, g, or t
tttatcaactgctgctnnanntnncgcactgccgcttggtgctc

SEQ ID NO: 425 - DNA, 46 bp, Artificial Sequence
  Primer
  misc_feature (16)..(17): n is a, c, g, or t
  misc_feature (19)..(20): n is a, c, g, or t
  misc_feature (22)..(23): n is a, c, g, or t
agcggcagtgcggcanntnnannagcagttgataaagctgttgcat

SEQ ID NO: 426 - DNA, 44 bp, Artificial Sequence
  Primer
  misc_feature (17)..(18): n is a, c, g, or t
  misc_feature (20)..(21): n is a, c, g, or t
  misc_feature (23)..(24): n is a, c, g, or t
agctttatcaactgctnntnnanntgccgcactgccgcttggtg

SEQ ID NO: 427 - DNA, 46 bp, Artificial Sequence
  Primer
  misc_feature (16)..(17): n is a, c, g, or t
  misc_feature (19)..(20): n is a, c, g, or t
  misc_feature (22)..(23): n is a, c, g, or t
ggcagtgcggcacttnnannannagttgataaagctgttgcatctg

SEQ ID NO: 428 - DNA, 44 bp, Artificial Sequence
  Primer
  misc_feature (17)..(18): n is a, c, g, or t
  misc_feature (20)..(21): n is a, c, g, or t
  misc_feature (23)..(24): n is a, c, g, or t
aacagctttatcaactnntnntnnaagtgccgcactgccgcttg

SEQ ID NO: 429 - DNA, 46 bp, Artificial Sequence
  Primer
  misc_feature (16)..(17): n is a, c, g, or t
  misc_feature (19)..(20): n is a, c, g, or t
  misc_feature (22)..(23): n is a, c, g, or t
agtgcggcacttaaannannanntgataaagctgttgcatctggtg

SEQ ID NO: 430 - DNA, 46 bp, Artificial Sequence
  Primer
  misc_feature (17)..(18): n is a, c, g, or t
  misc_feature (20)..(21): n is a, c, g, or t
  misc_feature (23)..(24): n is a, c, g, or t
tgcaacagctttatcanntnntnntttaagtgccgcactgccgctt

SEQ ID NO: 431 - DNA, 45 bp, Artificial Sequence
  Primer
  misc_feature (16)..(17): n is a, c, g, or t
  misc_feature (19)..(20): n is a, c, g, or t
  misc_feature (22)..(23): n is a, c, g, or t
gcggcacttaaagcannanntnntaaagctgttgcatctggtgtc

SEQ ID NO: 432 - DNA, 44 bp, Artificial Sequence
  Primer
  misc_feature (17)..(18): n is a, c, g, or t
  misc_feature (20)..(21): n is a, c, g, or t
  misc_feature (23)..(24): n is a, c, g, or t
agatgcaacagctttannanntnntgctttaagtgccgcactgc

SEQ ID NO: 433 - DNA, 44 bp, Artificial Sequence
  Primer
  misc_feature (16)..(17): n is a, c, g, or t
  misc_feature (19)..(20): n is a, c, g, or t
  misc_feature (22)..(23): n is a, c, g, or t
gcacttaaagcagcanntnntnnagctgttgcatctggtgtcgt

SEQ ID NO: 434 - DNA, 44 bp, Artificial Sequence
  Primer
  misc_feature (17)..(18): n is a, c, g, or t
  misc_feature (20)..(21): n is a, c, g, or t
  misc_feature (23)..(24): n is a, c, g, or t
accagatgcaacagctnnannanntgctgctttaagtgccgcac

SEQ ID NO: 435 - DNA, 44 bp, Artificial Sequence
  Primer
  misc_feature (16)..(17): n is a, c, g, or t
  misc_feature (19)..(20): n is a, c, g, or t
  misc_feature (22)..(23): n is a, c, g, or t
cttaaagcagcagttnntnnanntgttgcatctggtgtcgtcgt

SEQ ID NO: 436 - DNA, 46 bp, Artificial Sequence
  Primer
  misc_feature (17)..(18): n is a, c, g, or t
  misc_feature (20)..(21): n is a, c, g, or t
  misc_feature (23)..(24): n is a, c, g, or t
gacaccagatgcaacanntnnannaactgctgctttaagtgccgca

SEQ ID NO: 437 - DNA, 44 bp, Artificial Sequence
  Primer
  misc_feature (16)..(17): n is a, c, g, or t
  misc_feature (19)..(20): n is a, c, g, or t
  misc_feature (22)..(23): n is a, c, g, or t
aaagcagcagttgatnnanntnntgcatctggtgtcgtcgtagt

SEQ ID NO: 438 - DNA, 45 bp, Artificial Sequence
  Primer
  misc_feature (17)..(18): n is a, c, g, or t
  misc_feature (20)..(21): n is a, c, g, or t
  misc_feature (23)..(24): n is a, c, g, or t
gacgacaccagatgcannanntnnatcaactgctgctttaagtgc

SEQ ID NO: 439 - DNA, 44 bp, Artificial Sequence
  Primer
  misc_feature (16)..(17): n is a, c, g, or t
  misc_feature (19)..(20): n is a, c, g, or t
  misc_feature (22)..(23): n is a, c, g, or t
gcagcagttgataaanntnntnnatctggtgtcgtcgtagtagc

SEQ ID NO: 440 - DNA, 47 bp, Artificial Sequence
  Primer
  misc_feature (17)..(18): n is a, c, g, or t
  misc_feature (20)..(21): n is a, c, g, or t
  misc_feature (23)..(24): n is a, c, g, or t
tacgacgacaccagatnnannanntttatcaactgctgctttaagtg

SEQ ID NO: 441 - DNA, 45 bp, Artificial Sequence
  Primer
  misc_feature (16)..(17): n is a, c, g, or t
  misc_feature (19)..(20): n is a, c, g, or t
  misc_feature (22)..(23): n is a, c, g, or t
gcagttgataaagctnntnnanntggtgtcgtcgtagtagcggca

SEQ ID NO: 442 - DNA, 47 bp, Artificial Sequence
  Primer
  misc_feature (17)..(18): n is a, c, g, or t
  misc_feature (20)..(21): n is a, c, g, or t
  misc_feature (23)..(24): n is a, c, g, or t
tactacgacgacaccanntnnannagctttatcaactgctgctttaa

SEQ ID NO: 443 - DNA, 45 bp, Artificial Sequence
  Primer
  misc_feature (16)..(17): n is a, c, g, or t
  misc_feature (19)..(20): n is a, c, g, or t
  misc_feature (22)..(23): n is a, c, g, or t
gttgataaagctgttnnanntnntgtcgtcgtagtagcggcagct

SEQ ID NO: 444 - DNA, 46 bp, Artificial Sequence
  Primer
  misc_feature (17)..(18): n is a, c, g, or t
  misc_feature (20)..(21): n is a, c, g, or t
  misc_feature (23)..(24): n is a, c, g, or t
cgctactacgacgacannanntnnaacagctttatcaactgctgct

SEQ ID NO: 445 - DNA, 43 bp, Artificial Sequence
  Primer
  misc_feature (16)..(17): n is a, c, g, or t
  misc_feature (19)..(20): n is a, c, g, or t
  misc_feature (22)..(23): n is a, c, g, or t
gataaagctgttgcanntnntnncgtcgtagtagcggcagctg

SEQ ID NO: 446 - DNA, 46 bp, Artificial Sequence
  Primer
  misc_feature (17)..(18): n is a, c, g, or t
  misc_feature (20)..(21): n is a, c, g, or t
  misc_feature (23)..(24): n is a, c, g, or t
tgccgctactacgacgnnannanntgcaacagctttatcaactgct

SEQ ID NO: 447 - DNA, 44 bp, Artificial Sequence
  Primer
  misc_feature (16)..(17): n is a, c, g, or t
  misc_feature (19)..(20): n is a, c, g, or t
  misc_feature (22)..(23): n is a, c, g, or t
aaagctgttgcatctnntnncnncgtagtagcggcagctgggaa

SEQ ID NO: 448 - DNA, 47 bp, Artificial Sequence
  Primer
  misc_feature (17)..(18): n is a, c, g, or t
  misc_feature (20)..(21): n is a, c, g, or t
  misc_feature (23)..(24): n is a, c, g, or t
agctgccgctactacgnngnnannagatgcaacagctttatcaactg

SEQ ID NO: 449 - DNA, 44 bp, Artificial Sequence
  Primer
  misc_feature (16)..(17): n is a, c, g, or t
  misc_feature (19)..(20): n is a, c, g, or t
  misc_feature (22)..(23): n is a, c, g, or t
gctgttgcatctggtnncnncnnagtagcggcagctgggaatga

SEQ ID NO: 450 - DNA, 46 bp, Artificial Sequence
  Primer
  misc_feature (17)..(18): n is a, c, g, or t
  misc_feature (20)..(21): n is a, c, g, or t
  misc_feature (23)..(24): n is a, c, g, or t
cccagctgccgctactnngnngnnaccagatgcaacagctttatca

SEQ ID NO: 451 - DNA, 46 bp, Artificial Sequence
  Primer
  misc_feature (16)..(17): n is a, c, g, or t
  misc_feature (19)..(20): n is a, c, g, or t
  misc_feature (22)..(23): n is a, c, g, or t
gttgcatctggtgtcnncnnannagcggcagctgggaatgagggaa

SEQ ID NO: 452 - DNA, 45 bp, Artificial Sequence
  Primer
  misc_feature (17)..(18): n is a, c, g, or t
  misc_feature (20)..(21): n is a, c, g, or t
  misc_feature (23)..(24): n is a, c, g, or t
attcccagctgccgctnntnngnngacaccagatgcaacagcttt

SEQ ID NO: 453 - DNA, 44 bp, Artificial Sequence
  Primer
  misc_feature (16)..(17): n is a, c, g, or t
  misc_feature (19)..(20): n is a, c, g, or t
  misc_feature (22)..(23): n is a, c, g, or t
gcatctggtgtcgtcnnannannggcagctgggaatgagggaac

SEQ ID NO: 454 - DNA, 44 bp, Artificial Sequence
  Primer
  misc_feature (17)..(18): n is a, c, g, or t
  misc_feature (20)..(21): n is a, c, g, or t
  misc_feature (23)..(24): n is a, c, g, or t
ctcattcccagctgccnntnntnngacgacaccagatgcaacag

SEQ ID NO: 455 - DNA, 44 bp, Artificial Sequence
  Primer
  misc_feature (16)..(17): n is a, c, g, or t
  misc_feature (19)..(20): n is a, c, g, or t
  misc_feature (22)..(23): n is a, c, g, or t
tctggtgtcgtcgtannanngnnagctgggaatgagggaacatc

SEQ ID NO: 456 - DNA, 45 bp, Artificial Sequence
  Primer
  misc_feature (17)..(18): n is a, c, g, or t
  misc_feature (20)..(21): n is a, c, g, or t
  misc_feature (23)..(24): n is a, c, g, or t
tccctcattcccagctnncnntnntacgacgacaccagatgcaac

SEQ ID NO: 457 - DNA, 46 bp, Artificial Sequence
  Primer
  misc_feature (16)..(17): n is a, c, g, or t
  misc_feature (19)..(20): n is a, c, g, or t
  misc_feature (22)..(23): n is a, c, g, or t
ggtgtcgtcgtagtanngnnanntgggaatgagggaacatccggat

SEQ ID NO: 458 - DNA, 46 bp, Artificial Sequence
  Primer
  misc_feature (17)..(18): n is a, c, g, or t
  misc_feature (20)..(21): n is a, c, g, or t
  misc_feature (23)..(24): n is a, c, g, or t
tgttccctcattcccanntnncnntactacgacgacaccagatgca

SEQ ID NO: 459 - DNA, 45 bp, Artificial Sequence
  Primer
  misc_feature (16)..(17): n is a, c, g, or t
  misc_feature (19)..(20): n is a, c, g, or t
  misc_feature (22)..(23): n is a, c, g, or t
gctgggaatgagggannanncnnatcatcgagtaccgtcggttat

SEQ ID NO: 460 - DNA, 47 bp, Artificial Sequence
  Primer
  misc_feature (17)..(18): n is a, c, g, or t
  misc_feature (20)..(21): n is a, c, g, or t
  misc_feature (23)..(24): n is a, c, g, or t
gacggtactcgatgatnngnntnntccctcattcccagctgccgcta

SEQ ID NO: 461 - DNA, 45 bp, Artificial Sequence
  Primer
  misc_feature (16)..(17): n is a, c, g, or t
  misc_feature (19)..(20): n is a, c, g, or t
  misc_feature (22)..(23): n is a, c, g, or t
gggaatgagggaacanncnnannatcgagtaccgtcggttatcca

SEQ ID NO: 462 - DNA, 44 bp, Artificial Sequence
  Primer
  misc_feature (17)..(18): n is a, c, g, or t
  misc_feature (20)..(21): n is a, c, g, or t
  misc_feature (23)..(24): n is a, c, g, or t
accgacggtactcgatnntnngnntgttccctcattcccagctg

SEQ ID NO: 463 - DNA, 44 bp, Artificial Sequence
  Primer
  misc_feature (16)..(17): n is a, c, g, or t
  misc_feature (19)..(20): n is a, c, g, or t
  misc_feature (22)..(23): n is a, c, g, or t
aatgagggaacatccnnannanngagtaccgtcggttatccagg

SEQ ID NO: 464 - DNA, 44 bp, Artificial Sequence
  Primer
  misc_feature (17)..(18): n is a, c, g, or t
  misc_feature (20)..(21): n is a, c, g, or t
  misc_feature (23)..(24): n is a, c, g, or t
ataaccgacggtactcnntnntnnggatgttccctcattcccag

SEQ ID NO: 465 - DNA, 46 bp, Artificial Sequence
  Primer
  misc_feature (16)..(17): n is a, c, g, or t
  misc_feature (19)..(20): n is a, c, g, or t
  misc_feature (22)..(23): n is a, c, g, or t
acatccggatcatcgnntnncnncggttatccaggcaagtaccctt

SEQ ID NO: 466 - DNA, 44 bp, Artificial Sequence
  Primer
  misc_feature (17)..(18): n is a, c, g, or t
  misc_feature (20)..(21): n is a, c, g, or t
  misc_feature (23)..(24): n is a, c, g, or t
cttgcctggataaccgnngnnanncgatgatccggatgttccct

SEQ ID NO: 467 - DNA, 45 bp, Artificial Sequence
  Primer
  misc_feature (16)..(17): n is a, c, g, or t
  misc_feature (19)..(20): n is a, c, g, or t
  misc_feature (22)..(23): n is a, c, g, or t
tccggatcatcgagtnncnncnnttatccaggcaagtacccttca

SEQ ID NO: 468 - DNA, 45 bp, Artificial Sequence
  Primer
  misc_feature (17)..(18): n is a, c, g, or t
  misc_feature (20)..(21): n is a, c, g, or t
  misc_feature (23)..(24): n is a, c, g, or t
gtacttgcctggataanngnngnnactcgatgatccggatgttcc

SEQ ID NO: 469 - DNA, 45 bp, Artificial Sequence
  Primer
  misc_feature (16)..(17): n is a, c, g, or t
  misc_feature (19)..(20): n is a, c, g, or t
  misc_feature (22)..(23): n is a, c, g, or t
tcgagtaccgtcggtnntnnanncaagtacccttcagtgattgca

SEQ ID NO: 470 - DNA, 44 bp, Artificial Sequence
  Primer
  misc_feature (17)..(18): n is a, c, g, or t
  misc_feature (20)..(21): n is a, c, g, or t
  misc_feature (23)..(24): n is a, c, g, or t
cactgaagggtacttgnntnnannaccgacggtactcgatgatc

SEQ ID NO: 471 - DNA, 45 bp, Artificial Sequence
  Primer
  misc_feature (16)..(17): n is a, c, g, or t
  misc_feature (19)..(20): n is a, c, g, or t
  misc_feature (22)..(23): n is a, c, g, or t
agtaccgtcggttatnnanncnngtacccttcagtgattgcagtg

SEQ ID NO: 472 - DNA, 45 bp, Artificial Sequence
  Primer
  misc_feature (17)..(18): n is a, c, g, or t
  misc_feature (20)..(21): n is a, c, g, or t
  misc_feature (23)..(24): n is a, c, g, or t
aatcactgaagggtacnngnntnnataaccgacggtactcgatga

SEQ ID NO: 473 - DNA, 43 bp, Artificial Sequence
  Primer
  misc_feature (16)..(17): n is a, c, g, or t
  misc_feature (19)..(20): n is a, c, g, or t
  misc_feature (22)..(23): n is a, c, g, or t
accgtcggttatccanncnngnncccttcagtgattgcagtgg

SEQ ID NO: 474 - DNA, 45 bp, Artificial Sequence
  Primer
  misc_feature (17)..(18): n is a, c, g, or t
  misc_feature (20)..(21): n is a, c, g, or t
  misc_feature (23)..(24): n is a, c, g, or t
tgcaatcactgaagggnncnngnntggataaccgacggtactcga

SEQ ID NO: 475 - DNA, 45 bp, Artificial Sequence
  Primer
  misc_feature (16)..(17): n is a, c, g, or t
  misc_feature (19)..(20): n is a, c, g, or t
  misc_feature (22)..(23): n is a, c, g, or t
gtcggttatccaggcnngnncnnttcagtgattgcagtgggcgct

SEQ ID NO: 476 - DNA, 44 bp, Artificial Sequence
  Primer
  misc_feature (17)..(18): n is a, c, g, or t
  misc_feature (20)..(21): n is a, c, g, or t
  misc_feature (23)..(24): n is a, c, g, or t
cactgcaatcactgaanngnncnngcctggataaccgacggtac

SEQ ID NO: 477 - DNA, 45 bp, Artificial Sequence
  Primer
  misc_feature (16)..(17): n is a, c, g, or t
  misc_feature (19)..(20): n is a, c, g, or t
  misc_feature (22)..(23): n is a, c, g, or t
ggttatccaggcaagnncnntnnagtgattgcagtgggcgctgta

SEQ ID NO: 478 - DNA, 46 bp, Artificial Sequence
  Primer
  misc_feature (17)..(18): n is a, c, g, or t
  misc_feature (20)..(21): n is a, c, g, or t
  misc_feature (23)..(24): n is a, c, g, or t
gcccactgcaatcactnnanngnncttgcctggataaccgacggta

SEQ ID NO: 479 - DNA, 44 bp, Artificial Sequence
  Primer
  misc_feature (16)..(17): n is a, c, g, or t
  misc_feature (19)..(20): n is a, c, g, or t
  misc_feature (22)..(23): n is a, c, g, or t
tatccaggcaagtacnntnnanngattgcagtgggcgctgtaga

SEQ ID NO: 480 - DNA, 45 bp, Artificial Sequence
  Primer
  misc_feature (17)..(18): n is a, c, g, or t
  misc_feature (20)..(21): n is a, c, g, or t
  misc_feature (23)..(24): n is a, c, g, or t
agcgcccactgcaatcnntnnanngtacttgcctggataaccgac

SEQ ID NO: 481 - DNA, 44 bp, Artificial Sequence
  Primer
  misc_feature (16)..(17): n is a, c, g, or t
  misc_feature (19)..(20): n is a, c, g, or t
  misc_feature (22)..(23): n is a, c, g, or t
gtgggcgctgtagacnntnnanntcaacgtgcctctttttcctc

SEQ ID NO: 482 - DNA, 44 bp, Artificial Sequence
  Primer
  misc_feature (17)..(18): n is a, c, g, or t
  misc_feature (20)..(21): n is a, c, g, or t
  misc_feature (23)..(24): n is a, c, g, or t
aaaagaggcacgttganntnnanngtctacagcgcccactgcaa

SEQ ID NO: 483 - DNA, 44 bp, Artificial Sequence
  Primer
  misc_feature (16)..(17): n is a, c, g, or t
  misc_feature (19)..(20): n is a, c, g, or t
  misc_feature (22)..(23): n is a, c, g, or t
ggcgctgtagactctnnanntnnacgtgcctctttttcctccgt

SEQ ID NO: 484 - DNA, 44 bp, Artificial Sequence
  Primer
  misc_feature (17)..(18): n is a, c, g, or t
  misc_feature (20)..(21): n is a, c, g, or t
  misc_feature (23)..(24): n is a, c, g, or t
ggaaaaagaggcacgtnnanntnnagagtctacagcgcccactg

SEQ ID NO: 485 - DNA, 45 bp, Artificial Sequence
  Primer
  misc_feature (16)..(17): n is a, c, g, or t
  misc_feature (19)..(20): n is a, c, g, or t
  misc_feature (22)..(23): n is a, c, g, or t
gctgtagactcttcanntnnanntgcctctttttcctccgtggga

SEQ ID NO: 486 - DNA, 44 bp, Artificial Sequence
  Primer
  misc_feature (17)..(18): n is a, c, g, or t
  misc_feature (20)..(21): n is a, c, g, or t
  misc_feature (23)..(24): n is a, c, g, or t
ggaggaaaaagaggcanntnnanntgaagagtctacagcgccca

SEQ ID NO: 487 - DNA, 43 bp, Artificial Sequence
  Primer
  misc_feature (16)..(17): n is a, c, g, or t
  misc_feature (19)..(20): n is a, c, g, or t
  misc_feature (22)..(23): n is a, c, g, or t
gtagactcttcaaatnnanntnnctctttttcctccgtgggac

SEQ ID NO: 488 - DNA, 47 bp, Artificial Sequence
  Primer
  misc_feature (17)..(18): n is a, c, g, or t
  misc_feature (20)..(21): n is a, c, g, or t
  misc_feature (23)..(24): n is a, c, g, or t
cacggaggaaaaagagnnanntnnatttgaagagtctacagcgccca

SEQ ID NO: 489 - DNA, 44 bp, Artificial Sequence
  Primer
  misc_feature (16)..(17): n is a, c, g, or t
  misc_feature (19)..(20): n is a, c, g, or t
  misc_feature (22)..(23): n is a, c, g, or t
gactcttcaaatcaanntnncnntttttcctccgtgggaccgga

SEQ ID NO: 490 - DNA, 50 bp, Artificial Sequence
  Primer
  misc_feature (17)..(18): n is a, c, g, or t
  misc_feature (20)..(21): n is a, c, g, or t
  misc_feature (23)..(24): n is a, c, g, or t
tcccacggaggaaaaanngnnannttgatttgaagagtctacagcgccca

SEQ ID NO: 491 - DNA, 45 bp, Artificial Sequence
  Primer
  misc_feature (16)..(17): n is a, c, g, or t
  misc_feature (19)..(20): n is a, c, g, or t
  misc_feature (22)..(23): n is a, c, g, or t
gcctctttttcctccnngnnannggagctggatgtcatggcccct

SEQ ID NO: 492 - DNA, 45 bp, Artificial Sequence
  Primer
  misc_feature (17)..(18): n is a, c, g, or t
  misc_feature (20)..(21): n is a, c, g, or t
  misc_feature (23)..(24): n is a, c, g, or t
catgacatccagctccnntnncnnggaggaaaaagaggcacgttg

SEQ ID NO: 493 - DNA, 45 bp, Artificial Sequence
  Primer
  misc_feature (16)..(17): n is a, c, g, or t
  misc_feature (19)..(20): n is a, c, g, or t
  misc_feature (22)..(23): n is a, c, g, or t
ttttcctccgtggganngnngnnggatgtcatggcccctggcgtt

SEQ ID NO: 494 - DNA, 44 bp, Artificial Sequence
  Primer
  misc_feature (17)..(18): n is a, c, g, or t
  misc_feature (20)..(21): n is a, c, g, or t
  misc_feature (23)..(24): n is a, c, g, or t
aggggccatgacatccnncnncnntcccacggaggaaaaagagg

SEQ ID NO: 495 - DNA, 48 bp, Artificial Sequence
  Primer
  misc_feature (16)..(17): n is a, c, g, or t
  misc_feature (19)..(20): n is a, c, g, or t
  misc_feature (22)..(23): n is a, c, g, or t
tcctccgtgggaccgnngnngnntgtcatggcccctggcgtttctatt

SEQ ID NO: 496 - DNA, 44 bp, Artificial Sequence
  Primer
  misc_feature (17)..(18): n is a, c, g, or t
  misc_feature (20)..(21): n is a, c, g, or t
  misc_feature (23)..(24): n is a, c, g, or t
gccaggggccatgacanncnncnncggtcccacggaggaaaaag

SEQ ID NO: 497 - DNA, 45 bp, Artificial Sequence
  Primer
  misc_feature (16)..(17): n is a, c, g, or t
  misc_feature (19)..(20): n is a, c, g, or t
  misc_feature (22)..(23): n is a, c, g, or t
tccgtgggaccggagnngnntnncatggcccctggcgtttctatt

SEQ ID NO: 498 - DNA, 46 bp, Artificial Sequence
  Primer
  misc_feature (17)..(18): n is a, c, g, or t
  misc_feature (20)..(21): n is a, c, g, or t
  misc_feature (23)..(24): n is a, c, g, or t
aacgccaggggccatgnnanncnnctccggtcccacggaggaaaaa

SEQ ID NO: 499 - DNA, 45 bp, Artificial Sequence
  Primer
  misc_feature (16)..(17): n is a, c, g, or t
  misc_feature (19)..(20): n is a, c, g, or t
  misc_feature (22)..(23): n is a, c, g, or t
gtgggaccggagctgnntnncnnggcccctggcgtttctattcaa

SEQ ID NO: 500 - DNA, 47 bp, Artificial Sequence
  Primer
  misc_feature (17)..(18): n is a, c, g, or t
  misc_feature (20)..(21): n is a, c, g, or t
  misc_feature (23)..(24): n is a, c, g, or t
agaaacgccaggggccnngnnanncagctccggtcccacggaggaaa

SEQ ID NO: 501 - DNA, 46 bp, Artificial Sequence
  Primer
  misc_feature (16)..(17): n is a, c, g, or t
  misc_feature (19)..(20): n is a, c, g, or t
  misc_feature (22)..(23): n is a, c, g, or t
ggaccggagctggatnncnngnnccctggcgtttctattcaatcga

SEQ ID NO: 502 - DNA, 45 bp, Artificial Sequence
  Primer
  misc_feature (17)..(18): n is a, c, g, or t
  misc_feature (20)..(21): n is a, c, g, or t
  misc_feature (23)..(24): n is a, c, g, or t
aatagaaacgccagggnncnngnnatccagctccggtcccacgga

SEQ ID NO: 503 - DNA, 44 bp, Artificial Sequence
  Primer
  misc_feature (16)..(17): n is a, c, g, or t
  misc_feature (19)..(20): n is a, c, g, or t
  misc_feature (22)..(23): n is a, c, g, or t
gtcatggcccctggcnntnntnntcaatcgacgcttccagggaa

SEQ ID NO: 504 - DNA, 44 bp, Artificial Sequence
  Primer
  misc_feature (17)..(18): n is a, c, g, or t
  misc_feature (20)..(21): n is a, c, g, or t
  misc_feature (23)..(24): n is a, c, g, or t
tggaagcgtcgattgannannanngccaggggccatgacatcca

SEQ ID NO: 505 - DNA, 46 bp, Artificial Sequence
  Primer
  misc_feature (16)..(17): n is a, c, g, or t
  misc_feature (19)..(20): n is a, c, g, or t
  misc_feature (22)..(23): n is a, c, g, or t
attcaatcgacgcttnnanngnncaagtatggtgcgcaaaacggga

SEQ ID NO: 506 - DNA, 46 bp, Artificial Sequence
  Primer
  misc_feature (17)..(18): n is a, c, g, or t
  misc_feature (20)..(21): n is a, c, g, or t
  misc_feature (23)..(24): n is a, c, g, or t
ttgcgcaccatacttgnncnntnnaagcgtcgattgaatagaaacg

SEQ ID NO: 507 - DNA, 45 bp, Artificial Sequence
  Primer
  misc_feature (16)..(17): n is a, c, g, or t
  misc_feature (19)..(20): n is a, c, g, or t
  misc_feature (22)..(23): n is a, c, g, or t
caatcgacgcttccanngnncnngtatggtgcgcaaaacgggact

SEQ ID NO: 508 - DNA, 46 bp, Artificial Sequence
  Primer
  misc_feature (17)..(18): n is a, c, g, or t
  misc_feature (20)..(21): n is a, c, g, or t
  misc_feature (23)..(24): n is a, c, g, or t
gttttgcgcaccatacnngnncnntggaagcgtcgattgaatagaa

SEQ ID NO: 509 - DNA, 48 bp, Artificial Sequence
  Primer
  misc_feature (16)..(17): n is a, c, g, or t
  misc_feature (19)..(20): n is a, c, g, or t
  misc_feature (22)..(23): n is a, c, g, or t
gggaacaagtatggtnngnnanncgggacttccatggcctcgccgcat

SEQ ID NO: 510 - DNA, 45 bp, Artificial Sequence
  Primer
  misc_feature (17)..(18): n is a, c, g, or t
  misc_feature (20)..(21): n is a, c, g, or t
  misc_feature (23)..(24): n is a, c, g, or t
ggccatggaagtcccgnntnncnnaccatacttgttccctggaag

SEQ ID NO: 511 - DNA, 45 bp, Artificial Sequence
  Primer
  misc_feature (16)..(17): n is a, c, g, or t
  misc_feature (19)..(20): n is a, c, g, or t
  misc_feature (22)..(23): n is a, c, g, or t
aacaagtatggtgcgnnanncnngacttccatggcctcgccgcat

SEQ ID NO: 512 - DNA, 44 bp, Artificial Sequence
  Primer
  misc_feature (17)..(18): n is a, c, g, or t
  misc_feature (20)..(21): n is a, c, g, or t
  misc_feature (23)..(24): n is a, c, g, or t
cgaggccatggaagtcnngnntnncgcaccatacttgttccctg

SEQ ID NO: 513 - DNA, 43 bp, Artificial Sequence
  Primer
  misc_feature (16)..(17): n is a, c, g, or t
  misc_feature (19)..(20): n is a, c, g, or t
  misc_feature (22)..(23): n is a, c, g, or t
aagtatggtgcgcaanncnngnnttccatggcctcgccgcatg

SEQ ID NO: 514 - DNA, 45 bp, Artificial Sequence
  Primer
  misc_feature (17)..(18): n is a, c, g, or t
  misc_feature (20)..(21): n is a, c, g, or t
  misc_feature (23)..(24): n is a, c, g, or t
cggcgaggccatggaanncnngnnttgcgcaccatacttgttccc

SEQ ID NO: 515 - DNA, 43 bp, Artificial Sequence
  Primer
  misc_feature (16)..(17): n is a, c, g, or t
  misc_feature (19)..(20): n is a, c, g, or t
  misc_feature (22)..(23): n is a, c, g, or t
tatggtgcgcaaaacnngnntnncatggcctcgccgcatgtag

SEQ ID NO: 516 - DNA, 46 bp, Artificial Sequence
  Primer
  misc_feature (17)..(18): n is a, c, g, or t
  misc_feature (20)..(21): n is a, c, g, or t
  misc_feature (23)..(24): n is a, c, g, or t
atgcggcgaggccatgnnanncnngttttgcgcaccatacttgttc

SEQ ID NO: 517 - DNA, 47 bp, Artificial Sequence
  Primer
  misc_feature (16)..(17): n is a, c, g, or t
  misc_feature (19)..(20): n is a, c, g, or t
  misc_feature (22)..(23): n is a, c, g, or t
ccgcatgtagctgggnngnncnnattgattctttctaagcacccgaa

SEQ ID NO: 518 - DNA, 48 bp, Artificial Sequence
  Primer
  misc_feature (17)..(18): n is a, c, g, or t
  misc_feature (20)..(21): n is a, c, g, or t
  misc_feature (23)..(24): n is a, c, g, or t
cttagaaagaatcaatnngnncnncccagctacatgcggcgaggccat

SEQ ID NO: 519 - DNA, 46 bp, Artificial Sequence
  Primer
  misc_feature (16)..(17): n is a, c, g, or t
  misc_feature (19)..(20): n is a, c, g, or t
  misc_feature (22)..(23): n is a, c, g, or t
catgtagctggggcgnncnnanngattctttctaagcacccgaact

SEQ ID NO: 520 - DNA, 51 bp, Artificial Sequence
  Primer
  misc_feature (17)..(18): n is a, c, g, or t
  misc_feature (20)..(21): n is a, c, g, or t
  misc_feature (23)..(24): n is a, c, g, or t
gtgcttagaaagaatcnntnngnncgccccagctacatgcggcgaggccat

SEQ ID NO: 521 - DNA, 44 bp, Artificial Sequence
  Primer
  misc_feature (16)..(17): n is a, c, g, or t
  misc_feature (19)..(20): n is a, c, g, or t
  misc_feature (22)..(23): n is a, c, g, or t
gtagctggggcggccnnanngnntctttctaagcacccgaactg

SEQ ID NO: 522 - DNA, 43 bp, Artificial Sequence
  Primer
  misc_feature (17)..(18): n is a, c, g, or t
  misc_feature (20)..(21): n is a, c, g, or t
  misc_feature (23)..(24): n is a, c, g, or t
cgggtgcttagaaaganncnntnnggccgccccagctacatgc

SEQ ID NO: 523 - DNA, 46 bp, Artificial Sequence
  Primer
  misc_feature (16)..(17): n is a, c, g, or t
  misc_feature (19)..(20): n is a, c, g, or t
  misc_feature (22)..(23): n is a, c, g, or t
ttgattctttctaagnncnngnnctggacaaacactcaagtccgca

SEQ ID NO: 524 - DNA, 45 bp, Artificial Sequence
  Primer
  misc_feature (17)..(18): n is a, c, g, or t
  misc_feature (20)..(21): n is a, c, g, or t
  misc_feature (23)..(24): n is a, c, g, or t
ttgagtgtttgtccagnncnngnncttagaaagaatcaatgcggc

SEQ ID NO: 525 - DNA, 45 bp, Artificial Sequence
  Primer
  misc_feature (16)..(17): n is a, c, g, or t
  misc_feature (19)..(20): n is a, c, g, or t
  misc_feature (22)..(23): n is a, c, g, or t
ctttctaagcacccgnncnngnnaaacactcaagtccgcagcagt

SEQ ID NO: 526 - DNA, 46 bp, Artificial Sequence
  Primer
  misc_feature (17)..(18): n is a, c, g, or t
  misc_feature (20)..(21): n is a, c, g, or t
  misc_feature (23)..(24): n is a, c, g, or t
gcggacttgagtgtttnncnngnncgggtgcttagaaagaatcaat

SEQ ID NO: 527 - DNA, 48 bp, Artificial Sequence
  Primer
  misc_feature (16)..(17): n is a, c, g, or t
  misc_feature (19)..(20): n is a, c, g, or t
  misc_feature (22)..(23): n is a, c, g, or t
tggacaaacactcaanncnncnncagtttagaaaacaccactacaaaa

SEQ ID NO: 528 - DNA, 47 bp, Artificial Sequence
  Primer
  misc_feature (17)..(18): n is a, c, g, or t
  misc_feature (20)..(21): n is a, c, g, or t
  misc_feature (23)..(24): n is a, c, g, or t
ggtgttttctaaactgnngnngnnttgagtgtttgtccagttcgggt

SEQ ID NO: 529 - DNA, 47 bp, Artificial Sequence
  Primer
  misc_feature (16)..(17): n is a, c, g, or t
  misc_feature (19)..(20): n is a, c, g, or t
  misc_feature (22)..(23): n is a, c, g, or t
ttagaaaacaccactnnannanntggtgattctttctactatggaaa

SEQ ID NO: 530 - DNA, 46 bp, Artificial Sequence
  Primer
  misc_feature (17)..(18): n is a, c, g, or t
  misc_feature (20)..(21): n is a, c, g, or t
  misc_feature (23)..(24): n is a, c, g, or t
gtagaaagaatcaccanntnntnnagtggtgttttctaaactgctg

SEQ ID NO: 531 - DNA, 46 bp, Artificial Sequence
  Primer
  misc_feature (16)..(17): n is a, c, g, or t
  misc_feature (19)..(20): n is a, c, g, or t
  misc_feature (22)..(23): n is a, c, g, or t
accactacaaaacttnntnntnntttctactatggaaaagggctga

SEQ ID NO: 532 - DNA, 48 bp, Artificial Sequence
  Primer
  misc_feature (17)..(18): n is a, c, g, or t
  misc_feature (20)..(21): n is a, c, g, or t
  misc_feature (23)..(24): n is a, c, g, or t
ttttccatagtagaaannannannaagttttgtagtggtgttttctaa

SEQ ID NO: 533 - DNA, 45 bp, Artificial Sequence
  Primer
  misc_feature (16)..(17): n is a, c, g, or t
  misc_feature (19)..(20): n is a, c, g, or t
  misc_feature (22)..(23): n is a, c, g, or t
gattctttctactatnnannanngctgatcaacgtacaggcggca

SEQ ID NO: 534 - DNA, 48 bp, Artificial Sequence
  Primer
  misc_feature (17)..(18): n is a, c, g, or t
  misc_feature (20)..(21): n is a, c, g, or t
  misc_feature (23)..(24): n is a, c, g, or t
ctgtacgttgatcagcnntnntnnatagtagaaagaatcaccaagttt

SEQ ID NO: 535 - DNA, 42 bp, Artificial Sequence
  Primer
tcaaggctacaatggagcaaatgttaaagtagcggttatcga

SEQ ID NO: 536 - DNA, 38 bp, Artificial Sequence
  Primer
tttaacatttgctccattgtagccttgagagtgcagag

SEQ ID NO: 537 - DNA, 38 bp, Artificial Sequence
  Primer
ctacactggaggaggtgttaaagtagcggttatcgaca

SEQ ID NO: 538 - DNA, 37 bp, Artificial Sequence
  Primer
ctactttaacacctcctccagtgtagccttgagagtg

SEQ ID NO: 539 - DNA, 40 bp, Artificial Sequence
  Primer
aggctacactggaagaaatgttaaagtagcggttatcgac

SEQ ID NO: 540 - DNA, 34 bp, Artificial Sequence
  Primer
ctttaacatttcttccagtgtagccttgagagtg

SEQ ID NO: 541 - DNA, 42 bp, Artificial Sequence
  Primer
aaggctacactgcaggaggtgttaaagtagcggttatcgaca

SEQ ID NO: 542 - DNA, 40 bp, Artificial Sequence
  Primer
ctactttaacacctcctgcagtgtagccttgagagtgcag

SEQ ID NO: 543 - DNA, 37 bp, Artificial Sequence
  Primer
cgtttcaagatccctcttctcatggcacacacgtcgc

SEQ ID NO: 544 - DNA, 40 bp, Artificial Sequence
  Primer
tgtgccatgagaagagggatcttgaaacgggtttgtttcg

SEQ ID NO: 545 - DNA, 38 bp, Artificial Sequence
  Primer
tgccgtccgaaccaaacccgtttcaagataacaattct

SEQ ID NO: 546 - DNA, 37 bp, Artificial Sequence
  Primer
tcttgaaacgggtttggttcggacggcaccatagaag

SEQ ID NO: 547 - DNA, 40 bp, Artificial Sequence
  Primer
ccgtttcaagatcccaatcatcatggcacacacgtcgcag

SEQ ID NO: 548 - DNA, 42 bp, Artificial Sequence
  Primer
tgtgtgccatgatgattgggatcttgaaacgggtttgtttcg

SEQ ID NO: 549 - DNA, 45 bp, Artificial Sequence
  Primer
acaaacccgttttcagatcccaattctcatggcacacacgtcgca

SEQ ID NO: 550 - DNA, 43 bp, Artificial Sequence
  Primer
ccatgagaattgggatctgaaaacgggtttgtttcggacggca

SEQ ID NO: 551 - DNA, 38 bp, Artificial Sequence
  Primer
ggttgcggcgtcatacaattctattggcgtgcttggtg

SEQ ID NO: 552 - DNA, 38 bp, Artificial Sequence
  Primer
gccaatagaattgtatgacgccgcaaccgttcctgcga

SEQ ID NO: 553 - DNA, 40 bp, Artificial Sequence
  Primer
tggtgtagcctcgggtgtttcgctctacgccgttaaagtt

SEQ ID NO: 554 - DNA, 39 bp, Artificial Sequence
  Primer
cgtagagcgaaacacccgaggctacaccaagcacgccaa

SEQ ID NO: 555 - DNA, 42 bp, Artificial Sequence
  Primer
gtgtagccccgggtgttgcactctacgccgttaaagttcttg

SEQ ID NO: 556 - DNA, 43 bp, Artificial Sequence
  Primer
acggcgtagagtgcaacacccggggctacaccaagcacgccaa

SEQ ID NO: 557 - DNA, 44 bp, Artificial Sequence
  Primer
tggtgtagccccgactcttggactctacgccgttaaagttcttg

SEQ ID NO: 558 - DNA, 43 bp, Artificial Sequence
  Primer
acggcgtagagtccaagagtcggggctacaccaagcacgccaa

SEQ ID NO: 559 - DNA, 41 bp, Artificial Sequence
  Primer
gcctgggagcacaaggctctagtgcggcacttaaagcagca

SEQ ID NO: 560 - DNA, 41 bp, Artificial Sequence
  Primer
agtgccgcactagagccttgtgctcccaggctcatgttgat

SEQ ID NO: 561 - DNA, 37 bp, Artificial Sequence
  Primer
atggcccctggctattctattcaatcgacgcttccag

SEQ ID NO: 562 - DNA, 36 bp, Artificial Sequence
  Primer
tcgattgaatagaatagccaggggccatgacatcca

SEQ ID NO: 563 - DNA, 42 bp, Artificial Sequence
  Primer
tcgacgcttccaaggtccgtgtatggtgcgcaaaacgggact

SEQ ID NO: 564 - DNA, 44 bp, Artificial Sequence
  Primer
ttgcgcaccatacacggaccttggaagcgtcgattgaatagaaa

SEQ ID NO: 565 - DNA, 39 bp, Artificial Sequence
  Primer
catggcacacactgcggaggaacggttgcggcgttaaac

SEQ ID NO: 566 - DNA, 39 bp, Artificial Sequence
  Primer
gcaaccgttcctccgcagtgtgtgccatgagaattgtta

SEQ ID NO: 567 - DNA, 43 bp, Artificial Sequence
  Primer
gtcgcaggaacgattggttcaaacaattctattggcgtgcttg

SEQ ID NO: 568 - DNA, 45 bp, Artificial Sequence
  Primer
caatagaattgtttgaaccaatcgttcctgcgacgtgtgtgccat

SEQ ID NO: 569 - DNA, 41 bp, Artificial Sequence
  Primer
aacggttgcggcgcatggaaattctattggcgtgcttggtg

SEQ ID NO: 570 - DNA, 41 bp, Artificial Sequence
  Primer
caatagaatttccatgcgccgcaaccgttcctgcgacgtgt

SEQ ID NO: 571 - DNA, 43 bp, Artificial Sequence
  Primer
aacggttgcggcgagaggaggttctattggcgtgcttggtgta

SEQ ID NO: 572 - DNA, 46 bp, Artificial Sequence
  Primer
cacgccaatagaacctcctctcgccgcaaccgttcctgcgacgtgt

SEQ ID NO: 573 - DNA, 43 bp, Artificial Sequence
  Primer
aacggttgcggcgggaggcggttctattggcgtgcttggtgta

SEQ ID NO: 574 - DNA, 46 bp, Artificial Sequence
  Primer
cacgccaatagaaccgcctcccgccgcaaccgttcctgcgacgtgt

SEQ ID NO: 575 - DNA, 37 bp, Artificial Sequence
  Primer
tgcttcgctctacggcgttaaagttcttgcagcagac

SEQ ID NO: 576 - DNA, 39 bp, Artificial Sequence
  Primer
caagaactttaacgccgtagagcgaagcagacggggcta

SEQ ID NO: 577 - DNA, 43 bp, Artificial Sequence
  Primer
ttcgctctacgcctcatgttctgcagcagacggatcaggccaa

SEQ ID NO: 578 - DNA, 42 bp, Artificial Sequence
  Primer
atccgtctgctgcagaacatgaggcgtagagcgaagcagacg

SEQ ID NO: 579 - DNA, 41 bp, Artificial Sequence
  Primer
aataacatggatatatcttgcatgagcctgggagcaccaag

SEQ ID NO: 580 - DNA, 44 bp, Artificial Sequence
  Primer
caggctcatgcaagatatatccatgttattcgcgatggcccatt

SEQ ID NO: 581 - DNA, 43 bp, Artificial Sequence
  Primer
cgaataacatggatcttatctgcatgagcctgggagcaccaag

SEQ ID NO: 582 - DNA, 45 bp, Artificial Sequence
  Primer
ccaggctcatgcagataagatccatgttattcgcgatggcccatt

SEQ ID NO: 583 - DNA, 44 bp, Artificial Sequence
  Primer
taacatggatgtatgctcattgagcctgggagcaccaagcggca

SEQ ID NO: 584 - DNA, 43 bp, Artificial Sequence
  Primer
tgctcccaggctcaatgagcatacatccatgttattcgcgatg

SEQ ID NO: 585 - DNA, 37 bp, Artificial Sequence
  Primer
acatggatgtaatctgcatgagcctgggagcaccaag

SEQ ID NO: 586 - DNA, 39 bp, Artificial Sequence
  Primer
tcccaggctcatgcagattacatccatgttattcgcgat

SEQ ID NO: 587 - DNA, 38 bp, Artificial Sequence
  Primer
ggatgtaatcaacatcagcctgggagcaccaagcggca

SEQ ID NO: 588 - DNA, 38 bp, Artificial Sequence
  Primer
tgctcccaggctgatgttgattacatccatgttattcg

SEQ ID NO: 589 - DNA, 38 bp, Artificial Sequence
  Primer
ggatgtaatcaacgtaagcctgggagcaccaagcggca

SEQ ID NO: 590 - DNA, 38 bp, Artificial Sequence
  Primer
tgctcccaggcttacgttgattacatccatgttattcg

SEQ ID NO: 591 - DNA, 41 bp, Artificial Sequence
  Primer
ggatgtaatcaacgtaagcgcgggagcaccaagcggcagtg

SEQ ID NO: 592 - DNA, 42 bp, Artificial Sequence
  Primer
ttggtgctcccgcgcttacgttgattacatccatgttattcg

SEQ ID NO: 593 - DNA, 42 bp, Artificial Sequence
  Primer
aatcaacatgagcttcggagcaagcggcagtgcggcacttaa

SEQ ID NO: 594 - DNA, 42 bp, Artificial Sequence
  Primer
cactgccgcttgctccgaagctcatgttgattacatccatgt

SEQ ID NO: 595 - DNA, 40 bp, Artificial Sequence
  Primer
aacatgagcctgtacgcaccaagcggcagtgcggcactta

SEQ ID NO: 596 - DNA, 41 bp, Artificial Sequence
  Primer
cactgccgcttggtgcgtacaggctcatgttgattacatcc

SEQ ID NO: 597 - DNA, 43 bp, Artificial Sequence
  Primer
caacatgagcctgtcagcagatagcggcagtgcggcacttaaa

SEQ ID NO: 598 - DNA, 42 bp, Artificial Sequence
  Primer
gcactgccgctatctgctgacaggctcatgttgattacatcc

SEQ ID NO: 599 - DNA, 43 bp, Artificial Sequence
  Primer
caacatgagcctgaacgcacgtagcggcagtgcggcacttaaa

SEQ ID NO: 600 - DNA, 42 bp, Artificial Sequence
  Primer
gcactgccgctacgtgcgttcaggctcatgttgattacatcc

SEQ ID NO: 601 - DNA, 42 bp, Artificial Sequence
  Primer
atgagcctgggaaattcatctagcggcagtgcggcacttaaa

SEQ ID NO: 602 - DNA, 41 bp, Artificial Sequence
  Primer
gcactgccgctagatgaatttcccaggctcatgttgattac

SEQ ID NO: 603 - DNA, 40 bp, Artificial Sequence
  Primer
catgagcctgggatcagttagcggcagtgcggcacttaaa

SEQ ID NO: 604 - DNA, 38 bp, Artificial Sequence
  Primer
gcactgccgctaactgatcccaggctcatgttgattac

SEQ ID NO: 605 - DNA, 40 bp, Artificial Sequence
  Primer
catgagcctgggatcagatagcggcagtgcggcacttaaa

SEQ ID NO: 606 - DNA, 38 bp, Artificial Sequence
  Primer
gcactgccgctatctgatcccaggctcatgttgattac

SEQ ID NO: 607 - DNA, 40 bp, Artificial Sequence
  Primer
catgagcctgggatcaggtagcggcagtgcggcacttaaa

SEQ ID NO: 608 - DNA, 38 bp, Artificial Sequence
  Primer
gcactgccgctacctgatcccaggctcatgttgattac

SEQ ID NO: 609 - DNA, 40 bp, Artificial Sequence
  Primer
catgagcctgggacactatagcggcagtgcggcacttaaa

SEQ ID NO: 610 - DNA, 38 bp, Artificial Sequence
  Primer
gcactgccgctatagtgtcccaggctcatgttgattac

SEQ ID NO: 611 - DNA, 36 bp, Artificial Sequence
  Primer
gagcctgggagcagacagcggcagtgcggcacttaa

SEQ ID NO: 612 - DNA, 39 bp, Artificial Sequence
  Primer
tgccgcactgccgctgtctgctcccaggctcatgttgat

SEQ ID NO: 613 - DNA, 36 bp, Artificial Sequence
  Primer
gagcctgggagcagaaagcggcagtgcggcacttaa

SEQ ID NO: 614 - DNA, 39 bp, Artificial Sequence
  Primer
tgccgcactgccgctttctgctcccaggctcatgttgat

SEQ ID NO: 615 - DNA, 36 bp, Artificial Sequence
  Primer
gagcctgggagcagtaagcggcagtgcggcacttaa

SEQ ID NO: 616 - DNA, 39 bp, Artificial Sequence
  Primer
tgccgcactgccgcttactgctcccaggctcatgttgat

SEQ ID NO: 617 - DNA, 36 bp, Artificial Sequence
  Primer
gagcctgggagcaggaggcagtgcggcacttaaagc

SEQ ID NO: 618 - DNA, 38 bp, Artificial Sequence
  Primer
agtgccgcactgcctcctgctcccaggctcatgttgat

SEQ ID NO: 619 - DNA, 42 bp, Artificial Sequence
  Primer
agcctgggagcacacggcaatgcggcacttaaagcagcagtt

SEQ ID NO: 620 - DNA, 42 bp, Artificial Sequence
  Primer
tttaagtgccgcattgccgtgtgctcccaggctcatgttgat

SEQ ID NO: 621 - DNA, 38 bp, Artificial Sequence
  Primer
aagcggcagtgcgacacttaaagcagcagttgataaag

SEQ ID NO: 622 - DNA, 38 bp, Artificial Sequence
  Primer
aactgctgctttaagtgtcgcactgccgcttggtgctc

SEQ ID NO: 623 - DNA, 41 bp, Artificial Sequence
  Primer
gttaaagttcttcgtggttgtgacggatcaggccaatactc

SEQ ID NO: 624 - DNA, 41 bp, Artificial Sequence
  Primer
ctgatccgtcacaaccacgaagaactttaacggcgtagagc

SEQ ID NO: 625 - DNA, 40 bp, Artificial Sequence
  Primer
ttaaagttcttgcaggaggcggatcaggccaatactcatg

SEQ ID NO: 626 - DNA, 42 bp, Artificial Sequence
  Primer
tattggcctgatccgcctcctgcaagaactttaacggcgtag

SEQ ID NO: 627 - DNA, 41 bp, Artificial Sequence
  Primer
ttaaagttcttgcaggacgtgacggatcaggccaatactca

SEQ ID NO: 628 - DNA, 38 bp, Artificial Sequence
  Primer
ctgatccgtcacgtcctgcaagaactttaacggcgtag

SEQ ID NO: 629 - DNA, 40 bp, Artificial Sequence
  Primer
ttaaagttcttgcagacggcggatcaggccaatactcatg

SEQ ID NO: 630 - DNA, 42 bp, Artificial Sequence
  Primer
tattggcctgatccgccgtctgcaagaactttaacggcgtag

SEQ ID NO: 631 - DNA, 45 bp, Artificial Sequence
  Primer
taaagttcttgcacatggagattcaggccaatactcatggattat

SEQ ID NO: 632 - DNA, 44 bp, Artificial Sequence
  Primer
agtattggcctgaatctccatgtgcaagaactttaacggcgtag

SEQ ID NO: 633 - DNA, 40 bp, Artificial Sequence
  Primer
aagttcttgcagcacgtaacggatcaggccaatactcatg

SEQ ID NO: 634 - DNA, 44 bp, Artificial Sequence
  Primer
tattggcctgatccgttacgtgctgcaagaactttaacggcgta

SEQ ID NO: 635 - DNA, 45 bp, Artificial Sequence
  Primer
agttcttgcagcagtaggagatggccaatactcatggattatcaa

SEQ ID NO: 636 - DNA, 45 bp, Artificial Sequence
  Primer
tgagtattggccatctcctactgctgcaagaactttaacggcgta

SEQ ID NO: 637 - DNA, 43 bp, Artificial Sequence
  Primer
ttaaagttcttgcagcatgtagcggatcaggccaatactcatg

SEQ ID NO: 638 - DNA, 44 bp, Artificial Sequence
  Primer
tattggcctgatccgctacatgctgcaagaactttaacggcgta

SEQ ID NO: 639 - DNA, 43 bp, Artificial Sequence
  Primer
aagttcttgcagcagactcttcaggccaatactcatggattat

SEQ ID NO: 640 - DNA, 41 bp, Artificial Sequence
  Primer
atgagtattggcctgaagagtctgctgcaagaactttaacg

SEQ ID NO: 641 - DNA, 42 bp, Artificial Sequence
  Primer
ttcttgcagcagactctgtaggccaatactcatggattatca

SEQ ID NO: 642 - DNA, 42 bp, Artificial Sequence
  Primer
catgagtattggcctacagagtctgctgcaagaactttaacg

SEQ ID NO: 643 - DNA, 43 bp, Artificial Sequence
  Primer
aagttcttgcagcagacgattcaggccaatactcatggattat

SEQ ID NO: 644 - DNA, 41 bp, Artificial Sequence
  Primer
atgagtattggcctgaatcgtctgctgcaagaactttaacg

SEQ ID NO: 645 - DNA, 43 bp, Artificial Sequence
  Primer
aagttcttgcagcagacaattcaggccaatactcatggattat

SEQ ID NO: 646 - DNA, 41 bp, Artificial Sequence
  Primer
atgagtattggcctgaattgtctgctgcaagaactttaacg

SEQ ID NO: 647 - DNA, 42 bp, Artificial Sequence
  Primer
ttcttgcagcagacaatctaggccaatactcatggattatca

SEQ ID NO: 648 - DNA, 42 bp, Artificial Sequence
  Primer
catgagtattggcctagattgtctgctgcaagaactttaacg

SEQ ID NO: 649 - DNA, 43 bp, Artificial Sequence
  Primer
ttcttgcagcagacggaggaggccaatactcatggattatcaa

SEQ ID NO: 650 - DNA, 38 bp, Artificial Sequence
  Primer
atgagtattggcctcctccgtctgctgcaagaacttta

SEQ ID NO: 651 - DNA, 43 bp, Artificial Sequence
  Primer
ttcttgcagcagacggagatggccaatactcatggattatcaa

SEQ ID NO: 652 - DNA, 38 bp, Artificial Sequence
  Primer
atgagtattggccatctccgtctgctgcaagaacttta

SEQ ID NO: 653 - DNA, 45 bp, Artificial Sequence
  Primer
tgcagcagacggagtaggcaactactcatggattatcaacggcat

SEQ ID NO: 654 - DNA, 45 bp, Artificial Sequence
  Primer
ataatccatgagtagttgcctactccgtctgctgcaagaacttta

SEQ ID NO: 655 - DNA, 43 bp, Artificial Sequence
  Primer
ttcttgcagcagacggacgtggccaatactcatggattatcaa

SEQ ID NO: 656 - DNA, 38 bp, Artificial Sequence
  Primer
atgagtattggccacgtccgtctgctgcaagaacttta

SEQ ID NO: 657 - DNA, 43 bp, Artificial Sequence
  Primer
aatgggccatctctggtagaatggatgtaatcaacatgagcct

SEQ ID NO: 658 - DNA, 42 bp, Artificial Sequence
  Primer
gattacatccattctaccagagatggcccattcgatgccgtt

SEQ ID NO: 659 - DNA, 40 bp, Artificial Sequence
  Primer
aatgggccatcggacgtaacatggatgtaatcaacatgag

SEQ ID NO: 660 - DNA, 42 bp, Artificial Sequence
  Primer
gattacatccatgttacgtccgatggcccattcgatgccgtt

SEQ ID NO: 661 - DNA, 43 bp, Artificial Sequence
  Primer
aatgggccatcaattctggaatggatgtaatcaacatgagcct

SEQ ID NO: 662 - DNA, 42 bp, Artificial Sequence
  Primer
gattacatccattccagaattgatggcccattcgatgccgtt

SEQ ID NO: 663 - DNA, 36 bp, Artificial Sequence
  Primer
aaaacgggacttcccaggcctcgccgcatgtagctg

SEQ ID NO: 664 - DNA, 38 bp, Artificial Sequence
  Primer
tacatgcggcgaggcctgggaagtcccgttttgcgcac

SEQ ID NO: 665 - DNA, 40 bp, Artificial Sequence
  Primer
aaggctacactggaagaaatgttaaagtagcggttatcga

SEQ ID NO: 666 - DNA, 37 bp, Artificial Sequence
  Primer
ctactttaacatttcttccagtgtagccttgagagtg

SEQ ID NO: 667 - DNA, 38 bp, Artificial Sequence
  Primer
ctacactggatcatatgttaaagtagcggttatcgaca

SEQ ID NO: 668 - DNA, 40 bp, Artificial Sequence
  Primer
taaccgctactttaacatatgatccagtgtagccttgaga

SEQ ID NO: 669 - DNA, 36 bp, Artificial Sequence
  Primer
cttctatggtggattccgaaacaaacccgtttcaag

SEQ ID NO: 670 - DNA, 36 bp, Artificial Sequence
  Primer
ggtttgtttcggaatccaccatagaagcccctccag

SEQ ID NO: 671 - DNA, 39 bp, Artificial Sequence
  Primer
tttcaagataacaatacacatggcacacacgtcgcagga

SEQ ID NO: 672 - DNA, 38 bp, Artificial Sequence
  Primer
tgtgtgccatgtgtattgttatcttgaaacgggtttgt

SEQ ID NO: 673 - DNA, 34 bp, Artificial Sequence
  Primer
gtttcaagatgaaaattctcatggcacacacgtc

SEQ ID NO: 674 - DNA, 40 bp, Artificial Sequence
  Primer
tgtgccatgagaattttcatcttgaaacgggtttgtttcg

SEQ ID NO: 675 - DNA, 39 bp, Artificial Sequence
  Primer
aacccgtttcaagatccaaattctcatggcacacacgtc

SEQ ID NO: 676 - DNA, 38 bp, Artificial Sequence
  Primer
tgccatgagaatttggatcttgaaacgggtttgtttcg

SEQ ID NO: 677 - DNA, 41 bp, Artificial Sequence
  Primer
gtttcaagataaccaatctcatggcacacacgtcgcaggaa

SEQ ID NO: 678 - DNA, 40 bp, Artificial Sequence
  Primer
tgtgtgccatgagattggttatcttgaaacgggtttgttt

SEQ ID NO: 679 - DNA, 41 bp, Artificial Sequence
  Primer
gtttcaagataacgattctcatggcacacacgtcgcaggaa

SEQ ID NO: 680 - DNA, 40 bp, Artificial Sequence
  Primer
tgtgtgccatgagaatcgttatcttgaaacgggtttgttt

SEQ ID NO: 681 - DNA, 36 bp, Artificial Sequence
  Primer
tcaagataacaatcaacatggcacacacgtcgcagg

SEQ ID NO: 682 - DNA, 40 bp, Artificial Sequence
  Primer
acgtgtgtgccatgttgattgttatcttgaaacgggtttg

SEQ ID NO: 683 - DNA, 38 bp, Artificial Sequence
  Primer
tcatggcacacacgcagcaggaacggttgcggcgttaa

SEQ ID NO: 684 - DNA, 38 bp, Artificial Sequence
  Primer
caaccgttcctgctgcgtgtgtgccatgagaattgtta

SEQ ID NO: 685 - DNA, 33 bp, Artificial Sequence
  Primer
tgtagccccggatgcttcgctctacgccgttaa

SEQ ID NO: 686 - DNA, 35 bp, Artificial Sequence; identical to SEQ ID NO: 174
  Primer

SEQ ID NO: 687 - DNA, 36 bp, Artificial Sequence
  Primer
cgttaaagttacagcagcagacggatcaggccaata

SEQ ID NO: 688 - DNA, 40 bp, Artificial Sequence
  Primer
tgatccgtctgctgctgtaactttaacggcgtagagcgaa

SEQ ID NO: 689 - DNA, 36 bp, Artificial Sequence
  Primer
taatcaacatgagcgcgggagcaccaagcggcagtg

SEQ ID NO: 690 - DNA, 35 bp, Artificial Sequence
  Primer
ttggtgctcccgcgctcatgttgattacatccatg

SEQ ID NO: 691 - DNA, 36 bp, Artificial Sequence
  Primer
taatcaacatgagcacgggagcaccaagcggcagtg

SEQ ID NO: 692 - DNA, 35 bp, Artificial Sequence
  Primer
ttggtgctcccgtgctcatgttgattacatccatg

SEQ ID NO: 693 - DNA, 38 bp, Artificial Sequence
  Primer
atgtaatcaacatggcactgggagcaccaagcggcagt

SEQ ID NO: 694 - DNA, 40 bp, Artificial Sequence
  Primer
ttggtgctcccagtgccatgttgattacatccatgttatt

SEQ ID NO: 695 - DNA, 34 bp, Artificial Sequence
  Primer
tgggagcaccaccaggcagtgcggcacttaaagc

SEQ ID NO: 696 - DNA, 36 bp, Artificial Sequence
  Primer
gtgccgcactgcctggtggtgctcccaggctcatgt

SEQ ID NO: 697 - DNA, 37 bp, Artificial Sequence
  Primer
tgagcctgggagcacttagcggcagtgcggcacttaa

SEQ ID NO: 698 - DNA, 39 bp, Artificial Sequence
  Primer
tgccgcactgccgctaagtgctcccaggctcatgttgat

SEQ ID NO: 699 - DNA, 37 bp, Artificial Sequence
  Primer
tgagcctgggagcagaaagcggcagtgcggcacttaa

SEQ ID NO: 700 - DNA, 39 bp, Artificial Sequence; identical to SEQ ID NO: 614
  Primer

SEQ ID NO: 701 - DNA, 37 bp, Artificial Sequence
  Primer
tgagcctgggagcatctagcggcagtgcggcacttaa

SEQ ID NO: 702 - DNA, 39 bp, Artificial Sequence
  Primer
tgccgcactgccgctagatgctcccaggctcatgttgat

SEQ ID NO: 703 - DNA, 35 bp, Artificial Sequence
  Primer
gactcgagccatgaagatcttaaagtcgctggagg

SEQ ID NO: 704 - DNA, 36 bp, Artificial Sequence
  Primer
gactttaagatcttcatggctcgagtcgataccgct

SEQ ID NO: 705 - DNA, 40 bp, Artificial Sequence
  Primer
gcagtccgtgcctcaaggcgtatcacaaattaaagcccct

SEQ ID NO: 706 - DNA, 40 bp, Artificial Sequence
  Primer
atttgtgatacgccttgaggcacggactgcgcgtacgcat

SEQ ID NO: 707 - DNA, 40 bp, Artificial Sequence
  Primer
cagacggatcagcacaatactcatggattatcaacggcat

SEQ ID NO: 708 - DNA, 40 bp, Artificial Sequence
  Primer
taatccatgagtattgtgctgatccgtctgctgcaagaac

SEQ ID NO: 709 - DNA, 38 bp, Artificial Sequence
  Primer
gcagcagacggaaacggccaatactcatggattatcaa

SEQ ID NO: 710 - DNA, 39 bp, Artificial Sequence
  Primer
catgagtattggccgtttccgtctgctgcaagaacttta

SEQ ID NO: 711 - DNA, 40 bp, Artificial Sequence
  Primer
ttcttgcagcagacgaatcaggccaatactcatggattat

SEQ ID NO: 712 - DNA, 40 bp, Artificial Sequence
  Primer
tgagtattggcctgattcgtctgctgcaagaactttaacg

SEQ ID NO: 713 - DNA, 38 bp, Artificial Sequence
  Primer
atcgaatgggccgtagcgaataacatggatgtaatcaa

SEQ ID NO: 714 - DNA, 40 bp, Artificial Sequence; identical to SEQ ID NO: 73
  Primer

SEQ ID NO: 715 - DNA, 38 bp, Artificial Sequence
  Primer
gttgataaagctgttaaatctggtgtcgtcgtagtagc

SEQ ID NO: 716 - DNA, 38 bp, Artificial Sequence
  Primer
gacgacaccagatttaacagctttatcaactgctgctt

SEQ ID NO: 717 - DNA, 39 bp, Artificial Sequence
  Primer
gataaagctgttgcagatggtgtcgtcgtagtagcggca

SEQ ID NO: 718 - DNA, 40 bp, Artificial Sequence
  Primer
tactacgacgacaccatctgcaacagctttatcaactgct

SEQ ID NO: 719 - DNA, 38 bp, Artificial Sequence
  Primer
aatgagggaacaaaaggatcatcgagtaccgtcggtta

SEQ ID NO: 720 - DNA, 40 bp, Artificial Sequence
  Primer
acggtactcgatgatccttttgttccctcattcccagctg

SEQ ID NO: 721 - DNA, 39 bp, Artificial Sequence
  Primer
aacatccggatcaaaaagtaccgtcggttatccaggcaa

SEQ ID NO: 722 - DNA, 39 bp, Artificial Sequence
  Primer
ataaccgacggtactttttgatccggatgttccctcatt

SEQ ID NO: 723 - DNA, 40 bp, Artificial Sequence
  Primer
tgttgcatctggtccagtcgtagtagcggcagctgggaat

SEQ ID NO: 724 - DNA, 40 bp, Artificial Sequence
  Primer
tgccgctactacgactggaccagatgcaacagctttatca

SEQ ID NO: 725 - DNA, 38 bp, Artificial Sequence
  Primer
agggaacatccggaccatcgagtaccgtcggttatcca

SEQ ID NO: 726 - DNA, 40 bp, Artificial Sequence; identical to SEQ ID NO: 113
  Primer

SEQ ID NO: 727 - DNA, 40 bp, Artificial Sequence
  Primer
cttcaaatcaacgtgactctttttcctccgtgggaccgga

SEQ ID NO: 728 - DNA, 40 bp, Artificial Sequence
  Primer
acggaggaaaaagagtcacgttgatttgaagagtctacag

SEQ ID NO: 729 - DNA, 40 bp, Artificial Sequence
  Primer
tcaacgtgcctctgattcctccgtgggaccggagctggat

SEQ ID NO: 730 - DNA, 37 bp, Artificial Sequence
  Primer
tcccacggaggaatcagaggcacgttgatttgaagag

SEQ ID NO: 731 - DNA, 38 bp, Artificial Sequence
  Primer
tactatggaaaaggggtaatcaacgtacaggcggcagc

SEQ ID NO: 732 - DNA, 38 bp, Artificial Sequence
  Primer
ctgtacgttgattaccccttttccatagtagaaagaat

SEQ ID NO: 733 - DNA, 36 bp, Artificial Sequence
  Primer
tggcgtttctattgaatcgacgcttccagggaacaa

SEQ ID NO: 734 - DNA, 37 bp, Artificial Sequence
  Primer
ctggaagcgtcgattcaatagaaacgccaggggccat

SEQ ID NO: 735 - DNA, 36 bp, Artificial Sequence
  Primer
cttccagggaacacatatggtgcgcaaaacgggact

SEQ ID NO: 736 - DNA, 38 bp, Artificial Sequence
  Primer
gttttgcgcaccatatgtgttccctggaagcgtcgatt

SEQ ID NO: 737 - DNA, 36 bp, Artificial Sequence
  Primer
cttccagggaacctttatggtgcgcaaaacgggact

SEQ ID NO: 738 - DNA, 38 bp, Artificial Sequence
  Primer
gttttgcgcaccataaaggttccctggaagcgtcgatt

SEQ ID NO: 739 - DNA, 40 bp, Artificial Sequence
  Primer
tttctactatggaaacgggctgatcaacgtacaggcggca

SEQ ID NO: 740 - DNA, 40 bp, Artificial Sequence
  Primer
acgttgatcagcccgtttccatagtagaaagaatcaccaa

SEQ ID NO: 741 - DNA, 39 bp, Artificial Sequence
  Primer
tttctaagcacccgaaatggacaaacactcaagtccgca

SEQ ID NO: 742 - DNA, 38 bp, Artificial Sequence
  Primer
gagtgtttgtccatttcgggtgcttagaaagaatcaat

SEQ ID NO: 743 - DNA, 39 bp, Artificial Sequence
  Primer
ttctttctaagcaccgtaactggacaaacactcaagtcc

SEQ ID NO: 744 - DNA, 38 bp, Artificial Sequence
  Primer
tgtttgtccagttacggtgcttagaaagaatcaatgcg

SEQ ID NO: 745 - DNA, 36 bp, Artificial Sequence
  Primer
cacccgaactggcgtaacactcaagtccgcagcagt

SEQ ID NO: 746 - DNA, 40 bp, Artificial Sequence
  Primer
tgcggacttgagtgttacgccagttcgggtgcttagaaag

SEQ ID NO: 747 - DNA, 33 bp, Artificial Sequence
  Primer
cgtctgcttacctctacgccgttaaagttcttg

SEQ ID NO: 748 - DNA, 40 bp, Artificial Sequence
  Primer
actttaacggcgtagaggtaagcagacggggctacaccaa

SEQ ID NO: 749 - DNA, 36 bp, Artificial Sequence
  Primer
agcctgggagcacaaagcggcagtgcggcacttaaa

SEQ ID NO: 750 - DNA, 34 bp, Artificial Sequence
  Primer
cactgccgctttgtgctcccaggctcatgttgat

SEQ ID NO: 751 - DNA, 41 bp, Artificial Sequence
  Primer
ttcaatcgacgcttccaacgaacaagtatggtgcgcaaaac

SEQ ID NO: 752 - DNA, 39 bp, Artificial Sequence
  Primer
caccatacttgttcgttggaagcgtcgattgaatagaaa

SEQ ID NO: 753 - DNA, 39 bp, Artificial Sequence
  Primer
tggattatcaacggcgtagaatgggccatcgcgaataac

SEQ ID NO: 754 - DNA, 39 bp, Artificial Sequence
  Primer
cgatggcccattctacgccgttgataatccatgagtatt

SEQ ID NO: 755 - protein, 269 aa, Bacillus lentus
AQSVPWGISRVQAPAAHNRGLTGSGVKVAVLDTGISTHPDLNIRGGASFVPGEPSTQDGNGHGTHVAGTIAALNNSIGVLGVAPSAELYAVKVLGASGSGSVSSIAQGLEWAGNNGMHVANLSLGSPSPSATLEQAVNSATSRGVLVVAASGNSGAGSISYPARYANAMAVGATDQNNNRASFSQYGAGLDIVAPGVNVQSTYPGSTYASLNGTSMATPHVAGAAALVKQKNPSWSNVQIRNHLKNTATSLGSTNLYGSGLVNAEAATR

SEQ ID NO: 756 - DNA, 1143 bp, Bacillus lentus
gtgagaagcaaaaaattgtggatcgtcgcgtcgaccgcactactcatttctgttgctttcagttcatcgatcgcatcggctgctgaagaagcaaaagaaaaatatttaattggctttaatgagcaggaagctgtcagtgagtttgtagaacaagtagaggcaaatgacgaggtcgccattctctctgaggaagaggaagtcgaaattgaattgcttcatgaatttgaaacgattcctgttttatccgttgagttaagcccagaagatgtggacgcgcttgagctcgatccagcgatttcttatattgaagaggatgcagaagtaacgacaatggcgcaatcagtgccatggggaattagccgtgtgcaagccccagctgcccataaccgtggattgacaggttctggtgtaaaagttgctgtcctcgatacaggtatttccactcatccagacttaaatattcgtggtggcgctagctttgtaccaggggaaccatccactcaagatgggaatgggcatggcacgcatgtggccgggacgattgctgctttaaacaattcgattggcgttcttggcgtagcgccgagcgcggaactatacgctgttaaagtattaggggcgagcggttcaggttcggtcagctcgattgcccaaggattggaatgggcagggaacaatggcatgcacgttgctaatttgagtttaggaagcccttcgccaagtgccacacttgagcaagctgttaatagcgcgacttctagaggcgttcttgttgtagcggcatctggaaattcaggtgcaggctcaatcagctatccggcccgttatgcgaacgcaatggcagtcggagctactgaccaaaacaacaaccgcgccagcttttcacagtatggcgcagggcttgacattgtcgcaccaggtgtaaacgtgcagagcacatacccaggttcaacgtatgccagcttaaacggtacatcgatggctactcctcatgttgcaggtgcagcagcccttgttaaacaaaagaacccatcttggtccaatgtacaaatccgcaatcatctaaagaatacggcaacgagcttaggaagcacgaacttgtatggaagcggacttgtcaatgcagaagctgcaactcgttaa

SEQ ID NO: 757 - protein, 380 aa, Artificial Sequence
  Mutant of Bacillus lentus subtilisin
VRSKKLWIVASTALLISVAFSSSIASAAEEAKEKYLIGFNEQEAVSEFVEQVEANDEVAILSEEEEVEIELLHEFETIPVLSVELSPEDVDALELDPAISYIEEDAEVTTMAQSVPWGISRVQAPAAHNRGLTGSGVKVAVLDTGISTHPDLNIRGGASFVPGEPSTQDGNGHGTHVAGTIAALNNSIGVLGVAPSAELYAVKVLGASGSGSVSSIAQGLEWAGNNGMHVANLSLGSPSPSATLEQAVNSATSRGVLVVAASGNSGAGSISYPARYANAMAVGATDQNNNRASFSQYGAGLDIVAPGVNVQSTYPGSTYASLNGTSMATPHVAGAAALVKQKNPSWSNVQIRNHLKNTATSLGSTNLYGSGLVNAEAATR

SEQ ID NO: 758 - DNA, 27 bp, Artificial Sequence
  Primer
cgcgcttgagctcgatccagcgatttc

SEQ ID NO: 759 - DNA, 25 bp, Artificial Sequence
  Primer
gtctccaagctttaacgagttgcag

SEQ ID NO: 760 - DNA, 30 bp, Artificial Sequence
  Primer
gcaattcagatcttccttcaggttatgacc

SEQ ID NO: 761 - DNA, 30 bp, Artificial Sequence
  Primer
gcatcgaagatctgattgcttaactgcttc

SEQ ID NO: 762 - DNA, 1143 bp, Artificial Sequence
  Mutant of Bacillus lentus subtilisin
gtgagaagcaaaaaattgtggatcgtcgcgtcgaccgcactactcatttctgttgcttttagttcatcgatcgcatcggctgctgaagaagcaaaagaaaaatatttaattggctttaatgagcaggaagctgtcagtgagtttgtagaacaagtagaggcaaatgacgaggtcgccattctctctgaggaagaggaagtcgaaattgaattgcttcatgaatttgaaacgattcctgttttatccgttgagttaagcccagaagatgtggacgcgcttgaactcgatccagcgatttcttatattgaagaggatgcagaagtaacgacaatggcgcaatcagtgccatggggaattagccgtgtgcaagccccggctgcccataaccgtggattgacaggttctggtgtaaaagttgctgtcctcgatacaggtatttccactcatccagacttaaatattcgtggtggcgctagctttgtaccaggggaaccatccactcaagatgggaatgggcatggcacgcatgtggccgggacgattgctgctctaaacaattcgattggcgtacttggcgtagcgccgagcgcggaactatacgctgttaaagtattaggggcgagcggtgggggcgccatcagctcgattgcccaaggattggaatgggcagggaacaatggcatgcacgttgctaatttgagtttaggaagcccttcgccaagtgccacacttgagcaagctgttaatagcgcgacttctaggggcgttcttgttgtagcggcatctggaaattcgggtgcagactcaatcagctatccggcccgttatgcgaacgcaatggcagtcggagctactgaccaaaacaacaaccgcgccagcttttcacagtatggcgcagggcttgacatcgtcgcaccaggtgtaaacgtgcagagcacatacccaggttcaacgtatgccagcttaaacggtacatcgatggctactcctcatgttgcaggtgcagcagtccttgttaaacataagaacccatcttggtccaatgtacgaatccgcgatcatctaaagaaaacggcaacgagcttaggaagcacgaacttgtatggaagcggacttgtcaatgccgaagctgcaactcgttaa

SEQ ID NO: 763 - protein, 380 aa, Artificial Sequence
  Mutant of Bacillus Lentus subtilisin
VRSKKLWIVASTALLISVAFSSSIASAAEEAKEKYLIGFNEQEAVSEFVEQVEANDEVAILSEEEEVEIELLHEFETIPVLSVELSPEDVDALELDPAISYIEEDAEVTTMAQSVPWGISRVQAPAAHNRGLTGSGVKVAVLDTGISTHPDLNIRGGASFVPGEPSTQDGNGHGTHVAGTIAALNNSIGVLGVAPSAELYAVKVLGASGGGAISSIAQGLEWAGNNGMHVANLSLGSPSPSATLEQAVNSATSRGVLVVAASGNSGADSISYPARYANAMAVGATDQNNNRASFSQYGAGLDIVAPGVNVQSTYPGSTYASLNGTSMATPHVAGAAVLVKHKNPSWSNVRIRDHLKKTATSLGSTNLYGSGLVNAEAATR

SEQ ID NO: 764 - DNA, 1140 bp, Artificial Sequence
  Mutant of Bacillus Lentus subtilisisn
gtgagaagcaaaaaattgtggatcgtcgcgtcgaccgcactactcatttctgttgcttttagttcatcgatcgcatcggctgctgaagaagcaaaagaaaaatatttaattggctttaatgagcaggaagctgtcagtgagtttgtagaacaagtagaggcaaatgacgaggtcgccattctctctgaggaagaggaagtcgaaattgaattgcttcatgaatttgaaacgattcctgttttatccgttgagttaagcccagaagatgtggacgcgcttgaactcgatccagcgatttcttatattgaagaggatgcagaagtaacgacaatggcgcaatcagtgccatggggaattagccgtgtgcaagccccggctgcccataaccgtggattgacaggttctggtgtaaaagttgctgtcctcgatacaggtatttccactcatccagacttaaatattcgtggtggcgctagctttgtaccaggggaaccatccactcaagatgggaatgggcatggcacgcatgtggccgggacgattgctgctctaaacaattcgattggcgtacttggcgtagcgccgagcgcggaactatacgctgttaaagtattaggggcgagcggtgggggcgccatcagctcgattgcccaaggattggaatgggcagggaacaatggcatgcacgttgctaatttgagtttaggaagcccttcgccaagtgccacacttgagcaagctgttaatagcgcgacttctaggggcgttcttgttgtagcggcatctggaaattcgggtgcagactcaatcagctatccggcccgttatgcgaacgcaatggcagtcggagctactgaccaaaacaacaaccgcgccagcttttcacagtatggcgcagggcttgacatcgtcgcaccaggtgtaaacgtgcagagcacatacccaggttcaacgtatgccagcttaaacggtacatcgatggctactcctcatgttgcaggtgcagcagtccttgttaaacaaaagaacccatcttggtccaatgtacgaatccgcgatcatctaaagaatacggcaacgagcttaggaagcacgaacttgtatggaagcggacttgtcaatgccgaagctgcaactcgt

SEQ ID NO: 765 - protein, 380 aa, Artificial Sequence
  Mutant of Bacillus lentus subtilisin
VRSKKLWIVASTALLISVAFSSSIASAAEEAKEKYLIGFNEQEAVSEFVEQVEANDEVAILSEEEEVEIELLHEFETIPVLSVELSPEDVDALELDPAISYIEEDAEVTTMAQSVPWGISRVQAPAAHNRGLTGSGVKVAVLDTGISTHPDLNIRGGASFVPGEPSTQDGNGHGTHVAGTIAALNNSIGVLGVAPSAELYAVKVLGASGGGAISSIAQGLEWAGNNGMHVANLSLGSPSPSATLEQAVNSATSRGVLVVAASGNSGADSISYPARYANAMAVGATDQNNNRASFSQYGAGLDIVAPGVNVQSTYPGSTYASLNGTSMATPHVAGAAVLVKQKNPSWSNVRIRDHLKNTATSLGSTNLYGSGLVNAEAATR

SEQ ID NO: 766 - DNA, 1326 bp, Artificial sequence
  Artificial
gaattcatctcaaaaaaatgggtctactaaaatattattccatctattataataaattcacagaatagtcttttaagtaagtctactctgaatttttttaaaaggagagggtaaagagtgagaagcaaaaaattgtgagaagcaaaaaattgtggatcagtttgctgtttgctttagcgttaatctttacgatggcgttcggcagcacatccagcgcgcaggctgcagggaaatcaaacggggaaaagaaatatattgtcgggtttaaacagacaatgagcacgatgagcgccgctaagaagaaagacgtcatttctgaaaaaggcgggaaagtgcaaaagcaattcaaatatgtagacgcagctagcgctacattaaacgaaaaagctgtaaaagaattgaaaaaagacccgagcgtcgcttacgttgaagaagatcacgtagcacacgcgtacgcgcagtccgtgccatatggcgtatcacaaattaaagcccctgctctgcactctcaaggctacaccggttcaaatgttaaagtagcggttatcgacagcggtatcgattcttctcatccagatcttaaagtagcaggcggagccagcatggttccttctgaaacaaatcctttccaagacaacaactctcacggaacacacgttgctggtaccgttgcggctcttaataactcaatcggtgtattaggcgttgcgccaagcgcatcactttacgctgtaaaagttctcggcgccgacggttccggccaatacagctggatcattaacggaatcgagtgggcgatcgcaaacaatatggacgttattaacatgagcctcggcggaccgtccggttctgctgctttaaaagcggcagttgataaagccgttgcatccggcgtcgtagtcgttgcggcagccggcaacgaaggcacttccggcagctcaagcacagtgggctaccctggtaaatacccttctgtcattgcagtaggcgctgtcgacagcagcaaccaaagagcatctttctcaagcgtaggacctgagctcgatgtcatggcacctggcgtatctatccaaagcacgcttcctggaaacaaatacggcgcgttgaacggtacatcaatggcatctccgcacgttgccggagccgcggctttgattctttctaagcacccgaactggacaaacactcaagtccgcagctctctagaaaacaccactacaaaacttggtgattctttctactatggaaaagggctgatcaatgtacaggcggcagctcagtaaaactcgagataaaaaaccggccttggccccgccggttttttat

SEQ ID NO: 767 - protein, 382 aa, Artificial sequence
  Artificial sequence
MRSKKLWISLLFALALIFTMAFGSTSSAQAAGKSNGEKKYIVGFKQTMSTMSAAKKKDVISEKGGKVQKQFKYVDAASATLNEKAVKELKKDPSVAYVEEDHVAHAYAQSVPYGVSQIKAPALHSQGYTGSNVKVAVIDSGIDSSHPDLKVAGGASMVPSETNPFQDNNSHGTHVAGTVAALNNSIGVLGVAPSASLYAVKVLGADGSGQYSWIINGIEWAIANNMDVINMSLGGPSGSAALKAAVDKAVASGVVVVAAAGNEGTSGSSSTVGYPGKYPSVIAVGAVDSSNQRASFSSVGPELDVMAPGVSIQSTLPGNKYGALNGTSMASPHVAGAAALILSKHPNWTNTQVRSSLENTTTKLGDSFYYGKGLINVQAAAQ

SEQ ID NO: 768 - protein, 275 aa, Artificial sequence
  Artificial sequence
AQSVPYGVSQIKAPALHSQGYTGSNVKVAVIDSGIDSSHPDLKVAGGASMVPSETNPFQDNNSHGTHVAGTVAALNNSIGVLGVAPSASLYAVKVLGADGSGQYSWIINGIEWAIANNMDVINMSLGGPSGSAALKAAVDKAVASGVVVVAAAGNEGTSGSSSTVGYPGKYPSVIAVGAVDSSNQRASFSSVGPELDVMAPGVSIQSTLPGNKYGALNGTSMASPHVAGAAALILSKHPNWTNTQVRSSLENTTTKLGDSFYYGKGLINVQAAAQ

SEQ ID NO: 769 - DNA, 22 bp, Artificial sequence
  Artificial sequence
cgttgaagaagatcacgtagca

SEQ ID NO: 770 - DNA, 26 bp, Artificial sequence
  Artificial sequence
tttattttataaactcattccctgat

SEQ ID NO: 771 - DNA, 1351 bp, Artificial sequence
  Artificial sequence
gcttttcttttggaagaaaatatagggaaaatggtacttgttaaaaattcggaatatttatacaatatcatatgtttcacattgaaaggggaggaaaatcgtgaaacaacaaaaacggctttagtctagcaaaaggagagggtaaagagtgagaagcaaaaaattgtggatcagtttgctgtttgctttagcgttaatctttacgatggcgttcggcagcacatcctctgcccaggcggcagggaaatcaaacggggaaaagaaatatattgtcgggtttaaacagacaatgagcacgatgagcgccgctaagaagaaagatgtcatttctgaaaaaggcgggaaagtgcaaaagcaattcaaatatgtagacgcagcttcagctacattaaacgaaaaagctgtaaaagaattgaaaaaagacccgagcgtcgcttacgttgaagaagatcacgtagcacacgcgtacgcgcagtccgtgccttacggcgtatcacaaattaaagcccctgctctgcactctcaaggctacactggatcaaatgttaaagtagcggttatcgacagcggtatcgattcttctcatcctgatttaaaggtagcaggcggagccagcatggttccttctgaaacaaatcctttccaagacaacaactctcacggaactcacgttgccggcacagttgcggctcttaataactcaatcggtgtattaggcgttgcgccaagcgcatcactttacgctgtaaaagttctcggtgctgacggttccggccaatacagctggatcattaacggaatcgagtgggcgatcgcaaacaatatggacgttattaacatgagcctcggcggaccttctggttctgctgctttaaaagcggcagttgataaagccgttgcatccggcgtcgtagtcgttgcggcagccggtaacgaaggcacttccggcagctcaagcacagtgggctaccctggtaaatacccttctgtcattgcagtaggcgctgttgacagcagcaaccaaagagcatctttctcaagcgtaggacctgagcttgatgtcatggcacctggcgtatctatccaaagcacgcttcctggaaacaaatacggcgcgttgaacggtacatcaatggcatctccgcacgttgccggagcggctgctttgattctttctaagcacccgaactggacaaacactcaagtccgcagcagtttagaaaacaccactacaaaacttggtgattctttctactatggaaaagggctgatcaacgtacaggcggcagctcagtaaactcgagagaggacggatttcctgaaggaaatccgtttttttattttaagcttg